European Patent Specification EP 3 711 771 B1, published September 3, 2025. Title: Mitigating Tissue Damage And Fibrosis Via Latent Transforming Growth Factor Beta Binding Protein (LTBP4). Applicant: McNally, et al. The sequence listing filed with the application follows.

SEQUENCE LISTING (7 sequences)

SEQ ID NO: 1 - protein, 1624 aa, Homo sapiens
  MISC_FEATURE (357)..(586): TP2E fragment
  MISC_FEATURE (483)..(565): TP fragment
MPRPGTSGRRPLLLVLLLPLFAAATSAASPSPSPSQVVEVPGVPSRPASVAVCRCCPGQTSRRSRCIRAFCRVRSCQPKKCAGPQRCLNPVPAVPSPSPSVRKRQVSLNWQPLTLQEARALLKRRRPRGPGGRGLLRRRPPQRAPAGKAPVLCPLICHNGGVCVKPDRCLCPPDFAGKFCQLHSSGARPPAPAVPGLTRSVYTMPLANHRDDEHGVASMVSVHVEHPQEASVVVHQVERVSGPWEEADAEAVARAEAAARAEAAAPYTVLAQSAPREDGYSDASGFGYCFRELRGGECASPLPGLRTQEVCCRGAGLAWGVHDCQLCSERLGNSERVSAPDGPCPTGFERVNGSCEDVDECATGGRCQHGECANTRGGYTCVCPDGFLLDSSRSSCISQHVISEAKGPCFRVLRDGGCSLPILRNITKQICCCSRVGKAWGRGCQLCPPFGSEGFREICPAGPGYHYSASDLRYNTRPLGQEPPRVSLSQPRTLPATSRPSAGFLPTHRLEPRPEPRPDPRPGPELPLPSIPAWTGPEIPESGPSSGMCQRNPQVCGPGRCISRPSGYTCACDSGFRLSPQGTRCIDVDECRRVPPPCAPGRCENSPGSFRCVCGPGFRAGPRAAECLDVDECHRVPPPCDLGRCENTPGSFLCVCPAGYQAAPHGASCQDVDECTQSPGLCGRGACKNLPGSFRCVCPAGFRGSACEEDVDECAQEPPPCGPGRCDNTAGSFHCACPAGFRSRGPGAPCQDVDECARSPPPCTYGRCENTEGSFQCVCPMGFQPNTAGSECEDVDECENHLACPGQECVNSPGSFQCRTCPSGHHLHRGRCTDVDECSSGAPPCGPHGHCTNTEGSFRCSCAPGYRAPSGRPGPCADVNECLEGDFCFPHGECLNTDGSFACTCAPGYRPGPRGASCLDVDECSEEDLCQSGICTNTDGSFECICPPGHRAGPDLASCLDVDECRERGPALCGSQRCENSPGSYRCVRDCDPGYHAGPEGTCDDVDECQEYGPEICGAQRCENTPGSYRCTPACDPGYQPTPGGGCQDVDECRNRSFCGAHAVCQNLPGSFQCLCDQGYEGARDGRHCVDVNECETLQGVCGAALCENVEGSFLCVCPNSPEEFDPMTGRCVPPRTSAGTFPGSQPQAPASPVLPARPPPPPLPRRPSTPRQGPVGSGRRECYFDTAAPDACDNILARNVTWQECCCTVGEGWGSGCRIQQCPGTETAEYQSLCPHGRGYLAPSGDLSLRRDVDECQLFRDQVCKSGVCVNTAPGYSCYCSNGYYYHTQRLECIDNDECADEEPACEGGRCVNTVGSYHCTCEPPLVLDGSQRRCVSNESQSLDDNLGVCWQEVGADLVCSHPRLDRQATYTECCCLYGEAWGMDCALCPAQDSDDFEALCNVLRPPAYSPPRPGGFGLPYEYGPDLGPPYQGLPYGPELYPPPALPYDPYPPPPGPFARREAPYGAPRFDMPDFEDDGGPYGESEAPAPPGPGTRWPYRSRDTRRSFPEPEEPPEGGSYAGSLAEPYEELEAEECGILDGCTNGRCVRVPEGFTCRCFDGYRLDMTRMACVDINECDEAEAASPLCVNARCLNTDGSFRCICRPGFAPTHQPHHCAPARPRA

SEQ ID NO: 2 - protein, 18 aa, Mus musculus
EPRPRPEPRPQPESQPWP

SEQ ID NO: 3 - protein, 17 aa, Homo sapiens
EPRPEPRPDPRPGPELP

SEQ ID NO: 4 - protein, 18 aa, Mus musculus
ESQPRPESRPRPESQPWP

SEQ ID NO: 5 - protein, 19 aa, Homo sapiens
EPRPEPRPDPRPGPELPLP

SEQ ID NO: 6 - protein, 43 aa, Homo sapiens
FLPTHRLEPRPEPRPDPRPGPELPLPSIPAWTGPEIPESGPSS

SEQ ID NO: 7 - DNA, 155085 bp, Homo sapiens
aagctttatattataaatacaaagtaaacatgaaaataaaacccaaacatagcagtgttattaaactctggcctgtagcagtggctcacacctgtaatcctagcagtttggaggccgagacaggtggattacttgagacctggagtttgagaccagcccaggtgacacagcaagacctcatctctactaaaaataaaaaaaaattagccaggtgtggtggtatgcacctgtggtcccagctacttaggatgctggagtgcgaggatcgcttgagcccaggaggtcaaggctgcagtgaactatgatcactcattacaccccagcctgggtgacagagcgagatgctgtctcaaaacaaaacaaaacgaaaaacaactctggctagatgctattgcttgccaagggtgcagtcttccatttattaaaagtgaaaattagggccaggcacattggctcatgcctgtaatcccagcactttgggaggctgaggtgggtggatcacctgaggtcaggagttcgagaccagcctggccaacatggtgaaaccttatctctgccaaaaatataaaagattagccatgtgtcgtggtgggtgcttgtaatctcagctacttgggaggctgaggcaggagaatcacttgaacccaggaggcagaggttgcagtgagccaagattgtgccattgcactccagcctgtgcaacgagcgaaactccaactcaaaaaaaaaaaaaaaaaaaaaaacggaaaattaggtaatactgcagattcattaatatcacagcagcactaaactcagtcttcctctgtgctgggctcaagggaactgaaagggaagtaacttgctatgtggttcagtgtcatttcatgctgtgtcactgcaccacttaaaatcttcacccggagactatgtcccacacatggggaaatcaatcaccgtcatattttaagtgcttgctgtgtgacagccacgattacaatgactgttactctacctcttattctcactgtagtgttcccagtgaagcggcggaaccggcacagcctagtggggcctcagcagctaggaggacggccagcccctgtccgacggagcaacacgatgccccccaaccttggcaatgcagggctgctgggccgaatgctggatgagaaaacccctccctcaccctcaggtacgtttctatctcgtggaaggttggggcagctgtggggtccctgtgaccctcttctgatccctactcttcccctcaaggacaacctgaggagccggggatggtgcgcctggtgtgtggacaccataattggatcgctgtggcctatacccagtttctagtctgctacaggtgcttggggagggagtggcaggaggtcccagccctgttgatgggaagggcatgcggtgagggttggtgatgtcccctcgatcctacaggttgaaggaagcctctggctggcagctggtgttttccagcccccgcctggactggcccatcgaacgactggcgctcacagcccgggtgcatggtggggctttgggtgaacatgacaagatggtggcagcagccaccggcagcgagatcctgctatgggctctgcaggcggaaggcggtggctccgagataggtatgaccccaagccttttccagaaccctctgtcctttaaattctactgcctgttaaaatgacccaccccataaaatcctcaaacccataagaattctctgctctattagatctgtttgtgtcattagaatgctccagcccttcagaattctgtatcctgttagaattccctggcttcctagaaaaatccacccacatacaattctccctccatcagaattccctgccctgttagatctcttggttttgttagaatgcgctattctgtgtggccatgagaaatgtctgacttggcccggtgcggtggctcatgcttgtaatcccagcactttgggaggctgaggcgggcagatcacttgaggtcaggagttcgagacccccttggccaacagggtgaaacccagtctttatttcaaaaatacaaaaaaattagctgggtgtggtggcacgtgcctgtaatcccagctactcaggaggttaaggcaggagaatcactggaacctgggaggcagatgttgcagtgagctgagatcgcaccactgcattccagcctgagcgacagagtggacagagtgagacaccatctcaaaaaaaaaaaaaaaacaaaaaaagaaatctctgacttatggctgggcacagtaactcacatctgtagttccagcactttgggaggccatggcaggaggattgcttgaggccaggagttcgaggctgccgtgagctatgtaagccatgattgcaccactgcactccagcctggacaacagagcaagaccctgtctcaaagccacagcaacaaatctcggacttattaatctgtccccaaataaatctcagccctcgtaagaatcccctgccaccagtggaggtttttttgccttattgcaaatctcagtgctgttagaattccagaccgttttagaatcccataccccatcagaaatcttctggcccattttatcttctctaattcctgctggaatcttcactttttttttttttgaaatggagtcattctctgttgcccagattggagtacagtggtatgatctcggctcactgcaacctctgcctcctggggtcacgcaattctccttcctcaacctcccaagtagctggggctacagttgtgtgctaccacactcagctaatttttatattttttagtagagatggagtttcatcatgttggccaggctggtctcaaactcctggcctcaaatgatccgcccacctgagcctctcaaagtgttgggattacaggtgtgagccactgtgcccagcccctgatggaatcttctatccttcaaggattctgtggtcccactgaaccctctggtccttggagttcttcctcccacctctcctcctccatgaggcagggttccagctgagccctttttgcccactgcaggggtctttcatctgggggtgcctgtggaggccttgttcttcgtcgggaaccagctcattgctacaagccacacagggcgcatcggggtgtggaatgccgtcaccaagcactggcaggtcagagttctggccagcctggctgcccccttcccagttttccagactgtacagacccaggaaggggttcacgtctgcccccacccccaccccctaagcctggaggaagccagagaaccagcagctggccagagcctggggatgtctgtgataaaggcctaaggagcaccagggaagccttcctggaggaggtgctgcagagcccacatgaagcatgaatgggtttgaaaaggagtagggaggattgtcttgggactgggtgagagagcaggttaggggggatgctgtagaagacaagaactggcttggctcggtggctcacacttgtaatcccagcactttgggaggctgaggtgggaggatggctttgggagaaagacagacagaggcagagaaagagacagagaggcagaaaaccaggcaaatagaaatagaaaatcagaaagaggtgacagagaagggtagacagagtcaaaccagactgaaccactgtggcagatgggggaactcagagagataaatggagatgaattagagtcatgtcagaagtacatagtggaggccgggtgcagtgactcccgcccgtaatcccagcactttgggaggccgaggcaagaggatggcttgagcccaggagtttgacgccagcctgggaaacataataagactctgtctctacaaaaaatttaaaaaattaaaactttaaaaagtacagagtccaggagaggccaagagtcagacagacagatgcatcaaagggaggaagggagggaacaagacagggacaaaggcaggcctggggtggacggggctggggagcagtgggtgggttctggaggtggaggagagggcccatcctctgtgaggggtcaccacggaaggaaaggaatggaagggctcccggctgcagcctgtcctgccccacccccaggtccaggaggtgcagcccatcaccagttatgacgcggcaggctccttcctcctcctgggctgcaacaacggctccatttactacgtgggtgagcagcagcctgtgtcccgggtgcccgagaccctcccctgggagaggggaagggagggagagaggctggggcacttggaacaaacccgctccaccctccctgcccaccccagatgtgcagaagttccccttgcgcatgaaagacaacgacctccttgtcagcgagctctatcgggacccagcggaggatggggtcaccgccctcagtgtctacctcacccccaagaccagtaagctatgacccggcttcccctgctgctgtcacctgccagccccagccccagcctgcagctgtcccccaacttgtgtagcatgacccagaggggtttatcgaggggcggcagattcaactctctctcatttttttttctgagacagactctcattctgttgcccaggctggagtgcagtggtgcaatcttggctcactgcaacctccacctcctgagttcaagcgattctcctgcctcagcctcccaagtagctaggattacaggcgcccactgccacgcctggctaatttttgtagttttagtagagatggggtttcaccatgttggccaggctggtcttgaactcctgacctcagatgatcctcccgcctcagccccccaaagtactgggattacagacgtgagccaccgcgcccagccagattcaactctcatccagtcattcaacaaatatttactgagtatccctgtatataagcacgttctaggtgctagatggtggccaccctctccactaggggcagaatggaccattaggagttaatctttgtgtttctttcccacctttgtgattaaggcatgatgttcacatgttcataaaacaacacagatgcaggttttacagcagatgaacctgagttctcttacttgagacagttttttgttttgttttcttgacatcaaatgcagaatgggttaatttttgagacgtaattctcataccataaaatttcccatttgaacgtgcacaattcagcggattttagtatattcacaaggttgtacaactatcaccatgaacaaattccagagtatgttcatcacccccgtaagaaaccccctgatctttagcagtaactccacatttctcacttctgataccctctagaaatcactaatatgctttctctttttgtttgagacaaggtctcgctctgctgcccaggctggagtgcagtggcatgatctcagctcactgcaatctctgcctcttgggttcaagcgattctcatgcctcagcttcctgagtaggggaggattacaggtgtgcatcaccatgcctggctaatttttctactttaagtagagactgggttacgccacgttggccaggctcaatatgcttcctatacctatggatttgcctgttctggacaattcctgtaaatgggatcatacattatatggtcttttgtgtctgcatttttcacttagcatatttttttaaatggttagtgttttctgggtcttaagatatccttacctattctaggttacaaagatcttctcctgaatttcttctagaagatttacagtttagtttttacatggaagtctgttctatcagaaattaaattttatgtatggtgtgaagcagggattattcttttttaaaaaaaaatagagacagggtcttgctctgttgcccaggctagagtgcagtggcatgatgtgagttctctgccacctccgccactcgggctcaagcgattcttctacctcaacctcctgaacagcagaaccacaggcatgcatcaccacacctgtctaatttttgtatttttttgtagagacagggttttgccatgttgcccaggctactcttgaactcctgggctcaagtgatcctcacactttggcctccaaagtgctggaaatacagacttgagtcactgtgcttggccatagctgctgctgctgcttttcttttttttttaaagcagaaataagttaataatacacctaacttcatgacacattatcacctttcttctttgtaaggcccttttcttatttcttttttttctttctttctttttttttttttttgtcttttcctgagacagagtatcgctctgtcattcaacccaggctggagtgcaatggcgcaatctcagctcactacaacctctgcctcctgggttcaagcaattctccagactcagcctcccaagtagctgggattacgggtgcctgccaccatgcccagctaatttttgtgtttttagtagaggcagggttttgccacgttggctaagcaagttttgaactcctgggattctcctctcgtcgtctcccaaagtgctggaattacaggcatgggctgctgcacccggcctctttcttatttcacttacttactcatttcctcctcatctcccttcccgccacatgccactattatgtcatttttctttgttttttgagacagtctcgcttcgtcacctaggctggagtgcagtggcgcaatcatagctcactgcagcctcaccccctgggctcaagtgatcctcctacttcagcctcttgagtagctgggatcataggtgaatgccatcacacccaactagttttttaaaaatcttttgtagagatgagggtctcactatgttgcccaggctggcctcaaacgcctggcctcaagcaatcttcctgcctcggcctctgttctctgttttactttctctttcctctcttatttgctgtttcactgttacaatttctgtctctgggcctctcctcctttgacctgtgcctttgtctccctgttcctccatttcccacatctcatcaccatctttttgtgtccttccctctctccttgctttctgactgtgtctctgttctgtgtctctttctttctttctttctttttttttttttgagacagagtcacattctgtcatgcaggctggagtgcagtggcgtggtcttggctcattgcaacctctgcctcctgggttcaagcaattctcatgcctcagccttctgagtagctgggattacaggtgcgtactaccaccaccagctaatttttgtatttttactagagacagggtttcagcacgttggccaggctggtcttgaacgcctgacctcaagcgatccacccgcctcagcttcccaaagtgatgggattacggcgtgagccaccgtgcccggcctctccttgctttctgactgtgtctctgttctgtgcctgtttctttctccctgccctggtttctgtctctgtggcccaggccctctcctcatccttggcccctcaccaggtgacagtgggaactggatcgagatcgcctatggcaccagctcagggggcgtgcgggtcatcgtgcagcacccggagactgtgggctcggggcctcagctcttccagaccttcactgtgcaccgcagccctgtcaccaagatcatgctgtcggagaagcacctcatctcaggtgagcctctgtggggtgctccagtgctgggagagacagctcagatgggagtgtggagacaggaggatgagaatttccactggggagggacattgtgtaggaagagagctctggcggagaggattgacctgggatgggactgtaattgcagaagtgagagaataccataggggatcagtctggggaagagtgaatctgtgtgtgtttgggaatccatcaattcagcaacgatttacggggcacccaccatgtgccaggcataggggatacagtgatgaacaagacaggccaagtccctgccctcgtggagctgacattctagcagcgatggcagacaataaatctataaaaatggacatcaatggccagctgcggtggctcacacctataatcccagaactttgggaggccaaggcgggtagattacttgaggtcaggagttcgagaccagcctggccaacatggtgaaaccccacctctaccaaaaatataaaaaattagccaggtgtggtggcacgtgcctgtaatccccgctactcgggaggccgagggaggagaattgcttgaacctgggaggcggagattgcagagagcccagatcatgctactgcactccagcctaggcaacagagcgagactccatctcaaaaataaatagataaaaatgcaaatcaggctgggcactgtggctcatgcctataatcccagcactttgggaggccaaggtgggaggattgcttgaggctaggagtgtgagaccaacctggacaacaaagtgagacattgtttctacaaaaaatttttaaaaaattagccaagtatggtggcatgcacctggggtcccagcttcttgggaggctgaggtggagggatcacttgagcccaagagtcaggggctgcaatcagctatgattgcacccctgcactccagcccaggcaacaaagcaagactctatctcataaaatattaataaaataatctaaatcaacaccaggcaatgataagggctatgaataaacatgaagctgtgtgtggctagagagtgtcaagtcgctggagaggggtcattcagggaaggcctgaggaaggacctttgagcagaaataacagaatgagcagtgcagattggtagggacaagcattcaggccgagggaacaggcattgcaaaggctctgaggtgagaggatgcctgaggaagtgcagggagccacttgtgcctggaacagagtaaatgagggggagaatgggaggagatgagggtatggaggtgacaagggcaggagccacagagggctccgagcaggggagggacatgactagcttcaggtgttcacaggctccacctggctgcccgtgggagcacactactgggataggacaggagcagggacctctgggaggggcgtgctgatacggtccaggcaggtgacgaaatggaccaggaccggtgtggggcagaggatagggcaaggtgagatcaggctctggaacagttttggaggcagaggcaacagggtttttaacatttggaattctggggaggaaaggattctctgaaagggaagaactcagcaagggctgaccctcctgaaacggggctgtcctgaggctctggacgggcaggcagcattgatgcctgcaccaggcctgacttcctgctctccttgtgcccctcagtctgtgccgacaacaaccacgtgcggacatggtctgtgactcgcttccgcggcatgatttccacccagcccggctccaccccactcgcttcctttaagatcctggctctggagtcggcagatgggcatggcggctgcagtgctggcaatgacattggtgcctactggctcctggccttcccaccccactgacccccttacctgacccctgttgacctccgctgattcccacttgcggccacctgacccaggagcctgcaacgattggggtgtcctgatccttgaggcacctgagctccactgactgccacaaccccccagccctctctggccctgcccaactctaacaacctggggatgggactggggtcttggggtggtgggtttcatcagtggggaaggaagtctgaggctgagggaatcccagctggccctgacccctgcccctgcctggcccaggcccctacggtgagcgggacgaccagcaagtgttcatccagaaggtggtgcccagtgccagccagctcttcgtgcgtctctcatctactgggcagcggtgaggacagtcctgtccaacagggagggaggacagtcctgtccaacagggagggaggtcaggggagaaggcaagatgctagccagatcactgaggccagaaaggggtcccagccaaggagcattgaaggagcaaaggctgggagggaggacaggcctggtaggtttgtcttctggtatcaaaggtgtgacaggtgttggtgggactgacctggcgcagtgccagcccagtgcaggcagggccaggttgaaggcacagggggtggggtcagggtgggatggggggcccaggcggagggggaggggtgggatgggggcccagggggagaggtcggggtgggatggggggaccagggggaggggttggggtgggatagggggaccaggggcaggggtcgggatgggatggaggagacccagggagctgtaggagccttgcttcagctgggaaaggggcctcggaggatgttctggatgaagggactctgagcagagacctagaggacaagtaggaaggagcagaagaaagaaggcaggggaagggggccccagcctgagggaactgtatgtgcagaggctgagaagggccaaatagggtcacatgggaaggacacgtgggctcctgggctggagcacagaacaggaggtgaggatggggtgcagatgcgggcgggccttgtcaggctgtggaagggctgaggctttgtcctgtgcggggagccgtggccactgcatgggggatgaaaggaggcttgatgggaggccaggagcccagggaggaggccaggaggctgataggaggtgggggagcagctgggacgggcctcaggtcttccctgcagtgggagcagggaagagcagaagctctgggagactccctgggtgtttggggctgcggtgtccaagagctgctggacccttgggactggaactcaaaagcaggctagggatggataaagattgggatggcccctggagaggcaggaactgcagccacagtggtggggactgggacgaggaagggtgagaaagcgagggtgaccacctcccccactgcaccccccagggtgtgctccgtgcgctccgtggacggctcacccacgacagccttcacagtgctggagtgcgagggctcccggcggctcggctctcggccccggcgctacctgctcactggccaggccaacggcagcttggccatgtgggacctaaccaccgccatggacggcctcggccaggcccctggtactccctgccccaccccaatcccgtcccaagccccacagcctcacccagaaccactctccactgccaactgcttgatctctctcccaggcccttgccctctgaccccttttcctttgaccccctctctgctccccatcccttcctgcccttgtttttcaacccctgtctcagcctctggcccccatgcattgatctctgcttcctctctcctgtcctgaccctcggtgcttgcactgcaatgcaacccaggcccttgccctatgacccctgtcttgccccctgaccctgcttccgtgccccccagcaggtggcctgacggagcaagagctgatggaacagctggaacactgtgagctggccccgccggctccttcagctccctcatggggctgtctccccagcccctcaccccgcatctccctcaccaggtagccacaactccactgccccttctgtgcaatgaggggagaggggacagcatggtgttcccggggacagagtggcccagctgccccgtgatgacgtgcacttactgtccttacttcctcagcctccactcagcctccagcaacacctccttgtctggccaccgtgggagcccaagccccccgcaggctgaggcccggcgccgtggtgggggcagctttgtggaacgctgccaggaactggtgcggagtgggccagacctccgacggccacccacaccagccccgtggccctccagcggtctcggcactcccctcacacctcccaagatgaagctcaatgaaacttccttttgaacaacgcagctgccatgatgccttgggatgccctggtcctgggggactcaggtgcctccctgattcctgtgggaaccccgggttcagggccagggcctccttggaataaatggttattgttactaggtccccaccttccctcttttctggaagccaaagtcaccctccccaataaagtcctcactgccaacatcttgcttattcttagcaggtttgggactccccaggaaaggggtggggaagatgtgggacccaacccgatatatgcaaaatcaggaacatctacctctcttgtttaagcaaagggaggccaggcatggtggctcacatctataatcctggcactttgggaggccagtttgcttgtgctcagaagtttcagactagcctgggcaacataacaaaaccccatctctacaaaaaaatacaaaaattaagcaggcatggtggtgcatgcctgtggtcccagcttcttgggaggctgaggtgggaggatcgcttgagcctaggaggccaaggctacagtgagccatgatcacaccactgcactccagcctgagtgacagagtgagatcctgtctcaaaaacaaaacaaaacaaaaaaggtgttgcaggggaggaatgtgttggcttttactctgccttcaggcatggctggatccggggcttcaaacactaattcagaatatctttttttcttttttcttttcttttttaaagtctcactctgtcatccaggctggagtgtagtggtatgatctcagctcactgcaacctccacctcccgggttcaagcaatcgcaatcctcctgcatcagcctcccgagtagctgggattacaggtgtgcaccaccatgcccagctaatttttttatttttagtagagacagagtttcaccatattggccaggctggtctcgaactcctgacctcaggtgatctgcccacctcagcctcccaaagtgctgggattacaggcgagagccactgtgtccggcccagaatatctttttatctcctaacttcacttacctctggaatacatcttcaatcaggttttctctctgtggcaaggtgactctaagcagctgcttagcaactctttcttccctagcaacagcaaaaatcacaagactgattttcattggcttgaattaagtcaggtggccattcctgaaccaattactgtggccagtgtgatgaaggccttccattattgcagcctggatcatgtgtcctgctgtatttttagtagaggcagggtttcaccatgttggccaggctggtctcaaactcctgacctcagatgatccacctaactcggcctcccagagtgctgggattacaggcgtgagccacctttcctggctggccttgggattttttttccccaaataatgcccgttcctacggcacttccttgaggagattttctgcatcttttttccttgtgccaataaaaaagggacagaaagtggggacagactaggagtagagaatactagaacatgctaattctagaattccatagtttctggaatgccagagcttctgaaacatagtagagaggggtctcgaacattaggacatctcggacacaaggatattctggagtgctcatggattaacaatattagagttctcccctgcttatcagagaatccagaatatagaagtttctgacaaaaaggacctgaaaaatcactgattctagaataggggagtgtcaaggggagttcatacccatgaatctccaccggtaggaatatcttgcatgccaggatgtctggaatgctgagaattataggatacagaaaggaacctggattactaggaaatctagagaatgggagagatcctggactatccgcccttccagagcactggaaggtttgtttgcgttccaagaaatccataatggcaggagattccggattatcagagaatctggaacacaaatgggagacgtaaaaggtgagtgcctctgaaaccggggtgttctgaaatagctgtgcacctcaaaccctaattttgtttttgtttgtttgtttttgagacagggtcttgctttgttgcccgggctagggtgcagtggtgcaatcatggctcactgcagcctcggccttctgggctcaagtgatcctcctgcctcagcctcctgagtatttgggactacaggtgtgtgccaccacagccagctactttttaagtttttttgtagagacattgtctcactatgttgcccaggctggtctcaaactcctgggctcaagccattctcctgccttagcctcccaaagtgctgggattacaggtgtgagctaccatgcccagcctcacactctagaaaattttttacatgccaggatattcagaatattgggggatattggcatgttaggaaatctagtatgtagggggagggcctggaaggtcaggaaatctagaatatggtggtgttttgtaatgctcacagatctagaatattagagtcatttttttttccaggccggagaatccagaacgctcgtgttgctgaaatgctggtcattctattcttatttcatgtttaaatttttattattttctttatttcttttttttgagacagggtctttctctgttgcccgggttggagtgcagtggtgtgatctcagctcacctcaacctctgcctcccgggttcaagtgatcctcccaccttagcctcttgagtagccgggattacaggcgtgcgccaccatgcctggataatttttgtattcttagtagagacagggtttcactgtgttggccaggctggcctgaaactcctgacctcaagtgatctgccctcccacctcggcctcccaaagtgctgggattacagacgtgagccggccttattctgggggagggggtggggggggagagagagagagggagagagagaggagaatttgggatgttagcaaatctagaacactgaagagctgggttttttaaatgctagagatagtattatcctagtatagtattaactctgtgtgtttttgtgcgtgagagggcatggggggaggggtggaagattctggaatgcggggggactagaactctgagggattctgaagggttgagatgagttaggattcaagaggtgacatagacacgatcctgggagatagtgacactgatgggagggatggggagctggggactccaaattctagggggaggggaggctaacgccggaagttgcagtggtgagccagaggatgttgcctagcaacaagcattgaagatgcgctggatcccggacagaagggagaaatttcagcagcgcccccagcaaatgctccagccacagggtaggaggtggtgaggggggaagcgggtagggatatgctgtcctgcagggtcatgtgagcaggggtcttgggggttatacaaaaacagggtcatggagtacagtcatggggcagagccgggctctgggacagcccacgaatagctgtgaatggagtgtgagtgccgtcgtcacctgccccagggactgtgtgtccctggacggtgctggacccagatttctgggtgtcagtgtgggatggaggcatggattgctgtaggtggcagtaatggtgtgtagccgtgtgagtcagcctgtgtgtctcacagtgagcgggggtgaagggcttccccgtcagtcctgcacaccctcctggattggaagaaggagcaggagtggggggtggggggtgcaactggatcagttgccattcttggtctggggtgggctctgtggtcacggcgtgtggcctagtaccctgtgtgggtggagcctgggatccacgaggtgggggcggggctaacgctacagaactgggaagcttaagaatccaactgctttgggatatggggcctggaaccccaaagcgaagcaaacatgaaaggggtgggcttgggatcctacatgtggtcacgtcccagttttctgtgggaaagggtgtggcctgaaactctggaaaaagaggtgattaggggcagagtgaagctctgagggtggtgccttagggagagaaggggcttgtatttcagagaatatagggtggagccttgaatttataatgatcttctcaaagaattgatcccttctcaaggccctaggcttcaggggttccaggctcaccatctgcaaaagcttgctccccgaagctctgtccctcagtgaacccagccaggctctgcccctgacccacaggatctgctcccagggggtcctgggggctcctggctctgccccctcctgcacctcacttattgccatccccagagggtatcagacccccttccttgcctgagtctttgaatgctcccaagagctttgagtctcaagctgggcttgagaccctgagtttgaaggcttgaagcctggaaccccggtgtggacggggtttaagggcccctgtggcttgcagctcctagtggtggagactcttaggcaaggaagggatcggtactctcttttatatagttttatgtatttatttattattgagatagggtctcactctatcgtccaggctggagtgcagtgcagtgcagtggtgccatctcaactcactgcagcctccacttaccaggctcaagtgatcctcctacctcatcctcccgagtagctgggactactggctcatgccaccatacccggctaatttttggatttttttttttttttttttttttttttttttttgagacagagtcttgctctgtcgcccaggctagagtgcagtggtgtgatcttggctcactgcaacctccacctcctgggttcaaacgattctcctgcctcagcctcccgagtcgctgggattacaggcgcccaccactgcacccagctaatttttgtattttttagtagagatggggtttcaccatcttggccaggctggtctcgaactcctgacctcatgatccacccgcctcggcctcccaaagtgctgggattacaggcatgagccaccgcgcccggcctaatttttggatttttaatagagatggggtcctatgttgtactatgttgctcaggctcacctcaaactcctggactcaagcgatccacctcggccttccaaagtgctgggattacaggcccgcgccagggcacctagccggaactgggaactctctaaggagaaagtctgcaattctgggtggtgggaggctgctcttgggagcattcaaagactcaggcaaggaagggggtctgataccctctgggggcggcgataagtggggtgcaggagggggcagagccaggagcaccctgggagcagagtttgtggatcaggggcagagcctggctgggttcactgagggacagagcttcggggagcaagcttttgcagatggtgagcctggaatccctgaagcccagggtcttgagaagagatcaattctttgagaagatccaatgtgaacttgggaccctcagaggggcaggacctgggggctggtgcagggttggtgctccatttgcagaatcctcagtctctctcgtggaaaggggtacccgtggggggcttccagcttctacgccagcgagggagctaaattctgaccgaattctcccagaactgggagcagagagctgaggactgccagatggagtccagcttaggggaccctgcccccaaccccgctcccgtatccctcccatttttaagcacccctacgcctgggacctctgttccacgagaaggttcacggagccagtatccgagtcctaatttccccccaccgcgtggggaactcgaggtcccccgcgcccctagtccggcacctgtccctgctgcctcctgattggccgcgcggcgagcgctggcggcgccgggctgtgattggcgggaagttcgcagcccgtggctggactgtggagaaagtgagtcggcctcgggcgggggcgggggcgggggcaggggcggggccggggctagcctgacccgctggacagaccgcccgcccggagcgggactcggcgcccgacacgatgccgaggcctggcaccagcggccgccgccccctcctgctggtgctgttgctgccgctcttcgcagccgccacctccgccgccagccccagccccagccccagccaggtcgtcgaggtcccgggggtccccagccgcccggccaggtaagccccctgcttccttgtgccccttccacccaataagtctggtggtccaggaggaccacggctttcggattcaggggaaactcgaacccactgcttcgatgtggagatgcaaagagggcccttggatttattaggcgccctcaatttgtaggggttagattcggggagtactgagatttttaggggaaagagtcccctttattgtggtggagaaggctaagtctccagagaatcctggggttagttcggggaaaggtctctagtttattggggcagggggtggggggctgagctctcctagaatgatagagacgtgtggggtcttcgagctaggatggagcgccccaagtttcttgggcgcgtaaggaggaaaggtgttgggggattctggagggactttatgaggccgctgagttgtcctggttttctaggatttgggggctctgtgttcatgaaaagcgacctttgggtttttcgaattggtcaggaagacatagactcttgcgttgatggtggaggggcttgtggggagtggggtcgggtgggggagtcctcaggcttcagaacggttggggatgctcaagtttcctagaattagaggactctgggattgaatgaggctccagtgatttcaccgcgagagatccaggattccctatagatctgggggctataggcgcccttcctgtctgcgggtgacgggactgaaggaagccgtctgcccagcacccccacccaccctccccgcctggcggcccagcgctccgttacaaaggccccgggctcctctcccgcctgggtctctgcgaatgcgtttagtaacccgagccgcggcgggggcggggccgggaaggggttaacctggagaaaaggcgggagggatgacggcaagatcggggatccccgaggctccccaccagatggcctcatcctccactcggccccacccacctgagaggggcccacgcgctggacacccccctctctgcacccccccactgctctcctctcggggtctgggcgcgcgccctcgtctctagacccccttagcctggggataatggacttgtctggggggccccttcattgcgacgcacttgaaccggagctggaagctccgccactgagaccctctgggctgggagatgtctgcaagaacggcacctttctcctggtcaggcgggaaactgaggcccaaagaccaagaaacgctggcttctggacacacatcgtggaagggcaagaacgggctagaactcaggctctgggattctcagtcctggactgtgactcccgttatccccctccacctcagcaccctgctggacccacagtcagagggaagagccttccctccccagctgccgaggcctgtgaaaatggcgccacctgtcggccaggctcaggatggcgtctgagtcccggaccgggatgtgcgggagggcggggttctagattcccagacagtgcgggcttagaaatgctcttagaaatcgagtcttttgtttttgtttttgttttttaatcacttttaaaaggctttaaaataacgtattttttcaataaaatcgtacgccaaaatctcttcataagacaaaagtacggtttctgtgcccttcagcccgaagtctaagccaatttgcctcccattgtacagatggagaaactgaggcgtggggagaagaacctcgttagtcatatacctgtttcaagccccctcaggatgcgtcttggtttcccctccccgattgccctcctttgcagagttctggggtgctaggggcctgagtgacttccactccactatttatagcgttgctgtttgtcgctgctgcccgggccagacgtctaggaggagccgctgcatccgaggtgggttctggaagatggagtatgagtagggggcaaaagggaataggaggagaggggcagggagctccccatccctcccctcatcccagtgggagagctggatgcatttggtagagaagtacttggtcccctccttccccacttagtccctggctgtctccgaagccttctgcagggtccgaagctgccagcccaaaaagtgtgcaggcccccagcggtgcctgaacccagtgcctgcagtgcccagtcccagccccagcgtgaggaagagacaggtgtccctcaactggcagccactgacgtgagtgggcagtccctcccctaccaaatcctccctcaggaactcctagctttgcccccgtttccgctcctcctcccttcccctctccctctctctcccccctccctccccggctctttcttttgctatcagcctgtctgtccgtttctatttcatcccttgcctgcctatctcaggctcttcccatctctgcattatttctgtctctttctgtttctttctagttacctgtctcttttcctctctctctttctccctgtgtctcactgcctgcctctatgtctaagtctctctgccccttctctctttctctcccccaacccccatcatctctctttctctcagggtctttgtttctctcccactagaggcctggtccccataaataggtgttgtggggggagggttgggcagagccgctactgaaagacattttcctggcatggaggccctttggtggggaggtcagtttaacccggtgacagcagcttttccgtcctctcccacccaggctccaggaggccagagctctactgaagcggcggcggccccgggggccagggggccggggactactgagaaggaggcccccacagcgtgcccccgctggcaaggccccgggtaagcacatccgcctttcctccgcctggggcgaggggggttccgggccagataaagccgtctggttcccacggtccagccgccgcctacccgccccccgttgtagctcagcacccacccccaggacgaggccccctctagggaccccagcgtccggccgtgcgaggtgagcccgggacaggaccagacacaggccagaggcactgacccgcgggggtggggccgggaagccaggcgtccgggctccccgcggccgaagagggagggcgctggcccgttagaaagctccgccgaaccagcccagacaacaaaagcgattgtgcgggttggcgcctgcctgggcaccaaatgctcaagattgtggggcggctgggggccaaaggcctcctcctgtttcccgaatcttccccctgccctcctcccgctccagctcttgacccctagtctagaacacccctcatctcaaacaccctcaaaaccctcctcttgctgtagccttcagcccagatgtgacccctccccctaaagtcttccagatgtgagcctcgggccagatgttagtacccccgcccacagcctccctttatccattgtgacttctcccgccaggtgtggcgttctggccagatgtggctacatcttcacatgtatcccccccacctccagcctcctgcccaggatctagacgcccaattcctttatgtgcccaggtgtagcgacccttctcccatccctcagatgtcccacctggctgtccagatgtaccatgatagccccctatcaagatgaagcccctttctctgtgccccgggcagaagaggatcaactcttagctgtctccccaaatgtggcccccactactcttaatggatttcctctttatggattcagctctgtctggggggaaacccgcccgcccccacctgttcccttccccgccgctcccctacaggcccggtccacttgttggtgcgcggatggggacagagggggcgccccgctcacccctgcgagtctagcgcccagcctgcgagcctctggctaagcgcccagccccacgcgcccccgcgcggccgccggggagggagtggtgaggagggggggcctgagcgggggcgcgggcgacctcccccgcgggcgggcgggcgggtgcggccgggcccctcgggcgggctggggcggcggcgcggcggagcgcggcgctgcagccatggcgggcggcgtgcggctgctctgggtgtcgctattggtgctgctggcgcagctagggccgcagcctggactgggccggctcggagagcgtctccgcgtgcgcttcaccccggtcgtgtgcggcctgcgctgcgtccatgggccgaccggctcccgctgtaccccgacctgcgcgccccgcaacgccaccagcgtggacagcggcgctcccggcggggcggccccggggggacccggcttccgcgcctgtgagtgcggggtggtggtcccgagagagcggctccgggggggaggaggatccctggggatggaggagacagtcctccagggagagggagcccagattccatatgcaatagtgcaagggaatatcaggggctatttgaggaagggggccccaaattcctggcttttggggttgggtcctgagggttccgattttgcaagcaatgagggttcttagaggcctgtgatgtcccacgtgagggaattggcgccagctttcatgctttgcgtcaaaatggggatctcagaattgaggggcctgagaacttttgggaggggggctcgaattctgagacgctgagtaaggagtccccggggaccaagcaagagtctcaggaccgcatgggggacgtctcagtttctgtgtgtttgggtgggaaggttctgtatgggaatgcctgtgaggtggggtactagagagaagaaagttaatccgaagaactaagagggagaggggacagagacgggggttgtgtgtgtgtgtgtgtgtgtgtgtgtgtgtgtgtgtggcggcgggggtggggtgggggtgtctccgcaggacctgagttgcaggggtcccacgtgcgacagaaatccagataagagggcttacggaaggggcgccccctgggggcggaggggacaggaggtgtatgcaccaggcactcctagagatggggagccttgggggttcaggtgaggtgggggagggcgcaccacctgttgttccaggatgcaaaagtgggcagactctctgggatcgggccttcctgccccctaccccgcagaccctatggagtggggagtgggggcccctggagcggagaactcgcccagcctggcccccagccagcccagcccggccggcgtgagctcatctcccgcctgagcccccgcccgctgccactccctctctcctccccttcctccctctttctttcactctttcccggcccagccccaacgtgcctgtgccaggcgccatgcccaggcgggtgccaagcccttgggggtgcaaggagtggcatgtgaagtgggggctgacctcaaagggacccctatgtcctcaactccccgcttggccagggctgtggggcatgacgttggctgtggccatctagtggcccaccctgggtgtaggcacccccagggagctggcctgcgggcctgcattcaggccaagagaaggcagagaaatgcctctggagcctgggaaataccctcagacctggctggtttcccaccccctccatcagagacccttaccattctgcaattttgattcctagttaagcctctcctaggccccactactcaattaaaagcccccattagaccaccctggagtcatggccccacactcctacctaagggagctgagtttttgctccaggccctagacccgctctccaaccatggcaacagactttagagaccactcctccagtgaaattccctctcattcttccctcccacctcccaaactgtgcctttccccagataactctgtagtattgtccagaagtcctgttcttctagctcacccccttccccaggaacttctgatcccatttatcttcagagaaccccagggttggtcttgataagtgggttctcgcaagaggactccagacattgtgctccttacaggcagccattaataaaaagcctttggcacttaatccttagctgggaggggaggggattccacagagggactcggccaattgagcctcttaagtgctgatgacttccaggaattccacttcactatctaaaccctgttttcagcaccgtcaaactggttgtctcctaggcggcactagagtcctgttttctaggtaactgtccacaaaaggactcctgctgaaaggacgcctcagtttcctctgagctaggttcctccatcccagaaacctccagccgtctttgaactcgagaggactgccctttagtcgatctcctcccaggactccagtccctttatccttctaaacggaggtggctctctgcgtcctttcctctctacagttgtggctcagaatcccacacgcgcctcccccggccgcctgcctcctccctcccctccgcacagctgtctccagctgttctctgcagccccgggagagagagggagggggtgccctcgcaggacagcccggcctcctttggctcaaaggtcccggggctccccaagggtccggaatgtggagcctccgccctgcccccgccgcacctctctctttgtttaccccgccgcacagctggcagtgccccgcccagaggtggcctggggcccagcgagggcgcgcagaggggagtggaggcgcgttcccgctcgtggctccgccccggtgctactggaggctgtaaggccgagctagaactctaaagccccagccagaaagaagttgggcggagacacagcgcggtgggcggaactagggcacccggacagcctggaggtggggtgggaggggcgtgaacaagtgagccgggcgaatcagagtgcggaaaggaaggtgggaggggctagaggcagcaggttaagctcctggataggcggggtttagaatcccgcgggtagaaggtaatgtgagaggggctacaaagggggcacagccagggggcggaggtaggacttcgtggaccaagcagagggagtgtgggcgggcatagaatgcgaaggagacagagttgggcggggagttatgccagggagtggttaaaatgtggtttgagtcaatggaagggatcagcattgggtcggaggggctggaacagcaaagggttccgtcggactacggaatgggcggggtcagcgccgtctgggctggtctggaactccgtggactcagccagaaattgggatccgagaggttgacatgaaagtgaataaacagcctgagggctggctgggctcacgcctgtaatcccagcactttgggagactgaggcagaaggattgcctgagcccaggagttcaagaccagcctggccaacatagtgagaccccgcctctaccaaatttttaaaaaacgtagcccgatgtggtgcacgcctgtcgtctcagctacttaggaggctcagatgggaggatcacttcagcttaggaggtcgaggctgcagagccataatcacgctactgcattccagcctgggcaatagagcgagatcctgccgacttagtgggtgggaccgtacctctgatggctgaacaactggactgggccaatgctgatgccagaattggggcggggccacatgacagctaagggcggagcgacttagaaatgaatgataccttgagggagtagggaccccaggagaacctgccaggaatggtggcgcccctgagtgtcctcgttctcctcccagtcctgtgtcccttgatctgtcacaatggcggtgtgtgcgtgaagcctgaccgctgcctctgtcccccggacttcgctggcaagttctgccagttgcactcctcgggcgcccggcccccggccccggctgtaccaggcctcacccgctccgtgtacactatgccactggccaaccaccgcgacgacgagcacggtgaggaaagggtggccagagtcccctccgacccctgtcaagcatttcactttgcccctgaccctcatatttcccgccttcccgagcacctttgcccagctcgccctccccgccttgtctagccccaccccgtaagaacccgtgtagacatccgtttgcccggccgtgcctcccctaggcgtggcatctatggtgagcgtccacgtggagcacccgcaggaggcgtcggtggtggtgcaccaggtggagcgtgtgtctggcccttgggaggaggcggacgctgaggcggtggcgcgggcggaagcggcggcgcgggcggaggcggcagcgccctacacggtgttggcacagagcgcgccgcgggaggacggctactcagatgcctcgggcttcggttactgctttcgggagctgcgcggaggcgaagtgagaggaggcccgtggggaggggcccggagcttgcctccgcgcgggggcgcgctcacccaacacttccccgcagtgcgcgtccccgctgcccgggctccggacgcaggaggtctgctgccgaggggccggcttggcctggggcgttcacgactgtcagctgtgctccgagcgcctgggtaagccccaggacgtccccgaagtgctcggagctggggagtggtgacaacctcaccgttcctcctactctgccctagataaacccagttcacaaattgtagccacgcctaccccattgtggaggcgacttccagtcctgagcttttcataccgctctgggaccacccaccccattttctgactttggccactctgttctcaccctgcctttgtgccttggccccccaccatatactttgggagtctccaatgttgccatttcaactgccaacctaaggctgtccctgcacttaaactacagccaacatcttttagtccctcccaccccgtcttcgtctctgcccactccattctcgctctgcccacctgtccctggcccacccctctcctctcgccacagggaactccgaaagagtgagcgccccagatggaccttgtccaaccggctttgaaagagttaatgggtcctgcgaaggtgcaacggggcaggggtgggaggggcttggttctgggggcgggatttgcagggatcaagttcctgactccacggtgacctccccaaccctggcagatgtggatgagtgcgcgactggcgggcgctgccagcacggcgagtgtgcaaacacgcgcggcgggtacacgtgtgtgtgccccgacggctttctgctcgactcgtcccgcagcagctgcatctgtgagcaaccagcagggagctgaggctgggtcccgccctccctgccctcagaagtcccagagcatcctggggcctttaattccctcggacccccccagactcccgggttcctctgtcagccttagagccccctcagaacttctcagattcttatacagcttcagcatccctggaccacctttagacctttcaagccttttggatccagatccctccagactcccagacttttttttttggagatggagtctcgctctgtcgcccaggctggagtgcagtggcgcgatctcggctcactgcaatctctgcctcctggtttcaagtgattctcctgcctcggcctcccgagtagctagaactacaggcgggcaccaccatgcccggctaaatttttttgtatttttggtagagacagggtttcgccacgttggccaggctggcctcaaacccctggcttcaagtgatctgcccacctcagcctcccaaagtgctgggattacaggcgtaagccactgcgcccagctctcccagactttctggaatccttctcagacccccaaatcctctcgtccccctcaacgactcgactatcttcagatcttgagatccttctcagagtctctcattcaccactgacaccccattgaggctccaagcccttctcagacctccagagcccactgctctccttcagaccctctcagacctctcccaaatgcccctcgcacccaccaaccccccacccccaaccccagaaccattcccctctctcccaaatccctcagtgctacagcattcccagccccgccctgaaggatttcctccctgctcctcgcagcccaacacgtgatctcagaggccaaagggccctgcttccgcgtgctccgcgacggcggctgttcgctgcccattctgcggaacatcactaaacagatctgctgctgcagccgcgtaggcaaggcctggggccggggctgccagctctgcccacccttcggctcaggtgagcccctgcggcagtgcctagccctacgcgcaacacatgtggcgctcattctacgccccaccctccaaccctgagttcactgccccaacctgactggctgggctccagccttggccacgcagcagcctctgagacccgcaggcctcagactggacagcatccatggctccacctccatctgtagccacagccacccctccattcgtagccacagctaccccggagctcccaagttagtttttgtctcctgagcgtcaacgcccagtcccaccctgtccctgaactttgaccaagtccttggcttctgagacactgccttcagcttagccccaccccaggcatgcccctccctgagacacctccctggcattctatcttctgcttaaaactaaatctcacaagggagctatttcctagcctccaactctgtccctgtagacccaaccggaccctgccctcaaccctgttcctaccaccatcccaaatgtgggaaaacgctcttggccccacctgtagcctctaagacattctactctttggccaggacaccaccccatcccagcctccagctcaaacccctgacactctccagccaagccctgcccctagccaaggccagagtctgggctggccatcgttttcttcccgctctcttgtcctctctctgtctctcttacctattcccagagggtttccgggagatctgcccggctggtcctggttaccactactcggcctccgacctccgctacaacaccagacccctgggccaggagccaccccgagtgtcactcagccagcctcgtaccctgccagccacctctcggccatctgcaggtgagctggctctggcagaagtgggtgccatcttcaaggggctgccccagccccatagtgaaaggaggcaagagaggatttgggctccactcgttgataccccttctttatcaggctttctgcccacccatcgcctggagccccggcctgaaccccggcccgatccccggcccggccctgagcttcccttgcccagcatccctgcctggactggtcctgagattcctgaatcaggtttgctagaaagaactgagggcattgggcctgcagcagtggctcacgcctgtaatcccagcattttgggaggctgaggagggtggatcaccaggtcaggagttcgagaccagcctggccaacatggcgaaaccctgtctctactaaaactacaaaaattaactgggcgtggtggcagatgcctgtaatcccagctacttgggaggctgaggcaggagaatcacttgaacccaggaggcagaggttgcagtgagctgagatcgtgccattgcactccagcttgagcgacactccatctcaaaaaaaaaaaaaaaaaaagaattcagggcattgatgggggtattacaggtgggattctggggtaaaagactccaaggtgaagattccaggttacagcaaataggaatggtatgggcagagataagcgtttgaagggttgggtggtagttagatcaggagctggagtcacagttgggctcttctgtgtcaatcgagcaagccatttaacctctgagactcagttttctcattggtaaaatggggatggttgttgagatgcctctgaagtgtctgacacctagtaagtgctcagataaatacttatggtagataattatttttcattatctaatattagataattatttctcaggtagggcactaagaatgtatctcaggcggagggttggagagcaaactattcaaagccagagaccttggggtggcatgatgaggggattcggccaaggatctgatgagaacgttccaggataaaaaagatggagatcagaagaagactgggcttgcttggggaggagacatccatgaaggtgttttatggatgtctccgggggtgggggttttactgggatgaaaggaacggaggattcagagatgggggaaccctggctgactggaccccccaggtccctcctccggcatgtgtcagcgcaacccccaggtctgcggcccaggacgctgcatttcccggcccagcggctacacctgcgcttgcgactctggcttccggctcagcccccagggcacccgatgcattggtgagcaagacggagggcgcggaaggaggcggggcggggggctttgcctggtcaccttgtcaccagccccctccgtgtcctcagatgtggacgaatgtcgccgcgtgcccccgccctgtgctcccgggcgctgcgagaactcaccaggcagcttccgctgcgtgtgcggcccgggcttccgagccggcccacgggctgcggaatgcctgggtgagaaatttgccccacccggctccaggcccaccccagggtctcgctcctgctctcactccagagcctctccagccctcccacgcttcccctctcgggtcccgccccaggactgctctgccctggcccttggccctgcccttccctgacccgcctccacccagctccagcctccctttgaccccacccctacccagctcccaaactgccagtttctatcggggcctggtcgcaactcgtattgctccgcccccacgcccaggccccgcccttattggccacgcccctccctgactaactccctcccccaggccccgccactgtcctgcaactgcggcaaccaatctcctgaccgcgaccccgattccaaccctgccacaccagagccctatccccaaactgctcctttcttctctagcccctaccccaccttcccttagcttggtccccaaagctctcctttctgcccttgcgctaccaaaccctgccctccacaattgcctctctcactgtgcccctctccggctgtcctggccgggtccccatcctggctctggcccaagcttggtcccgctcccgcttccctctacccctgcctccttgcgtcgcttctcccggggctgtctgccccagtcccagccgcctggtctgtgcctacagatgtggacgagtgccaccgcgtgccgccgccgtgtgacctcgggcgctgcgagaacacgccaggcagcttcctgtgcgtgtgccccgccgggtaccaggctgcaccgcacggagccagctgccagggtgagggcctgggaggggcagctgggaaggggtgtgagcggttgggtagagcgcagtgatgagggccagagagactgaacaatagggcaaagcgagttgatttggagacagaggccaggctctcgagcagacgtgtggcctgatggcagtagagagagacctgggatgcagaggccaagtgatgggaaacagaaaggctgagtcatgaaagatggagaagcagaatgaggagggatggagatgtcagtaatcgggtaaggggagcagagttatggaggaaaggggagaaggaggccttctcatggggactacagagacagaaccagccaggcagcttagtagggattggtggaggatgcagagtcagatgatggtgacaaggaggaatagagatggggtcacggggacagaatgttggagggtggaaagccaaagtgacagaggtcagggaggcagaggggaacaagtgaccccgggccccctgccctgtgcagatgtggatgaatgcacccagagcccaggcctgtgtggccgaggggcctgcaagaacctgcctggctctttccgctgtgtttgcccggctggcttccggggctcggcgtgtgaagaggatgtggatgagtgtgcccaggagccgccgccctgtgggcccggccgctgtgacaacacggcaggctcctttcactgtgcctgccctgctggcttccgctcccgagggcccggggccccctgccaaggtgagggtgctgagcccagccctactccatcactgtttgctgtggagactggagagagattattgaggggcagagaggcagagtgatggggctcagggatggagaacaggggctgagggatggggacctcactccagagtcttctctcctttcaacaaaataaggcagtcctccccacccctcctccctttttgaaagatactcttgtgcttatgggaaccctgaggagggggtcacctgaggcagggcaggcaacatggagttggtgccttagcccccaccttagtagctggagagaccattgaatggggacacgaggaaggtgtctgtcttcctgggaagagggagcagcctgaggcaagtccagaaggcaggctcaagactggaatgctggggtgggtggtgatggccatgggaatggattcaggccccttcctcagcctcattggtcccctctgccccagatgtggatgagtgtgcccgaagccccccaccctgcacctacggccggtgtgagaacacagaaggcagcttccagtgtgtctgccccatgggcttccaacccaacactgctggctccgagtgcgagggtgaggccggggagggagggaggagtgtggatgggtgaggggggagttggaccacttcttcaaggccaccctctcccctgccccccagatgtggatgagtgtgagaaccacctcgcatgccctgggcaggagtgtgtgaactcgcccggctccttccagtgcaggacctgtccttctggccaccacctgcaccgtggcagatgcactggtgagaccaggccctggctgtgaccttgggcctgcatcatgacccccgacccttgacccagatcacaactatgacctggccgtaacctcctgacctggacctcagtccctcagtccccagagcctgtgactcctgaccctgacctggaccacaactcttgaccctgaatgtgactcctgagacccaacttgacagtaacatttgaccctaaccatcacccttgatgatagtccctgcccataccctgatagcaattgtgaccctcatgactctggccctgaatgtgacctataactcctgaatttgactgtgacatttgaccctaatcataaccactaaccatagcactgaccataaccttgactgtgtgactcttggtcctatctctttcacagcccctgcctcttctcagaatcccttctctggaacctggttgggttcataatccctgaccctggcccctgacttgaggcagaattctggaccctgactataacttctgatcctaactggattcagattccagtcactaactctgacccatggctcagccgaatcccatccaatgatcctagtttataatacttgactggtcccttgccctagttgatttctgatccctgtctgatccctctcctgactccaaaatcctggcacaggtagttcctagaaacctagacccacaggacttgcaaccatggtccccggaacccgagaaccttggtcagccctacccacctctgccatagagccctcccccagcctccaactcatgagacttcccaccacctcccccagacaccctactccaaggggattggtcgggtgtgtcccgagactggaccctttctgaacacccccaccccccacagatgtggacgaatgcagttcgggtgcccctccctgtggtccccacggccactgcactaacaccgaaggctccttccgctgcagctgcgcgccaggctaccgggcgccgtcgggtcggcccgggccctgcgcaggtgagcagcatagggacccgccagagagtctgggagtagggcctgggttccagggcaaagccggctggaaaggtggaggcgggaccaaggcgctgtgggaggagcttagaaacctggcattggtgggggcggggttactgcgatgtgggcggagcttgtctgggaggccgggtcccgtgactccgcccaatctcccgcgtaccctagacgtgaacgagtgcctggagggcgatttctgcttccctcacggcgagtgcctcaacactgacggctcctttgcctgtacttgtgcccctggctaccgacccggaccccgcggagcctcttgcctcggttcgtacccgggctgatcctggccccggaaagggtgggcttagggcaggaaaaggcgggacggggagaagagggcgaaaaggggaaaacgagtttttagccggggtattccagcaggatcagggggcagctggtgggagtctcgaggcagtgagggggggcggggcgtggagatgaaagggccgagtctgggtatttggaccgtgattgtaaagaagctgttctaaacccgtcggggggcggtgtttgcagggagggaagtagcgtgaggcaggttggggaaggcgtgagaggcctaggagagccgaggggcggtggaggggtgtggcctagaatgttaggcggagcgggaggtgggccgggccttcggacgccctgtcccgcagacgttgacgagtgcagcgaggaggacctttgccagagcggcatctgtaccaacaccgacggctccttcgagtgcatctgtcctccgggacaccgcgctggcccggacctcgcctcctgcctcggtgagaggccccgccccggcctgatccctcctcccttcgactccccgactcgccgattggcctcccacctctgtctttcctcctccgcttctcccctccccttacctctttcccccgcctcctctcctagcctccccaactctcctctaccccaatcttctcctgccctctcctctgcttccccggcctcccccttctgactctcctctcccctctttgtatcccccatcttgcctccctgcttcccacatccgaccacccgacctctctcctcagacgtggacgaatgtcgcgagcgaggcccagccctgtgcgggtcgcagcgctgtgagaactctcccggctcctaccgctgtgtccgggactgcgatcctgggtaccacgcgggccccgagggcacctgtgacggtgagcctgcccccacccgccttcgctagcgcttgcaacgcggtgctggaggctgctcccttggggactgaggaggggcgccctgcttcccagacttaggcggagggaaagaacaccctctcaccgtatctctgtagtggaaataagccgccaccgtgtccatgtattttcttgtgtcaggatcacggccaagcctcccttccagccgcagtccattccccctctgcagctgaagcccggtccacattttaggctatgcccccagtaagacaccgccccaaaactgttaggccccgccccttccaatcggcctctggattaaaaccccctcttcaggccccttctcttcctaacagaagtttggacgtgccctttccgcgccctccaccagtcctacttccagccttccctccaaagaggcccaatcccggtggccctaggccccattctttcccaatgagaaattcccaaggtgaaattctcctagcattggcccccgcccgtttaagctctgcccttccttggtctctctagacagggctttccattcgctcggatggctccagtctctcgaacacttaggccctcccttcctatctttgctccgcccacagacccgccccttgccttttcttactttccaggccttccctcccgccccgctctttcacccctcccgggtcaggctccagcgaggcaggagggtggggctaatcttccatacagtatatatttttttgtgtcggcgggggggggggggcggtgatggtgtgtgagtccgcatcttgtggaacacatgaaacaaaacatctgtgggctgccgttgactctgctagacctctgactcatggaaatctagcttcataagatctcattcattaattccacaagaattcactaagcacctactctatgccagcgtctggaaaaggtaataagagcaacaggaaataagtcatataaaaacccctgccttcctggagttattgtggggtaataaatatgtaaataaattcaagatttatacagcaggccaggagctgtggctcatgcctgtaatcccagcactttgggaggccaaggcggatggatcacgaggtcaggagatcgagactagcctggccaacatggtgaaaccccgtctctactaaaaatacaaaaattagctgggcatggtggcatgcgcctgtagtcccagctactcaggagactgaggcaggatactcgcttgaacccgggaggcggaggtggcagttgagccgagatcgcgccactgcactgcagcctcggcgacagagtgagattgtctcaaaaaaaaaatttatacaacaaaaaactggggggcaccttactatatgttgggcactggagatgtagcaaggaacaaaatagacacaaatccctgctattgtagagtttgtattctagagaggcgacagttggcataccaataaatacatacgtataacatcaggtttaggaaggaaaacaaagcaagacaaatgggacagagatgacagagcagtggatggaggagtgctaggagggcttgacctagacaccagacagaagcgagggaggcagccatgcagagagctgaggggagactgttcctggcagagggaagagccagtgcaaaggctctgaggcaggaccatgcttttgagaaatggcagtgaggacttgagagttatcaactatgctaggtgtggtggcacaagcttgtaatcccagctactcaggaggctaaggtgggagaactgcctgaacccgggaggttgaagctccagtgagccatgatcctgtcactacactccagcctgagcaacagagcaagaccccatttaaaaaaaagaaaaaaaagctggatggggtggctcatgcctataatcccagcactttggaaggctgaggcagctagattgcctgaggtcagaagttcatcaccagcctggccaatatgatgaaaccccatctctactaaagaaaaaaaaaaaagatagtggctgggcgtggtggctcacacctgtaatcctaggacttgaggaggccgaggtggacagatcgcttgaggtcaggagttcgagaccattctggtcaacatggtgaaatctcatctctactaaaaatacaaaaattagctaggcatgatggtgcatgcctgtagtcccagctgctctagaagctgaggtagaattgcttgaacctaggaggcaaaagttgcagtgagctgagattgagccactgcactccagcctgagtgaaagagcgagactccgtctcaaagaaaaaacaaagttttcaacattgttgatcttcagaagctcaggctcctagaataccagattgctaaagacttcttagtcttgggcaccggaagtggtgttagaacttctgaattcaggcctttgactcccctttcatctcctccacactctgcagatgtggatgagtgccaagaatatggtcccgagatttgtggagcccagcgttgtgagaacacccctggctcctaccgctgcacaccagcctgtgaccctggctatcagcccacgccagggggcggatgccagggtgggtgtccatcaggcatcgggtgagatgtggagatggtagaaggtccagaaatggcctgactgtctggtggttgcagatgtggacgaatgccggaaccggtccttctgcggtgcccacgccgtgtgccagaacctgcccggctccttccagtgcctctgtgaccaggttacgagggggcacgggatgggcgtcactgcgtgggtacgggacttcaggaggtggatgggaccaaagggggtgggggaggttggtcaggccctgtccctccccatatatctgaacaaatgggaattttcgggttgtggaatttagactttggaatataagatcatcttcatgccaggcacggtggctcacgcctgtaatcccagtactttgggaggccgaggcgggcagatcacttgaagtcaggagtttgaaaccagcctggtcaacatggtgaaaccccgtctctactaaaaatacaaaaattagccggatctggtggcaaatgcctgtaatcccagctactcaggaagctgaggcacaagaattgcctgaacccaagaggtggaggttgcagtgagccaagattgtgcaattgcactccagcctgggtgacagagtgagaccctgtctcaaaaaaaaaaaaaaaaaaaaaaaaatcagaactgttgtagtggctggtgacagaaacctgacttaatcaggttttatttttgtgtgtgttcttttaaaaatgtataaagtataaatgtataaagtactaatcttaagtgttcataaacattaatctttcctaacattttatgaggaaaatttctaaacacaaagcaaattgagagaatcatagaatgaacacctacctactcatgatctagattatattatcattttattacacttgcttcctcacatatctatccattaatccatctaattttttggacagagttaaaagtaaattgcaggcaccagtctgcttccccataaattcttcaatatgcatatcactaaccagaattcaatatgtgtttaccaatgtattcttctcttctctcttttttttttttactttgaggtggggtcttgctctgttgcccaggctggagtgtggttgtttgatcatagcttactgcagcctctaactcctgggctcaagccatcctccctccagaactgagcttccgagtagctgctaccacaggcacacgcaaccacgcccagctaatgtttttaatttttgtagagatgagttttttttttttttttggagacagagttttgctctagttgtccaggctggagtgcaatggcatgatcttggctcactgcaacctccacctcccgggttcaagcaattctcctgcctcagcctcccaagtagctgagattacaggtgcccaccactatgcccagctaattttttgtactttgagtagagatggagttttgccatgttggccaggctggtcttgaactcctgaccttaggtgatccgcccaccgtggcctcctaaagtgctgggattataagcatgagccaccacgcctggcctgtagagatgagttattgctctgttgcccagactggtctcaaactcctggctttaagcaaccctccctccttggcctcccaaagcactgggattacaggcatgagccattgtaccctacagatattttcattcaacgttcaatttatatacagtgaaatgcagcaatcttaattatacattctgtaaattttcacaaatgcaaacacaacaggttttatttctttaaagggaattaaaactataaagtcttgggatatatttgaactccaggcataactggatccaggaattttaacaaggctatttctatcttctctgagttctgctttcttctattgcatgattttcaggcagattatttttcacaatgatgaaggtggccctagaacctctgggctaacatctccagtgggccacccgagagctaaaaagggaggtttttttttcaatatttctagcaaaagcgccaggcctggctttgattgacccagcatgatcactgcctatgtctgaaccagagaaatgccgtcatctgtttggtcattcctggaacttgtgcccacctctcagagtagatatagccctactcaaagaacaggattgaaaatagaggagcacagggttcccaagggaaattcaaggtttctcactagaagaaaaacagatgatgggatctgggccattaaatatacacattatatttgaaagctgagactttcggacctttggaatcatagaagcttataaccactgagtccctctcccctgttgtctcctgcttacagatgtgaacgagtgtgaaacactacagggtgtatgtggagctgccctgtgtgaaaatgtcgaaggctccttcctctgtgtctgccccaacagcccggaagagtttgaccccatgactggacgctgtgttcccccacgaacttctgctggtgagactgatgtgtctatttaactgatggcggctggccccatgggaaaatcacgtggtctaatcattcctgatgtggacagctaccatcagctaaatactgttgttttaaacatcaacaaaagacacataagttaacatgggtagtgagactgtgtcaggagaattagaccctggtcctgactctaccagattctttcattcaacaaatgttcacagggtgtgcactgtgttcaggccatcttctgggcactgagaacatagtagtgaccagaagggatcactgtctgtcctcaaggggctcacaagccaatggggcagacagagatatcaccagatagtgacaacccagagaaatcaacaagactgtgacggggaaagcccaggggggttttggaggaggcgcctggcccagcatgagaagaggattagggagttcttcctgtaggagacgacatctgaactgagagctgtgggatgaatagaaatgagccaggcccgatgagtgaggagggcattctgggcagaggacacagcaagggcaaaggcctggcaaagccagagagcatctggcatgtgagaagaactgaaacaggttcaacatggcatgatttagagagcaaaggaaggggtagggagagatggggccagggaaagagtcaggtgcccgatcacactgacttatcacagtaagagagcactgcggtaccgtggaaggggtttcggcgttttttttttgaaaattttttttaaatgttttttttttaagacagggtcgtactttcacccaggccggagtgcagtggcgtgatctcagctcactgcaacctccacctcctgtgctcaaggaatcctccaacctcagcctgctgagtaactgggactacaggcacatatcaccacaacagctaatttttgtattttttgtagagatgtggttttgtcatgttgcccaggctgcagtatttttttttttttaatttttaaatgttacatatttaggctaggattggtggctgaaggccataatcccagctctctgggaggccaaggcgggaggatcacctgaggtcaggagttcgagaccagcatggccaacatggcaaaaccctgtctctactaaaaatacaaaaattagctgggtgtagtggtgcacgcctgtaatcccagctattcgaaaggctgaggcaggaaaatcgcttgaatccaggaggcggaggttgtgggattgcaccactgcactccagcctgggtgagagaggaagactccgtcccaaaaaaaaaaaaaaaaaaaaagctatgtatttatttatttttaataatttccatctttactttagattcaggggatacatgtgcaggctttttacctgggtatatttcgtgatgctgagctttgggatacaaatgatcccgtcacccagatagtaagcacagtacccaacagccagtttttttttttctttgagacggagttttgctcttgttgcccaggctagagtgcagtggcgtgatctcagctcactgtaacctccacctccctggttcaagtgattctcctgcctcagcctcctgagtagctgggattacaggtgtccgccaccacgcccagctaattttttgtatttttagtacagacggggtttcatcatattggtcaggctggtctcgaactcctgacctcaggtcatccacctgcctcggcttcccaaagtgcagggattacaggcgtgagccaccatgctcggcccaacagccagtttttcaacccttgtacctctgtccctcccccatctagtggtccccagcaactattgtgggcatctttacatccatgagtacccactgtttagctctcacttgtaagtgagaacatgtggtatttggtcttctgtttctgcattaatttgcttaggataatggcctccagctgcatccatgttgctgctaaggacatgatttcattctttttcatggctgtgtagtattcatggaagggttctaagcaggaaagatagaatcagattttgaaacctccctctggccgccatgtgaaggtgattgaagcgggtgatatggaggctgggagctcagggaacaggctggggcaggggcctggacaggagagaacagggctggaccaaggcaggggctgtggaaggggaggagaaggtggtgggagaaaaacccaagaggccatgtggacaagctgtggatgtctgggtggggaagctgtgtccaagacaaggcataggttttttgtttgtttgttttgtgacagagtctcgctctgtcgcccaggctagaatgcagtggtgtgatctcggctcactgcaacttccgctcccgggttcaagcgattctcctgcctcagcctcccaagtagctgggattacaggcatgcgccaccacacccggctaattttttctatttttagtagagaccgggtttcaccatgttggtcaggctggtctcgaactcctgacctcaagtaatccaaccgcgtcggcctcctgaagtgctgggaggacaggcaggagccactgcacctggcgacaaattgtaggttttgagatgaagactcagccagtttgccacacactggataagagacccagagaggcatccaggaagccagggaagttccctcaccacccacccaagctgttagctgcagtgacgggaaagtgtgaggtggggaggcaagagatgcagaaatgacaggaggtgacagtgggagaaagagaaacagtgacagaggagcgtgagaggtgtggagtctggttctgccactgatggctgccaccctctgtttccctatctatgccagcctcagtttccccatctatgatagtggcggggctggggattcagcccacactgggctaaagctccttgtctccccaggcacgttcccaggctcgcagccccaggcacctgctagccccgttctgcccgccaggccacctccgccacccctgccccgccgacccagcacacctaggcagggccctgtggggagtgggcgccgggagtgctactttgacacagcggccccggatgcatgtgacaacatcctggctcggaatgtgacatggcaggagtgctgctgtactgtgggtgagggctggggcagcggctgccgcatccagcagtgcccgggcaccgagacaggtgggcatgggctgatggggacacagggctgagggcttgggtggaaatactgggtggggtgtgggcctgggacaggggacacttttggacagggccttgaggtactagtactgtcagggcaagggcgagctgccaggcaggtgggcatgggcagacataaggctgagaggtgggcactaacaggcacagggccagagggacttttgtgacaagtgggcacgagcaggtcagggctggggctggggctctggtgtcctggctcaggcttgtctctgtgtgtagctgagtaccagtcattgtgccctcacggccggggctacctggcgcccagtggagacctgagcctccggagaggtgaggccagcctttgaccctccaccccactcagctctgaggcccagcttcgtctcttcctgttttctttgcctctgtctctcaccctttctgtttctctgtatctgtctccccgaccccacccatactctgtctctttctttcttttctttcttttttttttttttcttaagatagagttttgttcttgtcgcccaggctggagagcaatggcgagatcttggctcactgcaacctttgtctcctgggttcaagcgattctcttgcctcagcctctggcgtagctggctacagacactagccactacgcctggctaatttttttgtatttttagtagagacagggtttcaccatgttggccagattggtctcgaactcctgacctcaagtgatccgcccaccttagcctcctgaagtgctgggatttcaggcatgagccaccgctcctggcctctccatctttctttccctgtctctacttcttggtctatcaccagctctgtctctgtcttcccacgtcatgccctcacacactccacccatccagcccgcccccatctctctctctgcttttcgcacagacgtggacgaatgtcagctcttccgagaccaggtgtgcaagagtggcgtgtgtgtgaacacggccccgggctactcatgctattgcagcaacggctactactaccacacacagcggctggagtgcatcggtacaagccccacctcccccaacccccggcaactctctccaacccctagccttgccagctcccctctggaatgtggccaccaccagcgggaagtctttcctggagtctagactccatccatcacactgccaatgtgctgggaagagaaatgggaaagggtggggagagttgaaggggatgcctcttaatcatcctctccctagacaatgacgagtgcgccgatgaggaaccggcctgtgagggcggccgctgtgtcaacactgtgggctcttatcactgtacctgcgagcccccactggtgctggatggctcgcagcgccgctgcgtctccaacgagagccagagcctcggtaaccccgcccacgccatccaggccctccttcccttggctcggcctcacacccgcacccgggccacacctttgcgacggccacgccctccgaaggccacgccccatgctcctggctcgaccacgccccactgagccctcactcagtctctgtcccactgtctgtctctctgaggcgagctggctaggtggttaaaggcaaaagttttagggcaacctttgcatgttgcctcttggactccaggtttctttctgcacactgggtgaatagcccctaccttatagggtggctgtgaggaattttatttaattttatttatttattttttgagacggagtttcgctcttgttgcccaggctagagcgcagtggcgccatctcagctcactgcaacctccacctccggggttcaaacgattctcctgcctcaggctcccgagtagctgggattacaggcatgtgctaccacgcccagctaattttgtatttttttctttagtagagacagggtttctccatgttggtcaggctggtctcgaactcccgacctcaggtgatccgcctgccttggcctcccaaagtgctaggattacaggtgtgagccaccacacctggctgatgaattttattttattttattttatttttaatttttaatttttagttttattatttattttttactaagtaccacatgagtgctgcctgttattatttatctgcatctctaggtctctgtctctttccagctgtttgtggatttctgtctttggggttttctctgaatttctgacaccctctggatctttgttttcaggtccctttctcctgcctctgtatctttgttttcctgttttgagtctttgactctttggatgtgtttctctctctctctttgggtcttttttctcccttttcgtttctgactattttcctatctctaggcccctaacaacttctgctgaagctctgtctcttgaacactctacttgtcgttgtttgttttcatttttgagacaagatctcgctctgtcatccaagctgaagtacagtggcacaatcacagctcactgcagcttccacctctcatgcccaaatgatcctcccacctcagacttgcagtagctgggagtccaggagcccgccaccaagcctggctaatttttgtatttatatatatatatatatatatatatatatatatatatatatatatatatatatatatatatatatttttttttttaaagatgggtttttgccatgttgcccaggctggtcttgaactcatgggctcaagcaacccccccacctcagcctcccaaagtgctgggattacaggctccaacacactctctctgtgcttcttgccacctctctttttgcccactgtcccaaccactcttctctcatttcctgtgccttcagcacttacccccatacagtgagatgtcagacaatgctcagagaagcaaagcaactgccccgaggccacacagccctccagaggccagacttgggtagacccctctcaggccctacctcccagtcattggacaccttcttctgccctctcctcctatatgacagtctccttgttcctcaatccagaaccctggagtgacctcagagaacttccagagttagatcacagctgatgagaaggatttgctgataggcagagggtgcctgggctgctcagcaggggaagggtccagcccctgggaggacctgagtgccaggcccactctgacacatgctgtctccacctacagatgacaatctgggagtgtgctggcaggaagtgggggctgacctcgtgtgcagccaccctcggctggaccgtcaggccacctacacagagtgctgctgcctgtatggagaggcctggggcatggactgcgccctctgccctgcgcaggactcaggtgctggcactggcctaggctgaactcagaggccttgccccatgggctccaaatctaggccctcagatccccagtcgcagaacccccagactctatccaaactctgtcccctagaccaacccctatgtcgcagcccatcccaaaatcttggtccccgattcacactccaaagacttccaagtctcagccacagacatcccaaggcctgacccagcagatcccatagtaccagacccacaggcccctgaggtctggtctctcatatgctcagctcctggtctctagaaccaccagacacagcctatgagatgtcctcccctaaatcctgggcccttagacctgaaatgccagttgctcagacctcaccatcctggccccagaccccctggtcacagccccacagacctccaagtcccattgccttagacaccctccaagtcccattgccttacacaccacatccgggtgcctaagaccccaacacacagccccagagattcccaagtcttggtttctacaacctctgagtccctcagtcctcagcccttaggaacccagttccaaagccccagtcctgggtcctcagacctccaggtcccagtgcctcagactgtctcccatgcatcctgccccctcaggtccccagcagcaatccctgggattccccagtcctggtccacagaacacccccatctaatttcttcaggtccctagtcctagctcccatgggtcgctccaattccagcctctcagaccctgattcttagcaggcttcattacccttgatctcagcacgtccgaatcccagtctcagccttcagattctcagcgctggctccagaaaccccggggccacccaggaccctccccatccagtcctctgcctcctctcccaaggggggtatgtgagtggtgggtgtgggggccagcaggggctgattgtttgccttggctcctgttcccagatgacttcgaggccctgtgcaatgtgctacgcccccccgcatatagccccccgcgaccaggtggctttggactcccctacgagtacggcccagacttaggtccaccttaccagggcctcccatatgggcctgagttgtacccaccacctgcgctaccctacgacccctacccaccgccacctgggcccttcgcccgccgggaggctccttatggggcaccccgcttcgacatgccagactttgaggacgatggtggcccctatggcgaatctgaggctcctgcgccacctggcccgggcacccgctggccctatcggtcccgggacacccgccgctccttcccagagcccgaggagcctcctgaaggtggaagctatgctggtgagcactgccagcgcatgatgagactgagatgaggggtgaggtgtgcacggagagaggagggagggaaacagaaggcgggaggagagacggaacacaggtgcaactggagagagccacagaaagggacagagaagtgtctatagcccggcaaagaaagagaaggtggcagagggaaagctggcgagagaatgaggtaagcttactggccccgcagcacccgccacagccctggagcgggatggacagtttacagcgagaaagatggagccaaggacgcgcacccaccgttgtgggtaaggggtgaaggcagggacctcaagtcatagggtccccgcatttcccacaggttccctggctgagccctacgaggagctggaggcggaggagtgcgggatcctggacggctgcaccaacggccgctgcgtgcgcgtccccgaaggcttcacctgccgttgcttcgacggctaccgcctggacatgacccgcatggcctgcgttggtgagggcgggcccggggccagcatgcgcagggagaggcgaggcttgtccagggagggtggaagccctgactagggggtgctggtcagggacgggaaaggacctcactacaggggacgggccagcgcaaaagggaggagtaattcttccacctgggtggggcttgactgaagaaggcggagtcagggtgccagcagggcagggcttaaccacggggctggagccgggccttgaagcaggatagaggaatagaatagtgctggtgtgacttgcagtgctaccttgggcagtctgcaggacctctttggagagcctcagtcttcccacctgtaaaatgggaatattaatcaagtctgcctaatttggatggcagtaaagccaagtgattaaaatcaagaacatagccgggcgcagtggctcacgcctgtaatcccagcactttgggaggccgaggcgggcggatcattaggtcaggagtttgagaccagcctggccaatatggtgaaaccccgtctctaaaaatacaaaattagccgggtgtggtggtgcatgcgtgtaatcccagctactcgggaggaacccaggaggcagaggttgtggtgagccaagatcgcgccattgcactccagcctgggcaataagagcaaaactccgtctcaaaaaacaaacaaaactcgaggaggtcacatagacctcagactcagtccagcaacttgctgtgtgacgctggacaggtcactgtcccttacctaatttttctgatatgaaaaatggctacagtcaaagatcccatttcatagaattgcgaatattattaacactgatttacaataacattgagagtcatgtgcaaatggaggcacatgcgtaaaacgaattacagtacctacctaataggggtattagaaggacaaagttaatacttgtaatgtgcttaaaacaatgcatgaacatttattgttgttgacaccatcatcagtatttttttcttcttttttttttcttttcttggcgacagagactcactctgtcgcccaggctggagtgcagtggcctgatctcggctcacagcaacctcctcctcccaggttcaagcgattctcctgcctcagcctctcgagtagctgggattacaggcgcccgccaccatgcctggctaatttttgtattcttagtagagacggggtctcaccatgttggccaggttcgtctcgaactccggcctcaagtgatccacccgcctcagcctcccaaagtgctgagattacaggcatgagccaccgcgcccggccattattattttcttaacaaaatcctagtgcggtatgggccaccatatccatcttacagaacacgaaactgaagcacagtgaggttaagccacctggccgggctcacacagttagcagatggcagaggccagattggactccaaactgctcagcatctgtgctcctctgttccaagaacttaaggggccaaggaggcgagcttctggggccccagccttcagcagcgatcgttgtctcccctccgcagacatcaacgagtgtgatgaggccgaggctgcctccccgctgtgcgtcaacgcgcgttgcctcaacacggatggctccttccgctgcatctgccgcccgggattcgcacccacgcaccagccgcaccactgtgcgcccgcacggccccgggcctgagccctggcacccgctggccgcccacccgcgcccgccactcggggcccctgccgcgcatcctgcagcccgcttatgcgtatgtgcacggggccgcccgcctggacctggagaagggacctacggacgcctggaagctgcgacgccctgcactgctcccgcctccaccagcgcctcccactgatgtcgtggtcccgggcctggcccaggggcccctttacatgccctctcccttttataaaattttccattaaaaaccacctattttctatcttttgcctcctcctgtctatttctccaagtctaccccagtttgtgctttgagtcactaaatgacattcccttcccttctgacccctagtttcgtctgtctctctgcctctcttggtctctgtcttccttctctctctgtctctgtcgttctatctcatctctgtctctttctgatttgttttctctgcctaacctctacatcctgtcttttcatttctgtttctgcatgcgtctttctcttttcccttctctttgtttggttctttcatctcgagagcaatcttgcctctggattttttttttttttttttttttttttttgagatggagtctcactctgtcacccaggctggagtgcactggcgccatctccatccactgcaacctctgcctcccggtttcaagcgattctcctgccttagcctcccaaggagccgggattacaggtgcacactacaacccaggctaatttttgtatttttagtagagacggagtttcgccatgttggccaggctggtctcaaactcctggcttcaggtgatccacccaccttggcctcccaaagtgctgggattacaggtgtgagccaccgcacccagcttttattttttagagatgaggtctccctatgttgcccagtctggtctcaaattcctgggctcaagtgatcctcccacctcggcctcccaaagtgctgagattatagatgtgagccaccgtgcttggcctagaagtcttaagctgtcctggaacaagtggggcaagagcagggagcaggagtccctggagggccaaacccagacctgacgctccagctaggagttggctgtggatggagtatggagcggcagtcctgacagctggaggcgggaatgagctctgtgtgtgatggtggagtgcccagcacggacctcctccatgtgccctgcctgcttactggccatgttcctagtccagactcctcctccctaaaaaacaagaacggcctagatcagcataaacttagggcaggagtaggggtcgggaatcgtgggtgatcaacttggcactgggccaagctgggaaaaaaaaaaaaaatgtacctcagccaggcgcgatggctcacacatgtaatcccagcgctttgggaggcccaggcaggcggatcacgaggtcaagagatcaagaccatcctggccaacatggtgaaacctggtctcaactaaaaatataaaaattagcccgccatggtggcatgcaactgtaatcccagctatttaggaggcggagataggagaatcacttaaacccaggaggcagaggttgcagtgagccgagatgacgccactgcactccagtctggcgacagagccagactgcatctcaaaaacaaaaacccacaaaactgtacctgtcattcttcacccacctgtcaattcttgtgtccccagggtttcaaactcatatgctgcaaagaccagaaccggaatgttagcaggaagcagggaaaattgaggcacacattaccttctgcctaaggcttggttagactaggaaggggaattttccccattgttaatacttttttttggcctggcggggtggctcacgattgtaatcccagcacttcgggaggccaaggcaggatgatcacttgagctcgggagtttgagaccagcctggcaacatagtgagaccccatctctacaaaaaagtagctgggtgcgatggtacatgcctgtagtcccaactacttgggaggctgaggtgggatgattgcttgagcccaggaggtcgagactgcagtgagctgtgatcgtgcctctgcattccagcctgggtgacaaaggcataccttgtctccaaaaaagttttttttaatgtatatttttaataactatctgatattgtttggctgtgtccccacccaaatctcatctcaaattgtaatcagaattgtaatccggggaaggacctggtgggaggtgattggatcatggggacagtttcccccatgctgttatcgtgatagtgagtgagttctcacaagatctgatggttttataaggggctcttctcccttggctcgctgtctctcctgccgccttgtgaagaaggtgactgcttcccctttgccttctgccatgattgtaagtttctgaggcctccctagccatgcagaactgtgaatcaagtaaacctctttcctttataaattacccagtcttgggtggtatctttatggcagagtaagaatggaccaatagggccgggcacggtggctcatgcctgcaatcccagcactttgggaggctgaaacaggtggatcacctgaggtctggagttcaagagcagcctggccaacatggtgaaaccccatctctactaaaaatacaaaaattagcagagcatggtggtggatgcctgtaatactacctactcgggaggctgaggcaggagaatcgcttgaacccaggagccggaggttgcagtgagctgagattgggccactgcactccagcctgggtgacagagcaagactctgtctcaaaaaaaccaaaaacaaacagaaaaagactaatatagtaccctatggggcctatttggcctatgaggctccagttttaatcctctaggcactgctgaaattgcataaattgtggattggaggctgcttcctgacctgatctccagcccacccgctgagtgtcaggaggggtcacatgcccagcagcctcctgtgctacatcggggaatcatactaagagcgcctaccctgcaggattggtggtggtggttaaatgaattgtcatatatgtgcttagaatgtcacctggtacagagcaagggctcagtcattgttggcataaccctgggcctcccaggatatgctgagccctgtggctgggcagatagtaaggtcttgttcttttctcttttcctttccttcttccttttcttttctttctttctttctttcttttttttttttgacatagggtcttgctctgttgcccaggttggagtgcagtggtgccaccatggctcactgcagcctcaacctcccaggctcaagtgatcctcccacctcagcctctcaattagctggaactgcaggcatgtgccaccatgctcagctaattttttaatttttattttttgtagagaggggaccttactgtgttgcacaagctgatctcaaactcctgggctaaagtgattctcctgcactttggcctgccaaagtgctgggattacatgtatgacccacggcacctggcctggctaggtctttttctttaccaattctccctcccagggtggaggaggaggccagaccccatccccttcaacaggacagtgagaaacacctaacacaaggccttggtggggaggagtgtcagacaaggagtggctcaaggctccacaaaggggtgacagttgcacaaaactgtctgtaccaaaaatcattgaattatacactacacatgggtgacttgtgtggtatgtgaatcataagtcaataaagcccttctttaaaaacgccgactctacaaagcgtttcagaaagttaccctccagctgatacagggaacccgacccaaccactaattcctcagtcattcattcaacaaatattttcctgctttgcaataagtgaattcgaggaacacaaactttaacccagccttggggggtggttagggagggctcctggaggaggagatgttggagctgagagttgattactgtagggaaatgagcaagatgaaaggggtggaggtgcctataatcccagctactccggaggctgaggcaggagaatctcttgaacccgggaggcagaggttgcagtgagccaggattgcaccgctgcactccagcctgggcaacagagtgagactctgtcagaaagaaagagagagagagagaggaaggaaggaaggaaagaaggaaggaaaagaaagaaagaaagaaagaaagaaagaaagaaagaaagaaagaaagaaagaaagagaaagaaagaaagaaagagagagaaaaagaaaagagaaagaggtggagaaccatgttccaggtggaggggacagcacttccgaaggcctagaagtaagagagcaagtgtctgttagatgtctttcctttggtatctaaggcctgtattggacaacaatggtgacaatcttggtgcctgagaaatcccaggcccttgccttcatgggggacaccgacacatcaccacacatgagagcctgtgctgtatgggggaggcacaggcaggggtcaggctgcggtgggggaagatcagagggcatgcatgcccagaggagacacttgatccagtctgagagatgatcagggaaggctttctggagaaagagacaaagctctgaacagtctctgtttgggcgtctagatccctttgagaatctgtcgaaagctcattcacagaagaaaaactcacacaaacaaaggttgcaggcaatttccaagtattctcatccttcctcggaatcttctgtgggtatcccattcccaccccgcccccacaaccaccttgctgcataaatgtcccaggaattgcgacagggctggccaacagtgctggaaaactgcaatcgaatttcagcatcctgggagtgggatctttcttctgagatctcgcccgccgccgggcctggagggtgtgccccatggatctaattgttatcctgcctgcatcccctgcactaacccccagacctggcgttggggcttctggcactggccgggaccgacgcgttctcctctggaatgttcagagggaggtagtccaggcggtcaccgcgctcgccagacaagcaacgcagcgccccccgatggccaccgcgcgccggcgcagcccaagccggctgcgccccctagtggccgatgctcgtaaagtcttcagcgagccccgagcttttgctagccagcccttggttttgcaggctggggtcatcgtcgttgtcatcgttggcatcatcatcatcatcatcatcatcatcatcatcatcaatagctagtaggcttggcgtggtggcccacacctgtaatcctagcactttgggaggccgaggcaggtggatcacttgaggccagaagttcgagaccagcctggccaacatggtgaaaccccgtctctacaaaacagtacaaaaaagcaaccgggtgtggtggtgggcacctgtaatcccagctactcgggaggctgaggcatgagaatagcttgaacctggaaggcggaggttacagtgaactgagatcgaaccactgcactccagcctgggcaacagagtgagactctgtctcaaaaaaaaaaaaaaaaaaaaagctatgatcatccaggcagtgattcatgcctgtaaccgcagggctttgggaggccaaggcaggaggatgtcatgaggccatgagttctagactaacctgggcgacagagcaagagctgtctctataaaacaaaacaaaatgctatagaccagacgcagtagctcacacctataatcccagtgctttgggaggccaaggcaggcggatcacctgaggtcaggagttcgagaccagcctggccaacatggtgaaaccccatctctacactttgaaaaccactactttaactgtctctcccacagggagagctgcctccttcactctcagctcatttggttcacatgttgaccctactggaagactccagacctggccagtgagagaatcccttcccttcagcctttgcaactggcttagggacaggtgtgtccctgaagctggactgatgagcattggctctggaactactgctgattgttgaagaaggggcttcctagacatactgtgctgaaagggcacaggcttggaacactgggttcttacatgggagaagagctggcctgaaaatgcagccaacacgaggggaagcagcgctgggagaggaacagagagactggtgcctggcgcacgtcatctgcacctctgtctcacccttctccagaacatttctttgcatcttacatcaaatttgtcagcaaattctgtcggctctagttagaaaaggtgtcccattctgtgttggaggaaaagcgatgctgtctatcaggacgttaccgggtcagttgacagaactggaatacgaacagtcgattagaaaaattcacatactaatattaaatttactgaagttgatcactatattgtggtcatgtaagagaatatccctattcttttgttttgctttgttctgtttttgagacggagtctcgctctgttgcccaggctggagtgcagtggtgcaatctcagctcctgcaacctcctcctcctgggttcaagcaattctcctgcctcagcctcccgagtagctgggactacaggtgtgtgccaccatgcccagctaattttcgtattaatatttccagtacagacggggtttcaccatgttggccagggttctcgaacttacggcctcaagtgatctgcccacctttgcttcccaaagtgctgggaccacaggtgtaagccacgtcgcctggccagaaatatccctattcttttcttttcttttcttttttgagatggagttttgctcttgttgcccaggctggagtgcaatggcgaaatctcggctcactgaagcctctgcctctggggttcgagaaattctcctgccttagcctcctgagtagctgggattacaggcacccaccaccacacccagctaattttttgtatttttagtagagacagagttttgccatgttagccaggctggtcttgaacttctgacctcaggtgatccgcccccctcggcctcccaaagtgttgggattacaggcatgagccaccgctcccggccaaatatcccaattcttaagaaatacatagggcggctgagcacattacctcatgcttgtaatctcagcactttgggacactgaggtgggacgatcccttgagcccaagagttcaagaccaacctgggcaacatggcaagaacccatctctcaaaaactttaaaaatgatccaggtgtggtggctgcagtgtcaaggctgcagtgagccaggatcatgccactgcactccagcctgggtgacagagtgagaccctgtctctacggaaaaaaagaaagaaaagaaaaagagatacattacagaagtttttgtttgtttgtttgtttgtttgtttgagacagtcttgctctgtcgcccaggctggagtgcagagtgcagttcagttcactgaaatcctggttcactgcaacctcacctcccgggttcaagtgattctcctgcctcagcctcctgagtagccaggactacaggtgtgtgccaccacacccaggtaatttttgtatttttagtagagacaaggtttcttcatcttggctgggctggtctcgaacttctgacctcagatgattcgcctgccttggccttccgaagttctgagattataggcatgagccaccgtgcccagcccattatagaagcttttaggggtgatgttgtttgtaacttagcctcaaagatttttttaaaaatcagaaaaagaaaatacataacagagaagagagcaagtgataaaggaaatgaggtagaaatgttaccaatccatgaacctgagtataaaatacaagagagttctttgtcctattatttgtcttgcaactttttggtaaatttgaaattatttccaaaggaaaagttaaaacactttctaaaattgagagatctaaaatcttaggccaggcgtggtggctcacacctgtaatcccagcactttgggaggctgaggcaggtggatcacatgaggtcaggagttggagaccagcccggccaatatggtgaaaacctgtctctgctaaaaatacaaaaatcagctgggcatggtgggaggtgcttgtaatctcagctactcaggcacgagaatcgcttgaacctggggagcggaggttgcagtgagccgagatggcgccactgcactccaccctgggtaacagagcaagactccaactcaaaaataatatgaaataaaataaaatcttagacaacactatcattataagtaggattggggagatcaaaaacaacatgctctgtgctccaggtactgtttggtgtgatgttgaaaatattagattttaaacttgattttttcttttttttttttttgaggcagagtgttgctctgtcgcccaggctggagtgcagtggcgtcatctcggctcactgtaacctccgcctcctaggttcaagcgactcttctgcctcagcctcctgagtagctgggactacaggtgtgcgccaccacacctggctaatttttgtatttttagtagagacggggtttcaccatattggccaggctgatctcgaactcctgacctcatgatctgccctcctcggcctcccaaagtgctgagataacaggcgtgagccactgcgcctagcctagacttgattttttaaatttctgtcctccaatagaaatagacctgatttttaaaaatgtgcatggccaggcacagtaattcatgcctataatcctaggactttgggaggccaatgtgggaggatcacttgagcccaggagttggagatcaacctggacaacatagctagaccctgtctctacaaaaataaaaatattaggtgggtgtggtcttgtacacctgtagtgccagctacacagggggttgaggagggaggatccattgagaccaggagttccagcctgcaacgagctaggatctcaccactgcactgcaggctgggcaacagagcaagaccctgcctcaaaaaaaaaaaaaaaaaaaaaagcatgttaaaatttcaaagattgctacaaaaagaaagaaatggtgcatagattccaaactagtagagggaaaacaaagaataagaaaacataagacaaaactaaacaaaaaatgcagccaattcaaagaagcttaaatgagcatgaaaaaataaataaacgtagaaaaatgaggacactagaatcacaaagcaaaatggtagaagtaaataaaatacatcattaatcacatacacaaaaaatgtattcagggccaggtatggtggctcacacctgtaatcccagcactttgtgaggctggggcagacggatcacttgaggcaacaagtttgagactagcctggccaacatggtgaaaccccatctctaccaaaaatacaaaaaaaaaaaaaaaaaaaaagaagaagaagttatccaggcattgtggtgcacgcctgtaatcccagctacttgggaggctgaggtaggagaattgcttgaatccaggaagtggaggttgcagtgagctcagattgcaccactgcactccagcctgggtgacagagtgagactccctctcaaaaacaaacaaagaaaaaatgtattcagaggccaaatacttcttaccacctccatagctgccacccatatcttaccctcctcctagggtttggagttcctactcctggccccacaatctctccccgtcatgcagatagagggactctgggaataaccaagtcaactcaactccctctgctgctcaaaactttcctgtggctccatctcactcaaagattattttgctcattttttttttgtttttttttgagacagggtctcactctgttgcccaggctggagtgcagtggtgcaagtcatgactcactgcagcctagacttcctcggctcaagccatcctccaggcctccagggctaccacaacccagccaattttttgatagagacgaggcctcccttattgcccaagctggtcttgaacttatgggctcaacttatctacccacctcggcctcccaaaatgctgggattccaggcctgagccactgtgttccgccaatctcattcaaagtaagagccaaagtcctcactgtggtccagcagactctgcaccgtctgcttcttgttccctctctgacctcacctcccctccaccccccacacgctcctctgcagcaacacggatctccttgttgtttctctaagatccagacatgttcccatcccaccccaggaccttggcactggctgttccctctgcctaggggactctttccactaggttcagtttctctttttttttttttttgagacggagttttttcactcttgttgcccagactggagtgcagtggcacgatctcggctcacagcaagctcctcctctcaggttcaggcaattctcctgcctcagcctcccgagtagctgggactacaggcacccgccaccacccccagctaatttttgtattattagtagagacggggtttcaccatgtggccaggctggtctcgaactgctgatctcaagtgatccatctacctcagtctcccaaagtgctgggattacaggtgtgagccaccgcgcctggcccccttggctcagtccctcaccaccagcagaagaatggataaactgatcccacagtggcctgcaatgtgtgtgtgctgcaatgagaataacctgtaactgcacacgacaaccaggatgaatttttttcacggtgctgactgaaaaaagccagatgctaaaaagaacatattttcagattgcatttacatgaattcaaaacaggcacaaccaatctatgctgtcagaagtgagggtgataatgaccttggagggagggcaggtgataagggagcgccgagggggcttctggggggctggagatattgcttcttgggctggtggctggtgacacaggtgtgttcaatcggtgataattcctccagcggttacacttacggtttgtactttcctgaatatgggtctacttcaagaaaccactgctgaaaacgaggagctgcacccaccacccagtgtcccctccatccagtttaagcaacaggacattctcagccccccggggtccctccctcccaatgcaatgtgcttttatgtcttcaaggggcctggccaccaccttggttgcttcccccagcttgctatgcatgtcaccccacgcatgttccaggcagctccacagaggtccccagagagaaggcaggctgtgggtgggaggaagggcaggggtgggggacgtggcttcccagcggagcccgggcagggggaggaaacatttctgcaacaccccacaccaagtcctgacttcgggggggctttgcagggtgaattctaagtgcccagggccccatgtgaaggggtcaactgtgtctcactctgtgtctgtctctctgtctgtctctcttcctgtttcctccctccctcccagtctctctctcctcaagaagaaaaaaactcacaactatttacataacaattttatatcagactgtaacccaaaaacccaagttccaacttcgaatttttcaataaactttgaataaatagtagtgctatttttctttctttttttttttagtactgtaatgtttacttttaaatttaatttttactggcagactttacgtatatgaggttcaagaaaagaaaatctccactgtttacatttcttttctgactattaatattgttcatttcatttcctgattattactggcaataattttgtcctatggggaagggaggcgcttggcaggcctcgagttatcctttgagacatgggggtctgtggtcagatttagaaagtgcttgtgggtggctgggtgggagtgggtcatgggagacataagggcaggctggagtccagggaggaggccggccgggcagggacccaggcagcggagatggacagggccatggagaatctgggaggcgcaggccctggggactgtggattggggaaggagataattttattttattatatttttttgagacagagtttcagtctgtctccaagactgtagtgcaatggcacgatctctgctcactgcaacctctgcctcccgagttcaagggattttcctgcctcagcctcccaagtagctgggattacaggcacgcaccctcacacccagctaatttttaatatttttggtagagacggggtttcaccatattggccaggctggtctcatactcctgacctcaagcgatccacctgccccggcctcccaaagtgctgggattacaggcatgagccacgacgtctggcctaattttttgtatttttaggagagacagggttttgccatgttggccaggctagtcttgaactcctggcctcaagtgatccgcacacctcaacctcccaaagtgctgggattacaggtgtgagccactacgccccgccaagggaaggggagaatttgagtgctattgaaggtagaaaacacagaacataggctgggtgtggtggctcatatctctaatcccagcactttgggaggccaaagtgggaggctggcttaatcccaggagttcgagatcagcctgggcaacatagtgagacccctgtctctacaaaaaattaaaaattagccaggcatggtggcacccacctgtactcccaaggctacttaggaggctgaggtgggaggatcgctggatcccaggagatctgaggtgagccgtgatcatgccactgcactccagcctgggcagcagagtaagaccctgtctccaaaaataaaaaataatttaaaataaagcgcggaacactgtcaggttgtctgtgggggagcagcgggcaggcgaccaggagggctggctgctctgtgcagggctagtgcctgggttgggatgactcggcctcagagctgtaaataaagaaggaagagggccgggcgcggtggttcacgcctgtaatcccagcactttgggagggcgaggtggactaatcacctgaggtcgggagttcgagacaagtctgaccaacatagagaaatcccatctctgctaaaaatacaaaattagccgggtgtggtggcacatgcctgtaatcccagctactcgggaggctgaggcaggagaatcgcttgaacccgggaggcagagatcacagtaagccgagatcacaacactgcactctagcctgggcagcaagaacaaaactccatctcgaaaaaaaaaaaaaaaaagtagaagaaagaaagagctgccacagttgagagcttcctggatgcctttgttaactcttggggttttcacatacccatcttacagatggggaagctgaggctcagagagaggaaggcccaagtggaagagcaagcctggagcccaggtctcctcctgcctaatcctgggcttttgctggtggactcccgcccaatcttgaataacttcaggccttaaacaacctcccacgattgcttttcctcccattagaacaataaatgcagatacaaaaaccaactatgcttgtctacaaagcccaagagaatttttgaagtaataaaactgtcatgaatgcagactgtggtgattacatgacttacgaatttttcaaaactcagaatcgagccagatgaaatgatcctgcctgcaatcccagcactttgggaggctatggcaggaggatcatttgaggccaggagttcaagaccagcctggccaacatggtgaaaccccgtctctactaaaaatacaaaaattagctgggtgtggaggcacatgcctgtaatcccagctatttcagcagctaaggcaagaaaattgtttgaacccggaggctgaggttgcagtgagaaatgatcgtgccactgcactgtagaccctgtctcaaaaaccaaaaccaaaaccaaaaaaagaaaaaaaaacccttaagaatcaggattatacacgagcacacgcacactcacccataaattttaccatttgtagaaaagaagaagaaaattcaaaaccaaatacaatgaatgtactttctctggattccaattcacaccaaacaactgtaaaaatctgtttttgagacaattggggaacacaaactggcttttaggagatattaaggaatttcggttaattatgctagacttgataatgccattgtggttgggtaatgcccacataccatgccttggctgggcgtggtgactcacacctgtagtcccagcattttgggaggcccagatgggaggattgcttgagctcaagagttcgagaccaacctaagcaacatagtgagacctcatctctacacaaaattttaaaaaacattagccgagtgtggtggggtgcgcctgtaatctcagctactcaggaggctgaggtgggaggagtacttaaacccaggagtttgaggttgcagtgagctgagattgtgtcactgcactccagcctgagcgacagagcaagaccgtcaaaaaaataaagaaagaaaagaaaatgtaccctattcttctcttcaaggtgctcattgaagtatttacaaatgaaacaacataatacctctcacctgtaattttttaaaatttttatttattaattttttagagatggggtctcattctgttgctcaggctggagtgcagtggcatgatcacagctcactgtaacctcaaacttctaggctcaagtgatccgcccgcctcagtctcccaaatagctgagattacaagcactggccaccatgctttgctaatgttttaaaaattatttttgtagacacaagactatattgcccaggctggtctcagactcctggcctcaagtgatcctcccaacttggcctcccaaagtcctggaattacaggcctgagtcaccgtgcctggccaatttttttttttttttgaggtggagtctcgctctgtcgcctaggctggagtgctgtggcctgatctcggctcactgcaagctccgcctcctgggttcacgtcattctcctgcctcagcctcccgagtagctgagactacaggcccccaccacgcctggctaattttttgtatttttagtagagacggggtttcaccatgttagccgggatggtctcgatctcctgaccttgtgatctgcctgcctcggcctcccaaagtgctgggattacagacgtgagccactgcgtcctgccctgcctggcctattttttatttttatgttttttacagacagggcctcactatgctgcccggactcgtctcaaactctgggctcaagcgatccttctgcctcagcctcctgagtagctgggactacagggtgtgattttttttcaagtattcaaaaaaatggggaggggaaagaagatgaaatggcaaaatattgatggttcttgaacctgggtgatgagtatatgtaagcttattgtctcttgactttttgtgtctgtttgaaaattttcatgatataagagtttaaaaactgaaaataaaatttattgaaggagagtttgggccgggtgcaatggctcgcgtttataatcccagcactttgggaggccaaggcaggtggatcacctgaggtcagaagttcaagatcagcctggccgacatgacaaaacactgtctctaccaaaaatacaagaatcaggctgggtgcggtggctcatgcctgtaatcccagcagcactttgggaggctgaggtgggtggatcacaaggtcaggagttcaagaccagcctggccaagatggtgaaaccccgtctctactaaaaatacgaaaattagccaggtgttgtggtgggcgcctgtaaattccagcaacttgggaggctgaggcagagaattgcttgaacctgggaggcagaggttgcagcgagccgagattgcgccactgcactccaacctgggggacagggcgagactccttctcaaaaaaaaaaaaaagaaaaagaaaaagaaaaattagccaagcgtggtggcaggcacctgtaatcacagctactcgggagctgaggcatgagaatcgcttgaacccgggagacggaggttgcagtgagccgagatcgtgccactgcactccagcctggggtatagagcgaggctctatctcaaaaaaaaaaaaaaaaaaaaaaaaaaaaaaaaaaggagagtttggcgttcatcaagcaacatttggaaactacagagaactagcaaggcaaagacgcccctcccatccctaagtcctgtaccactatggttgttgacattttgatatatttcctttcagccttttctattctctgtgagctttttaaatgcgtgtgttgtgtgtgtgcacgtgtgtgttttacataactgtgtgagcaaattgtttatacagccctgttttttcccctcttaaaatgtaagctgttcccctgttaaaacatctttggataaacacaatctctaatgtttgcactatgtttattcaaaagggcagcattgccagaggttgaagctgtttccaatttcctcccattataaataatcccctcatggacctccttgtgtgtcccagaggagggattcttgggccaaagggtgcggaccctttggcagagctcatggtcaaaaatctcggcagagtttcagcctgacccgaagctaagatgacctcatacggttaaagtgagattggactgctatttatttcctgaacgtttgattcatgactcaggcttgtcaggggatcttttttttttttttcttctgtatgtgcttggttgcaagaaacagaaatccattcacactagctcacgtcaaaagggcaagagaatcgcttgaacgcgggaggcggaggttgcagtgagccgagatcgcgccactgcactccagcccgggcgacagtgcgagactccgtctcaataacaaacaaacaaacaaaaaaagggcggggggtgttgtatccttcagcaagtaaagctcatattcagcttggactagctgtctgcggagcatgttgttggggtatatctaggctatgttgattgttgaaatactgaattatttccgtattggttggtaaatcattctgtctcaagtcgctccaatgacgtcctccaccaaggccactctagctgccctggtccctctcccaggacttcccagacctctccacaatgcaggaagtaaagggtcaatatcgggcacagaagtgaaccatgctgctcggtcagtgcccaaagtattggttgtgaaattcattttttcttttcttttttttttttttggagacaaattctcactatggaactcaagcgatcctcctgccttggcctcccaatgtactgggattaaggtgtgagccactgcacctggactgcttgtaaaatatttgatgattcgcctagatgcaagtaccagaacagctgactcaaatggcttaaattgtaaggggaatctgtggctggaaaatccacacttgtgctggcttcagccaaagttgacacaatggctcagccatgtcaccaaggactttcttttctttctttccttctttctttcttctttctttttttctttcttttctctctctttctttctctctctcttttttttttttttttttgacgtagtctggttctgttgcccaggctggagtgcagtggcacaatcttggctcactgcggcaacctccaattccccggaattcaagtgattctcctgccttagcctcccgagtagctgggactataggtatgtgccaccacgcccagctaatttttgtatttttatttttttatttattatttttttaatcattcttgggtgtttctcgcagagggggatttggcagggtcacaggacaatagtggagggaaggtcagcagataaacaagtgaacaaaggtctctggttttcctaggcagaggaccctgcggccttccgcagtgtttgtgtccctgggtacttgagattagggagtggtgatgactcttaacgagcatgctgccttcaagcatctgtttaacaaagcacatcttgcaccgcccttaatccattcaaccctgagtggacacagcacatgtttcagagagcacagggttgggggcaaggtcacagatcaacaggatcccaaggcagaagaatttttcttagtacagaacaaaatgaaaagtctcccatgtctacctcttcctacacagacacagcaaccatccgatttctcaatcttttctccacctttccccattttctattccacaaaactgccattgtcatcatggcccgttctcaatgagctgttgagtacacctcccagacggggtggtggccgggcagaggggctcctcacttcccagtaggggcggccgggcagaggcgcccctcacctcccggacggggcggctggccgggcggggggccgacccccccacctccctcccggacggggcggctggccgggcagaggggctcctcacttcccagtaggggcggccgggcagaggcgcccctgacctcccggacggggcggctggccgggcggggggccgacccccccacctccctcccggacggggcggctggccgggcagaggggctcctcacttcccagtaggggcggccgggcagaggcgcccctcacctcccggacggggcggctggccgggtggggggctgacccccccacctccctcccggacggggcggctggccgggcggggggctgacccccccacctccctcccggacggggcggctggccgggtggggggctgacccccacctccctcccggacggggtggctgccgggcggagacgctcctcacttcccagacggggtggctgccgggcaaaggggctcctcacttctcagacggtgtggctgccgggctgaggggctcctcacttctcagacggggcggttgccaggcagagggtctcctcacttctcagacggggtggccgggcagagacgctcctcacatcccagacggggcggcagggcagaggcgctccccacatctcagatgatgggcggcctggcagagatgctcctcacttcctagatgggatggcggccgggcagagatgctcctcactttccagactgggcagccaggcagagaggctcctcacatcccagacgatgggtggcccggcagagacgctcctcacttcccagacggggtggcggccgggcagaggctgcaatctcggcactttggggggccaaggcaggcagctgggaggtggaggttgtagcgagccgagatcacgccactgcactccagcctgggcaccattgagcactgagtgaacgcaactccgtctgccatcccggcacctcgggaggccgaggctggcggatcactcgcggttaggagctggagaccagcccagccaacacagcgaaaccccgtctccaccaaaaaaatacgaaaaccagtcaggcgtggcggcgcctgcaatcccaggtactcggcaggctgaggcaggagaatcaggcagggaggttgcagtgagccgagatggcagcagtacagtccagctttggctcagcatcagagggagaccgtggaaagagagggagagggaaaccgtggggagagggagagggagagcgagagcgcatcagagtattttaacagcagaattgatcaaacagaagaaagaattagtgagtttgaagacaggctatttgaaaatacacagtcaggccgggcccagtggttcatgcctataatcccagcattttgggaggctgaggtgggcggatcacctgaggtcaggagttcaagaccagcctggccaacatggcaaaaccccgtttctagtacaagtacaaaaattagccaggaaatggtggcatgtacctgtagtcccaactactcaggaggctgaggcacaagaatgacttgaacccaggaggcagaggttgcaatgagccgagtttgttccattgcactccagcctgggtgacagagtgaggctctttaaaaaaaaaaaaaaaaagtccaggcgcagtggctcatgcctgtaatcccagcactttgggaggcggaggcgggcaaatcacctgagatcgggagttcaagaccagcgtgaccaacatggagaaatcctgtctctactaaaaatataaaattagccgggcgtggtggcaaatgcctgtaatctcagctactcaggaggctgaggcaggagaattgcttgaacccaggaggcagaggttgtggtgagccaagatggtgccattgcactccagcctgggcaacaagagtgaaactcttgtctcaaaaaaaaaaaaaaaaaaaaaaaaagatgaaagaaagaaagagaaagacacagagacaaaaaaagaagagaaagaaaaagaaagaggaagaaagaaagagagaaaagaataaaaaaaaagaggaagaaagaaaggaaagaaaaaaagaaaagagaaaggagggagggaaggaaggaagaaaggaaggaacgaacaaacacagtcacaggagacaaaagagaaaaagttttttgtatttttaatagagaccgggttttaccatgttggccaggctggtcttgaactcctgacctcaagtgatctgcctgccttggcctcccaaagtgctgggattacaagcgtgagcccccgtgcccggccagaccccatttctcccatttctttttatctctctgctttatcttttccagtggaagctcccaagatgactacctccagcctctggccacagggaaccttcttcatatcccacaagcaaaggagagcacctttggctcaggtttcctgccaaagtaatgaggctaactctgattgggccaacagagggcacgtgttcatgcaagagccaatcactgtgatcggagggacagaaggaaaaaccataatggccagattggctgagccaagtcacatgttcctcaaatagtaaggtgagtggctcacactagggctgcaggagccacacctgggttcaatttccattccaaacaaatttctgtcttctctgccctgtttcccgtcagtaacatagagataatgaaggcactcatatggtagagttcccgtgaggattaaatgagttagttaatgcaaagcactgagaatggtgcccatatacagaaagcgttcaaatgttagcttctgttatcgtcattacatggccattctcacctcttaaggctgcttttctttgcaagctccttatgctccacacatttccctctttctagttactattgcttggtaacaaatcactccaaaatatggtggcccaaaacaacaacagtcatcctattatttttcactgtgtctgtggtcagagttttgggaaggacccaactgggcagttctgacttggaatttcatatggttgcagtcacttggcagctgaaactggaacagggaagcagctgggggtggatggatctctctctctctctctttctcttactctctccccactccatgttgtctcagggcttctcaatgtggtctctccacgcgaactggtttgggctccctcacatcatgacagcctctgggcagttggacttacatggcagcttcggcatccagtacaagtgttttatgaaagtagcagccgcgactgggtgcggttgctcacgcctgtaatcccaacactttgggagcttgaggcaggtggatcacctgaggtcgggagtccaagaccagcctggaaaacatggtgaaatcccgtctctactaaaaatacaaaaattagctgggcatggtagcacgggcctgcggtcccagctactcaggaggctgaggcaggagaatcgcttgaacctgggaggcggaggttgcagtgagccgagatcacgccactgcactccagcctgggcgacagagtgagactccatcgaaatgaaagaaagaaagagaaagagagaaagagagaaagaaagaaggaaggaaagaaagaaagagagagaaagaaagaaaggagggaaggagggagggaaggagggaaggaaggaaggaaggaaggaaagaaggaaaggaaggggccttatctcttctgatctagccttggaatcatgcagcattacttctgccacatagtcttggttacaagcaagtcacaaactgcctagatgtaaggggagcttacacaaattccacttcccaatggaaggggtatcaaagttctagaggaatatatgggctgggaaacattgttgccaccatctttggaagttacatctggcttttactggtactgatttaagacccacctctatacagcctgtgcccaataacatccacctgggcacagctccaactccctgttctaaacagaaatagtttattgagaaatctcaatcccttgggatcaaaaacatgacagtttccatttgttctgcagtgactgctctctacctgctatctattgttttccaagactatgatccaaaatcacagcatccaagactgtgtcttttttatttatttattgttttcgagacagggtctcactctgtcgcccagactgtagtgcagtggcgcaatctccactcaccgcaacctctgcctcccaggctcaagagattctcctgcctcagcctcctgcgtagctgggattacaggtgcacaccactactgcctggctaatttttgaattttcagtagagacagggtttcaccatgttggccaggctggtcttgaactcctgacctcaaatgatccacccaccttggcctcacaaagtgctgggattacaggcatgagccaccacagctggccccaagactgtgtctttattattattattatttcgagacagagtctagctctgtctcctaggctggagtgcagtggtgcgatctcagctcactgaaaccttcaccttgccagttcaagccattctcgtgcctcagcctccggagtagctgggattacaggcacgcaccactacacccggctaattttcgtattttcagtagggacggggtttccccatattggccaggctggtcttgaactcctgacctcaagtgatccacccacctcggcctcccaaaggtggctcacagaagtgagccaccacgcccggcctgtctattatttttatttttaaaaataaatgtattgttaatttcctttttcctgttggataaaggctacagggaaacttaatgacaattttgctagagtctttaatatttctctcattttcattcatttaaaaacatagccttcaggccaggcacggtggctcacacctataatcccagcactttgggaggccgaggcaggtggatcacttgaggtcaggagttcaagaccagcctggccaacatggtgaaaccccgtctctactaaaaatacaaaaatttaaaaattagccgggcatagtggcatgtgcctgtagtcccagctactcaggaggctgaggcaggagaatcacctgaacccaggaggtggaggttgcagtgagctgagatcgcaccactgcactccagcctgagcgacagagtgagactcggtctcaaacaaacaaatacacaaaaaaacccacaaagttcatggggagggaaaggtgtagcctctcttgagaactttcctctctcattttccccccaaacaggatgatgcttcctttctcttctctatccttttctggacagccttgggtcctctcagtaacttatttgggtaagtggctggttataatggcagtgacctcgaacttaggctctggggtagttggccacttttgtcctcagttttgggcagtagtagcaattctggaagttctgggaaaaatccaatttgacatcatagtacgaacctgaaggaaaggtcttgatcccaaagagctctcggcagctcatggctgtgactgtcatccagggcctgggcctggggaaatgtttggggatctgtgggatcctttagggactgtcacagtgactcgggaaatgttgctataggcaactgttctggaactttttggtcttaggactcttttacattcttaatagtatcaaggaccccaaacagcttttatttgtgtgggttataacttttttttttttttgagatggagtttcattctagtcgcccaggctggagtgcaatagtgtgatcttggctcactgcaacctctgccccacaggttcaagcaatcctcccacctcagcctcccgagtagctgagactacaggtgtgcgccatcacgcctggctaatttttttgtatttttattagagacagggtttcaccgtgtcggccaggctggtctccaactcctgacttcaggtcatccatccgcctcggcctttcaaagtgctgggattacaggcatgagccactgcgcccggcctgtgtgggttatagctattgatatttaccatattagaacttaaaactggccatttaaacaaattttttattattgattgatttttgagacagggtctcaccctgttgcccagagtggagtgcagtggcatgatcacagctcactgcagcctcgaactcctggcctcaagtgatcctctcgcttcagctttctgagtggttgggactacaggtgtgcaccaccacacccaactaatttattgatttttttgtatacacagtcttgctgtgttgcctaggctaaaactgacaatattaaaatccagccatccacaagcacacactggcagagcaattatgtcatcacatgtcatggagccattgtatgctcataagtgaatgagattgaaatacgcaaaaaaagtcctggaattattatgaaagtaattttggccgagcgcggtggctcacgcctgtaatcccagcactttgggaggccgaggcgggcggatcacgaggtcaggagatcaagaccatcctggctaacatggtgaaaccccgtctctactaaaattacaaaaaaaaattagccgggggtggtggcgggcgcctgtagtcccagctactccggaggctgaggcaggagaatcgcggagcttgcagtgagccgagattgcgccattgcactccagcttgggcgacagagcaagactccatctcaaaaaaaaaaaaaaaaaagaaagtaattttaactttgtggacaaagtctcagggacctccaggaaaccctggaccaaactttgaaacttgctctaaaagcatttgtaagcctgggatggttaggtatgttcaacgtgcagccatgtaggagatagtgcatgtcaaaagggcccctttggatgggttaatatcactttggttcagttatctgtggcctggaaggggtcccttgtgtacaaacaaagctggggagtaggagggaagaatttttttttttttttgagacagagtcttgctctcgtcccccaggctggtgtgcaggggtgtgatcttggctcaccgcaacctctgcctcccaggttcaagcaattctcctgccttagcctccctagtagctgggattacaggcacctgccaccacacttggctacgttttgtatttttagtagagacggggttttgccatgttggccaggctggtcaaccctgacctcaggtgatccaccctccttggcctcccaaagcgcagggatttacaggcgtgagccactgcgcctggcccaggagggaggaatcttaaccataatgctcatcttgtactatctactggaaaccctaaaaatacagagaccctggagccactttctgggttctgctccccttcattgctttctagctgtgtgactttgggccaagttccttaaccactctgtggctcagtttctcttctggaaaatggagacaataatagtatctgcctctcagcgttgttataagagttaccttggcacacagtgttatgtgggtgtttacgctgagtattactgttattacagtaatcattcaaatccaagaagccatcaaaggtaagatgcattgttttttattttattttattttattttttatttttattttgagacagagtcctgctctgttgcccaggtgggagtgcagtggtgcgatctcagctcactacgacctccacctcccaggttcaaacaattctcctgcttcagcctcctgagtagctgggattacaggtgtgccctaccacgcctaagttttgtatttttagtagagatggggtttcaccatgttggccaggctggtctcaaactcctgacctcaagtgattcacccgcctcagcctcccaaaatgctgggattacaagggtgagccaccacacccagccaagatgcattgtcacttcaaatccccaggggagaaaaaacagctgccagttaaactatgacacataatcatttataagacacatcctgatttccaagtcattgaaaaggggtggggaggataaataagtcaattaaaaatggttttattcggcctggcgtggtggcttacgtctgtaatgccagcactttgggaggctgaggtgggtggatcacgaggtcaggaagttcgagaccagcctggccaacgtggtgaaaccccgcctctactaaaaatacaaaaaattagccatgcctagtggcacaggcctgtaatcccagctactcgggaggctgaggcaagagaatctcttgaacccagaaggcagagattgcagtgagccaagatcgtgccattgcactccagcctgggtgacagagcaagactccatctcgagaaaaaaaaaaaaaaagatggttttattctggaataggagagtatttaaggaaagaaaataaaaaataaaggaaaaaaagaaattttaaaattaaaaaaaatgatttcatgtgtacagaagaatttagcaacaaggatgtccaccacagcacttgtcataatggcaaacctgctgaaaccccaaccattatggattaactgcacaagttaagagagagccacaaaatattgtgactgaaggggttttcaaagattgttccaaaaccctggggatcctcaaaagtgaatcaatttctctctttcataatctttttcatcttcactctcctatgagtgcataaagcaaaaaataataagcaggtgacttctaaaaagaaaaaacctctggaaactatgcctcaaccccattctagagcctgctgggccactgctcagaaaaggaaatgtgtgccccaggctgacccactcttaagacaacccattctccacatgcctctgccttcagttacacagctgtacccagagaggggtcttgtctttactcagctgtccatccaccctccctgtgttgcaatgaatacatccctggtatcttctgtgcctggccccagcccaccccctcctcagagctccagccacacattccagtgccttcgagactcacctgctttgaaaggtagatccttacattcaattttcttgttgaaatacttcatgtggtttcttttttcttgacaagcctctgaccaacacttggtggtcattcttaaaccgttgatttttccccttcacacctattcccctccacgatcacaatcttcccagtctcaaaaatgtctctacctgggacctcaagccagaaacccaggcaatatggaggcacttcctctcctcattccacatatgccactcatggacaattcctgctttcctctaaggcagatgcttaccacacccctacccccacccttctatttagaaaatttctaaacatgcaaaagaattgcaagaaaagtagaagatataataatatactgtggatatggattcactaggtttttgcagttttttgtttgtttttgttttgagacggagtcttgctctgtcacccaggctggagtgcaatggtgcgatctcagtgcaagctctgcctcccaggttcaagcaattctccctgcttcaaccttccaagtagctgggattacaggcacccaccaccatgcccagctaatttttgtatttttcagtggagatagggttttgttacgttggccagctggtcttgacctcctgacctcaggtgatccgcctgccttggcctcccaaagtgctggattacaggcgtgaaccgtcacacctggccttttgtgtttttgtttttgttttggtttgtgtgtgtgtgtttgtttgtttgtttttgagatggggtttcactctgttgcccaggctggagtgcagtggtgtgatcacagctcactacagcctcaacctgctaggctcaagcgatcctcccttctaagcctcttgagtagctgagactgcaggtgcccaccaccacacccagctaatttttgtattttttgtagagacgggttttcaccatgttgcccaggctgttctcaaactcctgggctcaagtgattccccccaccttggcctcccaaagtgcttggattacaaacgtgagccactgtgctgggcctatttctttgtgttttaagaggcagggtctttctctgttgcccaggtggagtacgatgattcgatcatagctcactgcagcctcaaactcctaggcacgggagaccctcctgcatcagcctcccgagtagcccagactacaggtgtgtgccactatacctagctaatgaaaagaatttttttgtagacatgagttcttgctatgttgtctaggctggtctggaacctccagcctcaggcgatccccttgcttcagtcttccaaagcagtggggttacaggcgtgaaccacctggcctggtctcgctctttctctttcgacatctacattgatctgtagctatctacgtactatagatatctaaaagttatgtaaatgtctacttaagcttataggtatgagctactgtatgctatctaagcttataggtatgagctacaaattgctattgtgttatgaggggaattcaaaaagttgatggagaatggaattaagagataaaaattttaaaaaaatctttatttctcaccataaactccatcaaggtcaaagtcaagacacttttgtaaaccattataccagccatttagtctatccctaaataactgagggtcccaggaatttaatcatgtcagtgcagcctttttacattttctctttctttttttttttgatggaatctcactctgttgctcaggctggagtgcagtggtatgatctcggctcactgcaacctctgcctcccgggttcaagccattctcctgcctcagcctcctgagtagctgggactacaggcatgtaccaccacatctggctaatttttttttttttagtagagacgaggttttgccaagttggccgggctggtctcaaactcctaacttcaggtgatctgcccgcctcggcctcccaaagtgctagcattacagttgtgagccactgtgccaggccttttttttttgttcttgttgcccaggctggagtgcagtggcatgatctcggctcactgcaacctccacctcctgggttcaagtgattctcctgcctcagcctcccgactagctgggattacagtcatgagccaccacacctggctaatttttgtatttttttttttagtagagacagggttttgccatgttggtcaggctggtcttgaactcccaacctcaggtgatccaccctccttggcctcccaaaatgctaagattacaggcgtgagccactccgcccagcccagtctttttacattcttaactgaagaaaaatgggtgcccttcaaagattttaagattaggaaacaaaaagtcagaaggagccaaattgggactgccaagtggatgcctaataatttcccatcaaaacttgtaaaattgctcgtttgatgaggagaatgagcagaagcgtagacatgctggagaagaactctctggtgaagcttcccaggcttatttctactaaagcttcggctaactttctcaaaacactctcataataagcagatcttattattctttgaccctacagaaagtcaaccagcaaaatgccttgagcatccccaaaaactgttgctatgacctttgctcttgaccagtgtgcttctgccttgactggatcacttccccgctcttggcaatcattctctgattacgatttgtctttaggattgcacccgtgaaaccatgtatcatttcccgttacaatccttcaaggaaatgcattaggatctcgatctcacttgtttagcatgtccatggaaagctctgctcttctctgcagctgatctgggtgcgaccgttctggcacccatcgagtggaaagtttgtttagctttaatttcagtcagaattgtgtaagctgaggccgggtgaggtggctcaagcctgtaatcccagcagttcgggagaatgaggcaggaggatcacttgtgtccaggagttcaagaccagcctgggaaacctaatgagacccccatctctacaaaaaatacgaaaatttagtgtcaggcctctgagcccaagctaagccatcatatcgcctgtgacctgcacgtatacatccaggtggcctgaagcaactgaagagccacaaaagaagtgaaaatagccttaactgatgacattccaccattgtgatttgtttctgccccaccctaatgatcaatgtactttgtaatctcccccacccttaagaagtttctttgtaattcttcccatccttgagaatgaactttgtgagatccgccccctgcccgcaaaacattgctccaaactccaccgcctatcccaaaacctataagaattaatcataatcccaccaccctttgctgactctctttttggactcagcctgcctgcacccaggtgaaataaacagccttgttgctcacacaaagcctgtttggtggtctcttcacagggacgcgtgtgacacttagctgaacgtgctggcacgcacctgtagttccaactacttcggaggctgaggtggaaggatcgcttgagcccaggaggttgaggctgcagtgagccacaatctcaccactgtactcagcctgggcgacagtatgagaaccctgtctcaaaaaaaaaaaaaaaaaaaaagaaaaaagaattgtgtaagctgtaccaattgagatgtctatggtgttggctattgtttctgctgttaactgtaagtcctctttaattaaggcataaacaaatttaatttttttctgcaaaaattgatgtggatggtatgccacggtgggcttcatcttcagcatgacccaggctggagtgcagtggcgcaatcacggctcactgcaacctctacctcccagactcaagtgatcctcccacctcagcctcctgagtagctggaactacaagtgtgcaccaccacacccagctaatttatgtattttttgtacggatggggtttcaccatgttacccaggctggtctcgaattcctgagctccaatgatccgctggcctcagcctcccaaagtattgggattacaggcgtgaaccaccacgcccgaacttgtcccttcttaaaacgagttatccatttgtaaatggctgatttctctggggcactgtcaagtttttggaaaacatcaatgatttcatcattcttccacccaagcttcaccatcaatttgatgcttgttcttgcttcaattttagaattcgtgttgctctgataggggctcttttcaatctgatgttttattttagtgtctcaaactaggtcctgttcagacaagttataacaagttagtatgaatttattttggtgcaaaaaaaaaaaattgaactccatgcatagttttttcataatacacattttccatgaatttttggaagacccttctttttctctcttttttttttttttttttttttctgtagagatggtcttgttctgtcacccaggctggagtgcagtggcacaatcatggctcactgcagcctcgacctcctgggctcaagcaatcctcccacctcagcttcctgttactgggactataggtgtgcaccaccacaccttgataattaaaaaaaaaaatttttttgtagagatcggggtgggggggggggtctcactatattttccaggctggtcttgaactcctggcctcaagtgaccctccccaatcagcctcccaaagtgctgggattacaggcacaagccacagtgcctggccaataaatgttttttgaatgaatgaagaaattagtgcatggacatattttcccatcagctattacaataaccagactctgagttccctgaaggcagggcctgtgagtttcattgtgtaccctcagccctcaatagctgataaaaataaatattcagaaaatgcttgtaaaatgaagaagagaatatgtatgggacagaaagtagaccagtggttgcctggggctgggacagggaatagggagcgactgcaaatgggcagaagggatcttttcagagtgatggaaatgttcttgaattggctgtgatggctgcagaactgtaaaatcacccaaaatcagtaaatcacttataataggtgaattttatgacaggtagattatacctcagtaaagctgttaaaacaaaaccagtgttgagggaggaaataaatgttaccttggtaatactgaggactcagtagttatcaagacagctctcttccctgccctcatgaggttttctgtgcagggcggggacgccgacccattatagacagtgacagcctagagccatcacggcgggatggtggggaggggacaggcagaggggtgggaggccaggatgggggaagcccgggcagagaggttgggctggaatggggggcacaggcagaggggtcggggcggggactggtgaggtgcaggcagagggcaaaggggtcgaggtccagatgggagatgtacaggcagacggatccgggccagggcggggaggtacaggcccagttgaggagcataaggaaccataggagcccaaaggaggcgcccgaccagtcagggaggacttcccagaggggtgaatggctgagccagggcctgaagtataatgttcatgaatgcgacagcaatttttttttttttgagaccgagtctccctctatcactggagtgcagtggctcgatttcggctcactacaacctccacctaccgggttcaagcgattctcctgcctcagcctcccgggtagctgggactacaggcgcccgcccccacgtccggctaatgtttgcatttttagtcgagacggggtttcgccattttggccaggctggtcttgaacccctgacctcaggtaatgcacctgcctcggcctcccaaagtgctgggattacaggcgtgagccaccgcgcccagcacaattttaatttttcttaaacacttttcctgccttagcaaagtcttggaggggcggccgcccaggcgccgcgagcgcaagaccacgagggggcgctgcttcaccacgctagaggagcgctcccggcaaccacgtggccccacaggtgcgggaggtcggcgagcgcgcctggagggtggacggggtaggttacggccaggcagcccggggtggcgcgtggccctgcgcagggcagtggaagcagcgggccccagggagcatgagacgccgcgctccgtggggcggtcccagcgctgtgcagcgaggggccagggctgtccccggtcctgcgcggccggctcccggagaaactgtggcctcctgggggtggagctttaaaaaacaaaacaaaacaaaacaaaatcacccaacaggaagcggggtgggggcgcccggctctgtcacccgtggaatgcatcaaaatagcctgcgcggccgggggcggttccgggaaagggggcggccgcgaggggcggggctgcaacggagggcggagcttcccaaagaacgggagagaggagtgcagaaccggccccagggggacgtcctcctgttcccccaaaatgacctcgataggcgtttgtgtgggatggggttcctgggtagggcggggctttccagtgcgatgtccctggtctattcttagcgggctgaaacctggagaagtgggagtgggcggttgatccgggttccagggcctctttggagcgaaaagctccgtggagagccagagtctccatcctgggcgtgggagggaagatgggaaatgggccaagaggagcctgtgggaggtcctccccgggacggcccccttccatctgcatccgcgggaaccgttgtgggggcagctctgagaaaggctgctctgggcgcaaggaagggtggttgaacgaagagatcagtcagggacggggtgggggtgccttgactgtgtcccagatttgctgcgtgcttctgacctcagttccccatccttccagttgctcaaatcctctctgtcccagtcctaggccgtttctgcccctctcacttcctagtggtttgcagaggggaaacactgaggctgcctcttctgtgcctggccctgtgttggcacggggaagtgactgagacgccccagacccccttctccctcacagtccagtgaggcagacagacctgccaccagatagtgacagcccagaatgagtcattgagaggacgggggaggcacaggcagatgggtcagggctgggataggggaggagaggggcctgtaggatccaaggggagagtgggtgctgctgactcagtctgggggggttgaagagccgtctgaacttagaccaaaaaggtaggatggggccgggcgcctgttatcccagcactttgggaggcagagacaagaggatcgcttgaggccaggagttccagaccagattggacaacatagcgagacccccatctctacaaaataatttaaaaatcagttgggcatagtggtgtacgcctatagtcccagctactcaggaggctgaggtgggaagattggttgagcccaggaattcaaggctgcaatgagctatgattgccccactgcagtccagcccgggtgacagcgtgagacccctgcctccaaaataataatagcaaaaatactgggctgggcgcggcggctcacacctgtaatcccaacactttgggaagccgaggtgggcaaatcgctgaggtcaggagttccagaccagcctggccaacatggtgaaacccagtctctactaaaaatacaaaaattagctaggtgtggtggcaaggcatctgtagttccagctacttgggaggctgaggcaggagaatcgcttgagcccaggaggtggaggctgcaatgagatcacaccactgcactccagcctgggcgacagagtgagactctgtctcaaaaaataaataaatcctaatgaaaggataggatggggctcagggccttggaagagggtcaccttctaacaaaaggtatttgaacggagtcctaaagaatgagtagcattcttctgggaagtgctgtgtcaccatgaaggaaagggtgttctaggcagaaagaatgacaaatgcaaaagcttggaggtgagagtgtggcttatctctggcagggtcctctgctccctgcctgggacattcccccaacgtcataccccgacagagctgtcttaggtctcctagtcctggagtccacaagcaggttaatgggatgtaatggaaacgctatagagggcagacccctaggcttgttccctcacagcctgatgcttttttgtttttgagacagagtctcgctctgttgcccaggctggagtgcagtggcgtgatcttggctcactgcaaccttggcctcccaggttcaagcgattgtcctgcctcagcttcccaagtagctgagattacaggcacccaccaccacgcctggctaagttttgtatttttagtagagacggagtttcaccatgttggccaggctagtctcgaactcccaacctcaggtaatccacttgcctcggcttcccaaagtgctgggattaaaggcatgagccaccacgcccagccttttgttttgtctgcttttttagacagggtctcacgctgtcaccctcacaggctggagtgcagtgactgcatcacggaccactgcagcctggacctcccaggctcaagcaatcctcccacctcaacctctccagcagctgggactacaggcgtatgccaccacgcccacctaattttaaaattattttgtagagacagggtctcattatgttgcccaggctggcctcgaactcctgggctcaagcgatcctcccaccttggcctcccgaagtgctgggcttacaggtgagagccacctcagtgcccggcctcagcctgatggtttcacgactgcctttgactttggcccacactaatcaaatgtatcaccgtgggccactgactcaacttccccatctatccagtgggaatagaatattggactgcacaaaatcaaccacctcattttaaagagctataacgaaacaaaatttatatgttatatatttttaaaaatacatcttatagattaaaggactcaagaaacaatagcaagactgtaaaacgttgccacatcaggtgacactttggccagagttatggaaaatgctgacaaaacaagaatttgccagcatgggcaaagatatactgttaccaacccaacttgttaaaatattaatattgagctaattagaagtagtttttttttttttgttttttttttttgagacagagtctcattctgttgcccaggcaggagtgcaatggtgtgacctcaggtcactgcaacctctgctgcctgggttcaagcgattcttgtgcctcagcctcctggaattacaggcgcctgccaccacgcccggctaatttttgaatttttggtagagactgggtttctccatggcggccaggctggtctcgaactcctgaccttaagtgatctgcctgcctcgacctcccaaagtgctgggattacaggcgtgagccactgtgcccagccagcagttcataatatttgttttttattccttgattctaactctgtaaggaatagaaatggggtgattaattttggctcctttaatacccgcctggcaggtgctgagtcagtggtacctgttaccacgctatgactcagaggttatcactcagggacatccttctgactctgtttcagtccatgactcaggaggaaaggttctagggcctcaccagcgccctacacacaccctcgtttcccgaggggcaccattatattcttcctttattggctgtccttgtataatacaaatcttcaagtttagatacaaaaaaaatctggaaataaaagatagaaaagtacccgccaggcaccccttccccttcttcccggacccctccccagcgggcaccgacatgaggtaactgcgcatcttctcctcctcctccctccccgcctcctgggcccccaacttggccctagcccccatgagaccttggcccaaggaagacatgggccccaaagttggagggtgatggaggtgagtacagcattggcagtgaacgcagcgtgtgggcagagggcagcccttagcttgtgctgtgcatggggggaggagacgaccagatttggggtgggcactggtgtggggcccaggagagcccctaagcaagtgtcccccctccatcctgtccaacactggaaggtgggggtcaacagaaactgggaaatggagtgtgaaccaagggcattcagtgggattgtggccaacccctgtgtctggggttggggaagggggcattgccagcctaagtccggcagtgaaatggttcccttagccaggctgggtccgtccctgaattccatcctgttgcaacctgggcgtcacaatgttggttctgtagtggttgtcggggtggttgagggaggggggtgttgagagggtgttgaggggcgcagccccagggagcagggttaggggagaggttgtgcctccacccccaggcgtggggcacctggagatgatggagtgggtggggcggctcgggctacagttcaatctcgaatgtcttttgcaggtcgccagaaaaggggttggagggtttctctacagtggctttgccttctaatgccgcccactgggcctcaaaggggtccaactctggagctggggcaggcgctggctcagggggccagggggccccattggggcgagggcgggcctggctcccaggggcactgggtatggcagggggcgggaaggccccagctttcccaagcagagtggcaggctgaggctggagctgggcggctgagcagaaggcgtttgccaccatctgtgagggtgtgatgcccaccacgggcacccggggcatcggtgggtagcccaagcccgggtaggcgggcacaaaagggggctgcatgtgtgggggtggcaggaacacggccacttgggcaggtgcagcgtcaaagggccccacgggggcggggaaaggctgcagggcaggaggcatggtgggcactggggccactgaggctgcttgctgctgttgctgctgctgctgctgctgctgttgctgttgctgctgctgctgctgctgggccttggccacctgtgacacctcctccagccatcgctcagcctctgaaggtgtccgcttgtgcccaggctggaaggcagctgcagggggcacggagggctcaccccaggcagaagtccctggagagaggagagggacaggtgagggagggggcaacggcttcagcagaagaaccccaggctgggaactggcatggtgtggggatcagagcacggactctggagccagaccgcctgcctctgaatcccagctctgcacctcccgagcttgctgacttcaggcgagtgacttcaccattctggaccacgtaatggttctggagtgctaagaacatacaattctgagcttctaaggccctatgatgagaaagtctaagtaggactgacatcctcctagccccactacccttctgactggtcagtgccaagcctaggattcactattttgttttgtttgttgtctgttcgttttgagagtctcactctgttgcccagggatgccctatctgggctcactgcaacctctgcctcccaggttcaagcaattctcgtgcctcagtctcctgagtagctgggattacaggcgcgcaccattacgcccggctgattttttgtatttttagtagaggcgaggtttcaacatgttgcccaggctggactcgaactcctacctcaagtaatccccctgcctcggcttcccaaagtactaggattacaggcatgagccaccacacccagctggtattcactattttgaatatcacccttgattttctaataccttcagaatgtattgttttaggagttaagattctaagattgcatggatctttctccacatgtataatagtatcctaacatagtaaggtttgacagtttagggttgggctttctaagattctcgagttctacatttacagtgtttgagattctaaggtgcacctgtggttctaggataagcccatggctctaagatgatacatggttctcaaggattccatggttctgaaacgatctctgggctctaaggtgatcccaagattctagcatgagcacatgcctctgaggtgaccccgtggctctacaatgatcccgtatctctaagataattcatggttctaaagtgatcacttgattctcaggtaatcccacggctctaagatgatccttggttctaggatgatcctctggttctaagatgatctgtgtttctaaggtgatcctatggctctaagatgatccatagttctaggatgatcccatggttctaaggggatcccgtggctctaaaatgatcaagggctctgagatgatccatggctctaaggtgatcacatgattctcagataattccatggctctaagatgatccatggttctaggataatcccctggctctaagatgatccctgggtctaaggtgatcacatgattcttaggtaatcccatggctctaagatgaaccacggatctaggatgatcccctggctctaagatgatccatggctctaagatgatcacacgattctcagataatcccatggttctaggctgatcccctggctctaagatgatccctgcttttaaggtgattgcatgattctcaggtaatcccgtggctctaagatgatccatggatctaggatgatcccctggctctaagatgatccatggttctaaagtaatcgcatgattctcaggtaatcccatggctctaagatgatccatggttgtaggatgatcccctggctctgaggtgatccatggttctaagcctgtaggatcccaagacccctggagtgtctgggtagccctggatagaggaggggatacaggagggacatgcagggtgtctgcccagcagaaagcctggctttacctgttgtggcaggtggtggccctggtgctggcgctccagcactggcaaaagatgaactgatctgtgtgcacagagcgttgatgctgtcactgtcgccggcaccaggaggctccatctcaggcactgggaagcagggcaggacagaggtcagcaaacaggcccagaccctgccgcagccccgccctctaccccccgccctcggtggccctctcttctgacctggatcctttcccactgtagtaactaagtggccatgaccgccaaataactgtgcatatgtgtgtgtcacatctgagcggcagaacgactgagttagtgtgtgacatttgacggctgacagtaacagggaccccaaaccaaggacctcaagatttgtgtgtggccacaaaccagaagagttgtctaaaacacttagcaacatatattagtttaaaaatatgcccaaccacgtgcatggcaaggacatgggcccagtctgaatgggctgtggcatggccgctcactggctggggatcatttgtccagctttgggcagagaagtggggtcctgtccaccccacccaggctgatctatggcaaacatcatgagagcagagatacacctgtgccagcaaggcaggagacactgagcaggcatggcggccccgtgagggcttgtgatgagcaaaggtaccatccaaataaacaattaaggactcccatgtgtggtgtgtgacacatgtctgtgatgttttagccaatggctgtctccaagggaccatgtagatgctccagtgaacatcagaactggccgtaggagtctgcaggtgtgctgcgggggcgcccgggtgggacagccaatgtcgacaatgattgtgcatgttcgtccaaacaggaatgcagcttctgagagtgtgactggggtccgggtgtgtggcgtcctgatgcgtgactcccaggtgtgagtgcatctgccgtgtgatgtatgagtgtgtttgcaggtgtgcatggatctgcacatgtggctttggagtttgcataaatctgggtgtgtggtctgtgaaggtgtgtaaatctgagtgtgtttcttttttaaaaatatttatttatttatttttgacacagggtctcgctctgttgcccaggctggagtgtagtggcacaatcttagttcactgcaacctccgcctcccaggctcaagcaatcttcctgagtagctgggactacaggtgcatgccactgcacctggttaacaataaaggttaatttttaaaatttttttgtggagatgagatcttgctgtggtgcccaggctggtctcaaactcctgagctcaagtgatcctcctgcctcagcctcccaaagtgctgggattacaggtgtgagccaccacgtctggccatgtgtgacttctgactctgtgattttggagtgtgtgtgacttgagagtatacctgactgtgagtttgtgacttctgagcatgtgtgacatgtgtgtgggggggtgcaatgtctatgtgagtatgtgaaatttctgtgtggcaagtcacatccaaataagcgtgcagctggccacaggagtgtgaggcttccaaataaagcctggagctcctgccacctctcaggagcacgtgtgacagcctggggagtgtgcctgatgtcaggctgcgttaaggacagcaaatgtgagggtgtgtgatggcccaggaatgctgcaggcatggagggagcgtgcgtcactctcaacaagggttggcatctgctcaccggttaccttttggagcagcccagcctcctggatacagctcaacaccctcccacatcaatccccgaggacataacgggtaggcgatgcagatttggcatccaggagcaagagagtgggccagaccacatgggttcactggctgctggtggggaagacagcccttctgcctgcctccctcaggcaaaaactcagtagcgtgccacctctatcttccttccctatggcagagattgctcttaatttttttttttttgagacaggttctcactctgttgcccaggctggagtgaagtggcgcaatcttagctcactgcagctgggctgaagcaattctccttcctcagcctcctgagtagctgagactacaggcatgcgccaccacaccaggctagtttttgtatttttttgtagagacagggtttagccaagtgatctgcctcaagggatccttgagcccctcttgggctcaagtgatctgcctgccttggcctcccaaagtgctgagaccacaggcatgagccactgcacttggctagacatcacttttagatcatgatgtacaccacctgtctcctttccctggcccatggcagacattagtaatcaaacacaatgcttttttcccccacggagctctttgctcaccttacccgtcacctgtccagacctcatggctcccctggccaagtgctagaagaaacagatccttgtaactccatcttccctccaagtaaaacaggacctttatatctcctctctcttaccaccagccatggcagacaatgccaatcaattatgatgtgctgctccttttcgtgatgggtactgcctctgctcaactctgtgcctacaacaaatgttcctgatccatcactatgcccctgacccctgggatctctgagctcactggtgccctgcatgtcatgtttctactgaccaaattctgggagtctcccctttgggtaaaaacataacactcttgctactctttcttctcccttgcccatgacacacactgcatggagatcatgactgctaaccgatcatgatgtgtgccatctttctcgtttcccttaaccacagcagacattgctaattgatcatgacttgtgatgccttttttgccatcccttgatgctccctgccctaggcagacatttctaatccatcacaatcctcctttcctcagagcctgaggaatacctgtatccttcacctagccagatctcataggtgaatgcttggagggagggagcattaacctgtagtgcttcagtctactcctgagcaaaaacaggccaatggtgttgcttctcttctttccctggcccatggcaaacttccttatccatgcccgacttctttgtccatagccgactttgctaactaatcatgatgtgtgtcatctttctccttttccttaaccacaccagacattgctaactgatcataacttgtgatgcctttctactatcccttactcagagcagacacggcttatcaatcctgatttgtgctatctctttcctctcccttgcccactgctaatcgatcatgacatgttcccactctctctcctttgcccatggcagacagtgcaaatcaatcacagtgtgaaccatctcgcctccatcccttgcccacatcagatagtgccaattgattccaacgccgtttcccactgggcccagggctcacctgtgcccttcacctggaagtcagtgcggcgctgcagcgtggatggcagctcattcagccgtaggctcagctgccgtttgaaaggcgagttcttctggctgagtgctgggaacccacggaaggagccctggcgaaccagctgctccaggggtgcatggcgccgggggatggcggccgcagtggtgcctgcagccacaggggtgcctgcctcacccttctcaccaggggatgtggtggctggtgtcggggacacgtgcccaggctgggcagggccaggagccacagtgggggcagctgctgcctctgctggagacatgggggagatggatggttagatatctcaccatggcatgcaaggcctctcccacctggttctcttgatcattctccaaggctgccttccttgcccagtgagtcctgcccttaagacaagctagtcaaagccctgagatatccctcacccccacccaagtcatgatccccttccccaggaggctcttggaaaaccgtcccccaggctcaccctctgtgtctctccagcttcctgcccctttctgtcttgccctgctgctctcaccattcttccctctaagaccctctatctccctttttgatcacttaacaaacactgatttggtgctggaacaacgtatcaggcattgttccagatgcttttcaagtattcactcattcaatccacacgactacccatggggttgatatgattctcattttacagatgtggaaactgagacccagcaaaggcccagtgtgatgtgcccaagtcctactgctaggaaggggcaggctgactctggaccccatgctccaaatgactgcccgccctgtctccctctgacctgtctctccatatcatgttgtctttctctgtcactgtctgttcccctctgtctcccacctcccagccttcttcccacctcaagtagctcctcccttcctccagtcattctagacatggcttggatgcttcatcctctgagaagctttccagattgttccaggctctcagcctggctccctccactctgagactgttctctgtactctgggaggaaacctgacctccccactcagcaggagaggcaggctcttcaagggcagggctgccctcacccctgccaaaccacaaacacacatctaccctcctaccagggcctccccgagctgcagcctgaatgccatggagattaaactcaggcccagagagaccctcccataaggatgtcgcccagtgctgcttctcccatcgtgacacaatggggcacccatgcaggcctggcccaaggcagtggaaacagcccaggacaggttggaaccaggaaacctcctctgcctccactcactgtgtgacctcaggaagtcccctcccctctctgggctccagtttgccaactagaaacctgggataaacatctcagtgctacctcccaagcctctgagagggtcagtttaggtagtgaatgttaaatgttttggaatccaacaaaagcatgcctggacacagtggttcacgcctgtaatcccagcactttgagaggccaaggtggggggatcagttgaagccaggagttcaagaccagccttgccaacatggtgaaacaccatctctactaaaaatacaaaaaaagattagctgggtgtggtggcacacgcctgggattccagctactctggaggctgaggcaggagaatcgcttgaacccgggaggcagaggttgcagtgagccgagatcgcaccattgcactccagcctgggcaacagagcaagactctgtctcaaaaaaaaaaaaaaaaaaaaaaaaaaaacttagctggacgtggtggcgggcacctgtaatcccagctactcaggaggctgaggcacataaatgtcttgaaaccaggaggcagaggttgcagtgagctgagatggcactactgcattccagcctgggtgacggagagagactctgtctcaaaaaaaagatgttcttttttttccccttacaatccaggatctaattcaggatcacatctcgcatctattaatacctgttaaacctcattagtctcccttaatcaggatcagttcccaatggtaaattctttgtaaattctaagtagtgttttcccaaagaacttaaattcacagtaaaataaataaataaattaattaattaataaataaattaattatatggtgactcaggacatacatacaattatattttaaacacacacacacacacacacacacacacacacacacacagagttttagaacttacaaagtatttaaccatttacctagaaagttagttttaccaagtatgtttcaaactttcttgatggcaatccagagttaagagatatcttttatatggtagcctcttacacacgcgtgcacacacacacacactctctctctcaaataaaagtatcattaaattatatttaacccttatgccattcaatatactctgatattttctatgattctctatttcattgtttttaaattaatttttttttttttgagacagggtctcactctgtctgtcacccaggttggagtgtggtggtgcaatcgcagctctctgcagcctctacctcctgggcccaggtgatcctcctgcctcagcctcctgaggagctgggaccacaggttgcaccaccacgcctggctaattttttaatgatttgtagagacagggtttccctatgttgcccaggttgatttcatttttttaaatgtcagccacatgggctgggcccagttgtccacacctataataccagtgctttgggaggctgaggtgggaggatcgtttgaggccaggagtttgagaccagcctgggaaacacagcaagatcccagttctacaaaatataaaaataaaattagccagatgctgtggcttgtgcctatattcccagctacatggaggctgaggcaggaggattacttgagcccagcagtttgaggctgcagggagctgtgatcgcaccactgcactccagcctgggcaacagaattagacctcaactcagacaacaaaacaaaacaaaaaatgccagccacagtacagcaaattggcttcccaggtcttaatacacaggttgaaaagccctgagaaggccaggcgcggtggctcacctgaggtcaggagttgaggccaacatggtgaaaccccatctctactaaaaatacaaaaattagccatgcctgtaatcctaactactcgggaggctgaggcagaattgcttgaacccgggaggtggaggttgcagtgagcctagatcacaccattgcactccagcctggttgacagagcgagactccgtctcaaaaaaaaaaaaaaacaaacaaaaaaagaaaagcctcgaaaagccccgaattggtggatagtaaaccacttggtgcgcccttagaatattgcccagagaactctttccatggaagttgctttatttatttatttattttttgagacagagtctcactctattgcccaggctggagtgcagtggcgtgatctcggctcactgcaacctctgcctccagggttccagcgatcctcctgcctcagcctcccaagtagttgggattacaggcgtaggccaccatgcccagttaatttttgtattttagtagagacgaggttttaccatgtcgcgcaggctggtctcaaacttctgacctcaagcgatccgcccatctcggcctctcaaagtgctgggattacaggtgtgaaccatggcgcttggcctgaagcatcccctactttgtaaactgttgagtctctgcacctctgcagctccctgccccctgatactgggtaccctgtgcccactctgtgctctgctggcgcttggggcaacacccacctttcttcttgtccggggcctctcgctcagcaggccgcccacccccagacaggcggaaggagccctcgcgggcgaagctggtgcggctggcatcgaaggcggccgtgaccccacattccttctcccgtcgctgttttcgctccaggcaggcggcaaaagcacagcccacagcgtggctcagcctctcgccctatggggagaggatgggcgggggggttagaggcgctgggcagtgcggacaggggccaggggcactgggttatagccgctaggtactgggttgccccggatgagtctctgcacttctctgggcctcagtgctcatctgcaccacaaggaagggctggaaatgacagctccaagtgagagaagccagaaaccaatgagcctgttgtgtggctccacttactggaaattccagaagaggcaaaactaatctatggttctatggtgaaaaaaagtcagaacaggccaggagtggtggctctcgcctgtaatcctagcactttgggaggctgaggcgggaggttcccttgagcccaggaggtcaaggctgcaagcagctatgatggggcaactgcactccagcttgggtgacagagtgagattctgtctaaaaaaaagtcagaatagtggtagtttcctatggggtggggaatgactggaaagtgtatgaggggatgaccgggtggtggcaatgttctagatattgataggggtttcgttacatgggtgtatgcagttgtcgaaattcgttgactgtacaccaaaggcttgtgcattgctatagactaaacgtgtgtgtctctctcagttctaacgctgaagccctcatccacaatgtgctggtatttggaggtgggcctttgagagacaataaaagttatgttagatcatgaggtggggtcctcatgatggaattaatgcccttatttatttattttttttctgggacagggtcttactctgatgctatgctggagtgcagcggcatgacctcagctcactgcaacctccacctcccggcttcaagcgattctcctgcctcagcctctcaagtagctgggattataggcatgcgccaccacacctggttaatttgtgtatttttagtagagatgggatttcatgatgttggtgaggctggactcgaactcctgacctcgagtgatctgcccacctgggcctcccaaagtgttggggttacaggcgtgagccaccatgcccggccgggattaatgcccttaaaaaggaaaaagagacaagagatctcccctccaccttgagaggtgaagatacagaaagcaggcatccatctgcaaaccaggaaaagagccctcaccaagaaatgagccatttgacaccctgacctcaggtatccagcctctagaactgcggcaaacaaatgtttgtcatttaagccacacagtctacactatctggttatagcagcctgaactaagacaatcatatctttcgctttgaagaaaaaaaaaatctggaaacaaatacgaattctacttaatggtgtgcatgctgaagtagtccaatgcctacaaatttgacatacaaaaagaatcagacggtgtgactgcagtcgctcacacctgtaatcccaggaggccgaggcaggcaaatcacttgaggccaggagttcgagaccagcctggccaacatggtgaaaccccatctctactaaaaatacaaaaatctgccaggtgtggtggcgtgcacctgtaatcccagctactagggaggctgtggcaggagaatcacttgaaggttggaggcggaggtttcagtgagccaagatcgtgccactgtactccagcctggggcaacagagcgagactccgtctcaaaaaaaggaatgaaccactgatacaagcagctcacgcctgtaatccgagcactttgggaggccaaggtgactggatcgcttgagtccaggagttcgagaccagcctgggcaacatggcgaaatcccatctctacaaaaaattagccaggcatggtggcgtgtgcctgtagtcctagctactcaggaagctgaggtgggagaatcgcttgaacccaggttgcagtgaggcgagattgcaccactgcacaccagccttgatgacagagagagacgctgtgtcattaaataaattaattaaaaacattgccgggcagggtggctcacacctataatcccagcactttgggaggcagaggcaggcggatcacctgaggtcgggagttcaagaccaacctgacctgcatggagaaaccccatctctactaaaaatataaaattagccagctgtgatggtgcatgtctgtaatcccagctacttgggagactgagacaggagaattgcttgaacccgggaggcagaggttgcagtgagctgagattgctccattgcactccagcctgggtaacaagagcgaaactctgtttcaaaaacaaacaaaaacacaacattacactaagtaaagaagccagacacatattatatgattccattaaatgaaatatccagaataggtaaatccacagagagacaaagcagattagtggttgccagggggctggggtagtggggagacggggtgaattgatgaatggagatggggtctcctttagcggtgatgaaaatgtttcaggactgctaaagtcaatggttaaacaacactgaaaatgtattaaatgccattgaattgtacacttttaaatgattaattttatgtgaatttcacctcaagaaaaaaaaaaagttgaacttggggaattctactgcttaatggttaaaacttccttcagaagtaggaaggaattcatccaacatcacattctttacccacaggagatggtcctgctcttttctggctttcattctcatccccaaatagttttttttttttgttttcttgagacagagtctcgctctgtcacccaggctggagtgcagtggtgcagtcttggctcactgcaacctccgtctccagggttcatgtgattctccccacatgtgattctcctacctcagcctctggagtagctgggatcacaggcgcctgccaccatgcctgtctactttttttgtatttttagtagagatggggttttaccaggttggccaggctggtctcaaattcctgacctcaggtgatctgcctgccttggcctcccaaagtgttgggattacaggcgtgagccaccacgcctggccaatactcttttttttttgagatggagtctcactctgtctcccaggctggagtgcagtggtgcaattttggctcactgcaacctccacctcccgggctcaagtgattctcctgcctcagcctcccaagtagctgggactacaggtgtgcaccaccacacctagctaattttttgtatttcagtagagatggggttttaccatgttgtccagggtggtcttgaactcctgagctcaggcaatccccccgccccagcatcccaaagtgctgggattacaggtgtgagccactgcacccggccctcacgtgaatactctaaattgggaaccgtgagtatactttcttctccagatgaggaaactgggcacacagaggttagtgatgtgcctgaatgcaggaagcttgtaggggtggggctgggatgccagggcatgggagggaagagttggccagctgtggcaatactcacggagtccttcagtgccagaaaacagtggcagatccagcggcgggtagtcccgtcacgacagatataggagaaagccttgtccaggttgcggtcaggagcacaaaaggagaccttttcgatggtctggtcgaccagaagatcctaggaggggccggggaggccaggagaagagtgtgaactctctttcaagtgttcactcaacattctctctgtgtctgctgaaatccagtcctgaacagggtggggacccagcagtcactgagacaccctgtgccttgcctgcagagggctcccaggtcagcgggaagatcagacccatcacgagatgggcagcccagagtcatagccaggatgtgatgaaggaggcccaggcagaggggtcagggccaggaccatggaggcacaggcagaggggtcagggccagcatggcagaagccagcttggggtcagtcaggcaaggcttcctggagcaggtactaactaagaaaaaaagtcaaggaacagtattttgggctgagggaactgccttgcaaaggtggtgatcttgttctgttattaacccaactctcagcatgtcctgggcacctcctagggcagtctctgggctgggggcagcagattcaaggtgagcaaacagatacctagattgtggcctcatagtgcttccttctgactgggcagggtgacaataaacacttaatggctaacattcattgatctgagcagttacgatgtactagaccccatttaaatatatatatatatttttttcccagaaggagtcttgctctgtcacccaggctagagtgcagtggcatgatcttggcttactgaaacctctgcctcctgggttcaagtgattctcctacctaagcctcccaagtagctgggattacaggcacgcaccaccacgtctggctaatttttgtatttttagtagaggtggggtttcaccatcttggccaggctagtctcgaactcgtgacctcaggtgatccaactgccctggcctcccaaagtgctgggattacaggcgtgagccaccgtgcccagcccacatttaaatttttttaaaaattattttgtatagatggagccttgctatgtttcacaggctgatcttgaactcctggcttcaaggggccctcccagccaggcaccatttcaaataacttgcatatgctttctcacttaatggtagggtctattataatccctgtttttctgcgatggagtttagctcttgttgcccaggctggagtgcaatggcatgatctccgctcaccgcaacctccaagtctcgggttcaagagattctcctgcctcagcctcccaagtagctaggattacaggtacacaccaccatgtccagctaatttttgtatttttagtgagatgaggtttcaccatattgccaggctggtctcgaactcctgacctcaggtaatctaccctccttggcctcccaaagtactgggattacaggcgtgagccaccactcccggcctataatctgcatttttcagatgacacaactgagactcagagaggttaaatctcatgcccagggtccctaagctgggatcggagctgaggcagctgctccagtctctctcacccacagcctatgccagttcccaaataatcacagcatttattcctgagttatgacgacagagggagcacacggcatcgtctagaaggtccctgagggagggatgtgcagaggaggcgggaaggtgtcctccgccctgattccagcagggtgagcagacaggccccctggcgtccacccccacaggcctcctaccttggttttgtcgtccaccactcggagcccatcggctgacacccacaggacagacttcacggactttcggcccatctggagggaggcaaggggacaaaggagccgggtcagggtgcctctccctgtctgaccttgccccctccctcatggcagccccctcactcaccgccttcagcttcttcaccgcatcttcacacacgtgcattccccgggactcctctacctccacgtgacccaggtacttgggttggagggaatggggggggggacatgaaacagcacagtaatcactcattctcagtgtccactgagcatctgccatgcagtagacaatattttaagcacatgatgtgtatgcaatcatttattctgcatctcaactctacaaggtggagaccccattcctggtctagacatgcagatggggaaactgaagcacagcacgtagtagtgattccagtctagctatacccctgggccctaacccggcaccgtggtcctcccgagagctagtatttgcatctctgtgcgtgaggactggccacaggccatgcaaagctgctttgcctaccctaaagcagctagaaagagcctgggccagtccccacaatgactgaagggagttagggtacctgagccccagctccctcatctgcaggtgggatgactgttgcctcgagtttcccaggggaaagctcagttgcacactgctgcagttttaataacacaccctttactggctgccttactttcctcactcccaacaccatttcctgcacctcccaaatgaagccgtcacattcaaagtctgcttccagggaagggaacgtaaggtggtggaggggctgtgaccatggtcagtcatcacccagccaggaaggggctgagctccacagtccacgccgtgaatcctgctctccccctcacaggaatgtaaaagcgtagggtatggctaaaccagaacgtccttatcggtagagcgctttgcaaatgctacaccacatgacggcttccaggtaatagtttgctggtacaaaaaaatgtgttctggttttttgtttgttttcaagattgggtatcactctgttgcctaggctggagtgcaatggcacaattaaggctcactgcagcctcgaccttcctggactcgagtgagcctcccacctcagccttgtgagtagctgggactacaggtgcgtgccactgtgcctattttttgtagagacagggtctccctgtgtttgcccaggctggtcttgaactccttgactcaagcaatcctcccaccacagcctcccagtgtgctggaattacaggtgttagccaccactacgcttcaagtttttttttttttttttttgaaacagagtctgctctgtcgcccaggctggagtgcaatggcgctatctcggctcactgcaatctccgcctcccgggttcaagcgattctcctgtctcagcctccccagtagctgggactacaggcgcccgccaccacgcgaggctaatttgttgtatttctagtagagccggggtttcaccgtgatagccaggactgccggcctcacgctttttaacaccaacttcaaacgacttgggctggtgtcccagccaggccgcgcacccgcacagcacagcacagcggcccccgtccccctcgccccgccgcaccctgccgcgcccactcaccctgaccgggaagctgcacgtgcccttccgcaccgcgtcctcgtctgcctgccactggtgcgggcgcgacgcctcgggcacgtaggctggcttcctccgccgcaggctctgccgtaacttgttcatggtgcccgccccgtctggtgacacaggacagtgatgtgggtcaagggtgggggtcagaaggtatggagctcaacggggagggaccagtgctcagggagcatggggtcagataacaagataactggaagcggggttacagggtcagttggcagcgcacatgggatcagcagctcaagtcaggggacagtgaggaaaggagccaacagaagccaggggagtgcgaaagttgggcactggggattcagaaccatggggctaaggggctggaggtctggggtggggggtatggggcacaggcttcagggcattggagggcttcttgtccatgtggtggatgcttcctcattcccagggccgtgaggacacaaagggtgggaaatcagacgtaggagggcatgggggctagagggcatagaagtcaggggccgcacggtcaggggttttaggggtatgagagtcaggcagtggggtgatcagagggcagcagaggagttgggaattgcatgggtcaggggtgcaggagtcaggtgcatggggtatgggggatggtggcttgtctctggaactctgagacacagccattctgtgacaactgtgtctagtccccaggcaaggcttctggggccttgcactgatgactgtcagaggcagggctgtgggtgtgtggagtgggtgtggaggtggccagccactaggacagtcttcactgatcagccatcctgacagtcccaggactgggagcaccaacagcagagggggatgtgtgtgtgtgtgtgtgtgtaagcaagtgtgcaatggtatgttctggaacgctgtctatgaggggctctatatctgagcaggcaagtaatgtctgtgagtgtgtttctgaaggctgtctggaagaacgcatgtctgagaatggtgtaggatagtgtgcatctgtgaatgctgtccgtgagggatgcatccaaaagtgtggttgttgtctgtgagtctgaggccctgaaggttgttgctgaagggcatcgatgtctgagagtggttgtgagtgtgtgtctgctgtctatatccgagagtgccgttgttgtctatgagaacttgtggctcagtgcctgttgcctgtgagggtgtgtctgtgtttgagatgaggctgtcgtctttcaaagggtgtgtccatggctgttatccatgtagctatgtctctgtgtgaaggtgtggctattgtctgtgatgacattgcctcggagagtgcatctgagggatctacaagactgtctgtgtccaagagtgcagctgttggcggtgagcctgtgtgactgtggctgttgccttagagtgtgggtgtgtgggtattgcacagagggtgtatctgtgtgcagtggtgcatccgttagggtgtgtgggaacatgaggttgtctttgagagtgttttcatgagggttatttgtaagggtgtgactgttgcctgagagagtgctgggtgttctttgtgagactgtgtgcatgtttgtacacaaccgtagctccctgtgagagcctgggcccgcgggtgctgtctgtgaaagtgtggctgtcgtctgtagaaatgtgggtctgtgtgtgttgtcagactgtgcaagagtgtgtctcttttttttttttttgagacgaaattttgctcttgttgcgaatgaaggctggagtgcaatggcatgatctcagctcacagcaacctctgcctcccaggttcaagcgattctcctgcctcagcctcccaagtagctgggattacaggcatgtgccaccacccctggctaattttgtatttttagtacagacagagtttctccatgttggtcaggctggtctcgaactcctgacctcctgacctcaggtgatcctcccgcctcagcctcccaaagtgctgggattataggcattgagccaccacgcccggccaagagtgtgtctcttgagagtgtgtatctcagagtctgtatccagcgagcgtctgtggtcacctgtgaatctgggtgttgtctaggaatgtgtgtgtgtgtatatatgtgtgtacattagtgtgatgaacatctacttcagcatgtgttcaagtgtgtcactgcattagcaagtgtgtgtgatctgaaagagatctgtgtgtgtgtgtgtgtctctaaccgtatatctacagatgtgagtgtttgtgactctgcacttgaggctgtaagggtgtcagggtgtgggtctgtgcatgagtggggctctgacagtcgctgaggaagatgcctgagggtgtccactcatgagtgtgattaagcctgtgtgaccgcagggacagctcctctggtcgtgttaggcaagaccacatacccattcagccctgccctgtcccaggctggtcgctcacctggctccgtcctgcaggtttctgggggccccggggccccacagggggctgggggcaggtgccgctcaggcctccggggtccgccctgcccgagtaggggaggagaaggtgagaagtttgtctgggttggggctcagtctgatacttcaccccgactttggacttcggccagccccctccatcttgggctccctgatgagagtcctagttgtcctagcaactgttaccagggagatcagccacctggttccaagggcccaggaaggagtaggtatgtttggggggcatatgttggggatgtgctggcctcaggagagcctcactgcccaaggggatgctgtgagagtggccttgccctccagatgcatgtgcagggctacacacatacgcagccaactcatatctacaggtgtccctagcatctggccacagctttacacacttggttacacatagacgcaatcacagctacacacctcagatcgcagatacacagaaacagtcccaaacccagaaagctgccactgtaaacatctggccgcatattcatgttcggacacacacagtctctactacagacatttgtccacatacatgcagcatgtcctggcccactcagttcccaccgcagacacctggtcacaccacccactgaaatttggtcacttccacattctcagccacatacaaagaacggggcccagacaacccactagagccgcacatgcgtggccacacccagtgacagctatgtttcctcaggcacccgcccaagatactgacgtcacaggcccacccagatagaatcacacccagagttcacccatttgctgacccagtcccacacgacacaatcgcagctatatacacttgttacacgtatctccactgctgcacactgacatctggtcacagatgcacacggacagacacacatttggtcccacggagaccacatgcagcctcaaccagaccagtcacaccaacacactgtttttggccacacactgtcacgtggtcacacatactcagtcataggtgctcaaatctggtcacagcatcagtcacacagtctattgtgacagccacactcatagggacagtcctctatacacaaccacatacagaggtactgatggccacagcatgcaaccacccacaaacaactgtccccaaggatggcctccctcaagacacagccatggtggtcctataggcatggccacagcatcaatgtccatgtgacccagccacctatcatggtcataatcccgtcacccagtgtccatacacagctgtaccatgtcactccaatgcagcgaaacatatagcctttcttcatgcaggcacacaagtcacacagacaagtatgtggccatatagaatcacagccccgtgtggacaggtgcacaaagtcacaagccccacctacacacatatctcacacatagagacataagcacacagttttagtttcccatgtcacaagtacacagtccagtgtatgcacataaatgcagtgaccaggatgtggcatttatagctgggtttacacagaagacacaggtcctgacggagccatgtgcacagtcaggggccaatctcatcaccaaatcacacattctaacacaggtagtccagcacatacacacagagacaaaaacaggcacacagctacagaccccacactctcacagatgatgacatagacacagacatctatagtcacccagggtcagacatgcaggtcaaacacaataatatggaagccataatcatatacacacccctacaaacataatttcctggcaccagcacggagacacatccacagctttagtcacacacaaataatccctctaaatagccagggtttcagacaccaagtcaaatacataacccaaatcacacatgcaaggctagaaatacacacaatcactcgttatcacacacactgctagatacagtcatttatattaatacaacctcagtcacacactcagacatggttctgcatacgcaaccactgtcatacacaatactgtcacacaaccccagtcacacagatacaatgtgacttcagacacaatggcagtcacacaggcagagttgcacagacaggtgtgtgtcactcacgtatataaaatcaggtagagacacaactataaacattgtcagtcactgggagggtcacacatgcacatggagccatagacaactccactcacacacagtcacaactccacccacgtcctgtcagtcacacgcatgcccacccccagactcaacacatactgtcacatacccagttatagttaccgaggcatacaaacacagggtcacaaaagacacaatcacagacaaccacagtcacaaccatgcacacctccaaacacagacagactaaaaagtacaggattctgcacagtgagcagctgtcacacacacatacacagtcacacagatactagggtcacagacacaatcatagacaccaccacaagcacacacacacgacacaggattcctcagtcaccagctgcagcgtacgcgtgcacacacacacacacatacacagccacagtcacacaaacacagggcacactcctagccacctccccatcgcttgcttccccccttccccccaggtaccacacacaaagccgccgtcaccgtcaccgcagacactgcagacagacagggctgcacccggtccctggggagccgcccccagcccagcctgtatcctggagcctgagggccaggtccaggagggggaagcggtgcattgtctgcgggtggggccactcttggacagctgggcagccctggggacaaagggggtggcctagggatcctgtgccctgggacccatgaccaagccagggggtggagggattgggggttgcctgaaattgtccttattttattcaggctggggtggggtggagtcccaggcacagggaccttgttttgagaagtggctgtgcctgggactccgcccaaggattggggggatgctgtgcccagggtgcctctgagacctgggggcaggctgtgcttggagtccccctaggccttggcgtggtgggaacgctgtacccagtgaccccatcctcgagaccgtacctaggcagttgttgtgctgagacccccttaggcagggagaggtagggattgtgtctggaatcgcgtcctggaggccttggtttgatacgggggctgtgtccccgaccccatctccatccccatctagttctaggagttgtacctagaatctctgtacccctgtccttggttttgtggggggtctgtgtccaggatccctatttccagggccttggcaagagatggcccaggggtctgtgcccaagaccccggtctcctgggctttggcttgttgggcctgttcctggacccccacccgggaccaccctctccagccttggcaccctctctccatccgggcgccgcggccgcctcccaccctccgccacatcagcagcggcgccgcccccgacccgagcccccctctcccgcccttctcacgctggccgccgcgctgcgggacatccagggcccgggcgcccccgcctcccgcggccctggctgggcctggctccccgactgctgctgctgcggtggtggcggcggcagctcggtctgacgccggccagggcccggggccgggggatggtgcgggatgcacgcgcgcgagcctcctcggctcccgggaggattccgttccgggggcgggggagcgtccctcggcctcggctccccgccccgaccccgcccattggcccgccgcctgccgtatatgcagaaaggtcccgccccgccccgccccttggcctgaagaccccgcccacacgcagacaccatcccgccttccccggcgcggccaccgccccgccacgcccattggccagtcccgagctgagcatgcctatgaacatcgccgagtcctttcccccggtccgtcctggcctgggctccctttccctccgtgacacctgacctcagatcccctccagctccgcgtccgaaagagttgcttctagaggcgccttgccgccccacacccccaaatcttcccgctaaccccatggttccccagcccggcgggggcgggcaggagcggtgacgaggcactttttgcaaggaaggggagggggtgtgaacagaccaaggcgtcctgatgcgcgatcggttcggctttgggaacgggggcgccggggtgggaccagggcgcggttctggccgctacggcgcccccgccgccccctacgccaatcctgtgggtttggcaaagcagctggcagggacattagagcccattagtaaaggcgaggttgccaggagtgaggggagggagcccgcagccaagaggcactgtgtgtgtgggaggcctcagctgccacagcccttagagcaggtggtcagcacgtgggggggggtggggaaggcgagaaggaggttcccggcaacagatggcacaggcagggctgaggctttcagacaagggggtgcaggggggctggccatctgcacctggaggccgctggcgagctcctccccctctccccccaaccctagcgcagagaaaagagctgggggaaggggagggctgcttttattccgattgaagattcagctcccccccaccccgcacccctacctctccaacacactgagaggctggaacccgggagaaggcagctgttggaggagcgagggaggcagaggtgaggactgcctccaggaccatctcgccttccacgggaggcttgaggcagaggtgagggctccccctgatgagtctgatctgcataacgacatgcagcggcccaaggctccctcaaatgttggcaaagataagttaaccgcttccctggcttagttttcggatacccactttcgagtggggaggtgcaggatctagggcacgaagttgggagttccccagccccagggatcctgagctcctgggccaaggaggagagccaggcaagactgggaagcccaagggggctcctctgacccagggcagacggggaagggataagaggcactacagcagggtacggcctgctctggggactgaatcccccatggaggctgtcatgagggatccacccaggagtcccctttggtggggaggctgccggcagtggctgcgtctggctggcgactggcccagtagcggtggtaggtgtcctggaagaggtccctgcaggcgatgtgggctcggaggtgggcacaggccaggaaagcccctgccagcttgcggtgcagggcataggtctcctcgggtgggggacacagccggtgccgcagcagcaccgggatgaggtcctgtatgcggcgggccgtttcccccgacccaaagtcataagggccctgggtggcgaaaggctcccccaggatcatcactgcctccacgtgggcgtcggagaatgcctgggagtgggggtggggggagagcaaaggcagccagtgtggacatagagccctctgcataacccagaaacaacgtgtagcctccactccctccagtctccaccatcaacacaagccccgactcccccaagagtgagcagcttccactccttccagagcctggactagacaagcagctgcctattccccgagtaagcaccccttacttccctgcagagcctccaacagacaagtagccctctactctctctacaacagagaagcggccttcgcccctcctgaacagatccacggtgcccatgttcccagggttcctgagaagtcaggcagccacctccccccactcctccccaaagcccccagcatggataagcatccctcctagagtcacccactccccaggtatagacacacagcctccattctccctagtggagacaagcccctcctagagtcccccagtccccgggtatcgacatgccccatcacctactcgagttcctcagtggagataagcagccccccactgcaccccaccaacagacaccagcccctttctcccccagtgtctccccaccttggtttcaaagcctgtgaggaatttgaggtccctggacttctgcaggacacagtctctgtctccatcagctgcagccttcaccacctggggagacgggtgggagttagagggacaaaggccggggctcaagggggctctggagaagaggagctggaagcctgggcctcccatgtacccacctccattctcatctgcctgggccctccctcacctggaagcttcctgctcccaactttgcctgtctgtgactcccttaaagactcttccagagcctgggagtggaggtggttagggatcctgcccacctagagggcaatgtggggcctgcccgggaactgccacagtgaaacagtgcaagaaacaagtgtcagggctgctggtgagtccaaacactcaactggacgggtatgagcgtgacccagaactgcatccaaagttgccaggggccatctctctgtctcccacactggactttgagccccgtgagagcaaggatcccagttgggtttagtcgcacggggcacagggtctggtgctgaggaggccctgggtgaaccttgctttagcaaatgagcgtgtggagcagagcagctctccagccatgagctcacacacacagggcaggagttgtgggcatggagagatgcccagctggggccagctggctagggttccgtcccagctctgccacctgccggcctgttgggcctccactttctcatctgtgaagtggggatgccaaaagtgccttcctcatggggctgttgggaggataaagaaggtgatgcctgtggcctgcctggcgctgtgtctcatgcaggaagcaccgtaaatactataatctaccattattaagaggtgggcacgggggtccctatttcacagaaggggaagcagacccggagtagggagtggaaccgggtcacaccactcactactgggttgcccttttttgtgaggagggggattcgggattaattccattccctctctgctccccctgcccgagcatgtctggccatctgtcaggcctgtggtcctcagaagccagggcttttataaagtggcaaaggctgcaggcctgggtgggaggggagggtgtcagtggggagaagaagggtctcagctttgtgcctcagtggccggcagagagggccccaaggggcctgtgtgtaaggggttatcacctcctcttcctgttcctgtctcagaggtggccccaccagtccccagaccagacccctagacacctctgtccccaacttctagcccgtctgctcccatggactgccagctgggcatctcccagccacccctctgcccctctccacagctgccctgagctcccacccccaggcttagagaccacttcttattcagagggagttttcaaattctgactgcatcccttccctgctcaaatcttttccacggctccgcagggcacctggatacagtacgagctgtagagcgcagcctctaaaatccgcagtgatttgctgcagcctcgtcactgtgctgccccccgacctgccctcccactcagaatgggagcttcctttgggtgctctagggccttactactaccagtgtggtccccatacgggtagccctggcctcacatgggtgcgtgtcagaacatagcatcttacacccacctccagaccagaatctgcacttgcacaggatcaccaggcttcacatgcacatccaagtctgagaaatgctgctctaatgggactgtcccttatcactgcctcgtcttggcacatgttgtctatctgaaataccctccgagccttttcccagttggcccccctcatccctcaggtctcaatgctgacactccctcctccgggaagccctccttggctccccaggctggctcaggctcctcctctgggctcacagtgccctgcgcttcccccatcccagccctgtccatgctaggtcctcactgtcgcctcactgactatgagttctgtgaggaggggcctaggctgggcccaggtcactgctgtgtctccagctttgcctagaatagagctgggcacagaggaggggtcagaaaacatttagattggctgggcaggagggctcatgcctgtaatcccagcactttgggaggccaaggcaggaggatcacctgaggtcagcagttcgagaccagcctgggcaacatggtgaaaccccatctctactaaaaatacaaaaattagccgggcgtggtggcacatgcctgtaatcccagctactcgagaagctgaggcaggagaatcgcttgaacccaggaggtggaggttgtggtgagccaagatcgagccactgcactccagcctgggcgacagagcaagactctgtctcaattaaaaaaaaaaaaaagaaaagaaaaaaaaggaaaagaaaacgtttagattgatggctacatgattagaggacccagggcaaatgtccaatctcaacaacgaatgaaatggtattctctgcagcctctaagacaaactgaccccagtgggtgggagagacgagccaagtacgtgaggaaacacctcctgtagacagagttgcccccagggacacacacctgggctggacaccagggccctggacagcatggggtctggagaggtgacaagatggtcactgtgggcctttctcttaggagggagctgggcagtggttggaagcttgggctctggacctggaccacctgaatttgaatcccaagtctgctgtgatcttgggcacgtgacttaacccctccaggacccagttacttcatctggcctaaaacgggcctaaaaacggtccttttcgcattgtgttgctgtgtggtttatatcggttcctatacgtaagcactaaagatggagcctgacatattaagtgcttggtgtgtgctagttgctacgagtattactattatttattatttcttaattccagaaactgcatttcgccttcttactcctctgcctcagtatatggcttgagcctcagcctttcagaggccctggggtctgggggagactcacctcgatgtaatggtctgtgaactctgtcccaaactcccggcttgcaccaaagtccagcagggtcacctggaagcaaggaatggtgaaaggaatgctgggatcccattcacaccctcactgtctattggggcagccaggatctgtctccctccccatgaccctgcctgctcctgccagagtccctgcctggctgcctcactgggctcctggcctcatctcccgtttccaaccgaccccctagctgaaggcttttttttcttttagttctaattgtttatgcaataacaaattttagacccagaaaaaaaatccagagaataataaaagatatagaaaagtaaaatgaatactcacaaatcctgccacccagcctaaaatataaaatactccccatccggccacacgtggtggctcacacctctaaccctagcactttgggaggccaaggtgggtggatcatgaggtcaggagtttgagaccagcctggccatcatggtgaaatcccgtctctactaaaaatacaaaaattagccaggtgcggtggtgcgtgcctgtaatcccagctacttgggaggctgaggcaggagaatggcttgaacctgggaggtggaggttgcagtgagccgagattgtgctattgtactccagcctgggcaacagagtgagactccgtctcaaaaaaaaaaaaaaatactccccatccacgtggagcctcctgtgtatcccgccctgatcacacctcccccaggtccccagggtcacctctttcctacaatcattattaaattatttcctgaaattctcatttatgcatttctatattttctatgtatgtgtacagctgtaaacaatctagagtaatggtgtgcatattttcaaacttcacagaagtggtatttactgtcgttctcctgcaacttgtgctttttgcccagcatggttttgcgatttatccctgttgccatgtgtcgctccagctcagtcactcatttcacactgctgtgtaaggacttcgttgcgtgaatctatcacagtgcatttatctggctgaggaatactgtggttgtttctgattttttttccttctttttaaatatgtttattagttataaactctgttctgacatttttttttttttttgagacagggtcttgatctgttgcccaggctggagtgcagtggcacgaccatggcttactacagcctcaaactcccacgctcaagtgatcctcccgcctcagcctcctgggtagctgggaccacaggtgcaccccaccacacctggctaagtttgaaacattttttgtagagatagggtttcactacgttgcccagactggtctcgaactactgggctccagtgatcctcccacctcagcctcccaaagtgcagagattacattagtgagtcatctcacctggcctgtttctaatttttgtgctcaatgaacacctgtaagaatgtttctagggcagtagagtttgaactgaccacaacccacagtaagaaattgtttctactggtggctgggcgtgatggctcacacctgtaatcccagcattttgggaggctgaggggggcggatcacctgaggtcaggagttcaagatcagactggccaacatggtgaaaccccacctatactaaaaatacaaaattagctgggtgtggtggcgcacgcctgtagtcccagctagttgggaggctgaggcaggagaatcacttgaacccaggaggtggaggttgcagtgagtcgagattgtgccactgcactccagcctccattctcaacaagagcaaaactctatctctaaacaaacaaataaataaaattatatatatatatatatatatatatatatagagagagagagagagagagagagagtttctactgggcgttcatgcaaatgcacacaaaaacgtcaaacaaaagtgtcccaaggccaggcgcaatggctcatggctgtaatcccagcacttcgggaggccaaggcaggcggatcacctgaggtcaggagttcgagaccagcctggccaacatggtgaaaccccatctctactaaaaatacaaaaattagctgggcgtggtggcaggcacctgtaatcccagctacttgggaggctgaggcaggagaattgcttgaacctgggaggcggagggtgcagtgagccgagatcacaccattgcactccagcctgggtgacaagagcgagacttcatctcggggaaaaaaaagaaaagtgtcccaaaataatatggatccctcccatctgtgacatactgacatcatctattccataaaaaaaaaaaaagtgctggtggatcatgaggtcaggagttcaagactagcctggccaaaatggtgaaacctcatctctactaaagatacaaaaaattagccaggtgtggtggcgggcacctgtaatcccagctacttgggaggctgaggtgggagaatttctcgaaccccagaggcagaggcttcagtgagctgagatcgtgccattgcactccagcctgggcaacaagagcaaaactctgtctcaaaaaaaaaaaaaagtcctgttggaaaccaataaattgatgtcaggactcctatcacttggagttgggtaaacatatccctggggtatgaacctaggaggggacacagggtgtatgcacattgtggagaaagaagaggcaagggactagggctggagactccgtggggccacaggatgctcagcaaagggttcagacttgattctgagggggctgtgaagctgtaggagggatatcttgaccagatttgtgctttagaaagacccctctggggacaaaatggggatagaccactttggaaaacagttggcaacccctgataaaggtaatgatgtatccaccaacactcaagtctgcaggtccaaaccttcactacaggtctttgtacaccccctgccctctgctgggaacactctgctctctggatggttgtctccttttcccctgtcccatctcagccttttttttttttttaaatagagcccaggctggttttaaattcctggcctcaagggatcctcctgcctcagcatcccaaagtgctggaattacaggcatgagccaccatgctcagcctctggtctcagctttttttttttttctttggtgagacagagtctcgccctgtcacccaggttggagtgcagtggcatgatcttggttcgctgcagcctcgacctcctgggctcaagccatcctcccacctcagcctctcagtggcctcagctttaatggcacttgctttaagaagcctcccttaatccctgctcaccccacagtgagtcaggcactttccctgggatcccataacttcctgtgcctcccccaactccagcccccacccctctgcctgtgcctcccccatcccggtcctgacccatctggcctgtgctcctcattgtggttggtacgaaccactctaggtcatcgctgtgtggtgccaggtccccccactggactgggcactctgagaaggcaagggtcagggatgtctttttattgctgtcaagaggcaagggcaggtgatggtgtgttctgtatggatgacgagtgtggtagtgatggctaactgccttccaaaagctgtacttcccctctgtgctgtcacattgccaccaggaaccactgcctagccagggactccattttccagcatgccttgcacctaggcaggctatgtcactagctctcactgatggaatggcaacggaagtgctatgtccattgccccaggatgagcttagtgtatttagcctgggcattactttttccacttctggccaaagcagttaggcagggggctaccctcaacctctcttaccctttccttgggaagcagagcgttgcaaggccccagggatggcaaaaccacaaaagggaaggagctgggtccctgaatcccacttggaaaagggccacccctgcctattgtgggggtaatcaactgctattttgttgagctaccgaaatatcaaggaatatttgttacaacagcaaatgtacccagacacacatcactaggaaccaacctggtggctggaggcatcatacaggaagttggcccagttggggtcagtctgcatgaatcggaactcaaacagctcccgcagacacagcgtcaggagctggaagcaaatctggggtggggagaattaacaggcatctcagtgtgatctcccttgtggtgccactgctggcctggagagagaccatgagcctggcccacccgccctggggccatgcccttcccactgtgccaccagacagcatacctggttccgcaggtcctggcttaggccctggcactggtccagggggacccctccagccagctccatgcccagcacccgtgtcgtgcacagctccttaaccacggctgggacccggaagaaggggtcatttgccagcagctgcctggggcagaaggaaagggaggaaggggacttcgtgcttcaggcttgtgacccagcttgagacctcctccttgtgctctcagaagtcctccatgaacagtctgcgccatgccctccctcctgcccatctcttgctgctgtctgccctgggtgatgaccaacacctggctggactgagatttaacaagtatctccaaggtgcctactctgcacctgcctctcaactgggtgctgctggaaacccagtcaccacttccctacccgaaacccttctatgacttctggttgccccagaaggatgagttcaggtgtatttcagcctttgcattactttttcattaatttattaattcattcatcccaaaagtagtcactggtatcaaaatctgtgaagtctatagtgatacccatgggtcagtccttgcaatcactactctgaacacaggtaaatagcgggaaagaatcttctgtgtccatccttgtgctaaatgatgctggggacagagcagtgaatgaaccagtccctggacctggcccccaaccccgagaccacactctcacaaacagacggattatagattgaggtaagtgtgttggctgggtgcagtggcttacacctgtaatcccagcagtttgagacaccgaggtgggagaatcgcttgagcccaggagttcaagaccagcctgggcaacatggtgaaacctcgtctttatgaaaaactacaaaaattagctgggcgtggtggcctgcgcctatgttcccagctactcaggaggctgaggtgggaaaatcacttgagcctgggaggtcgaggctggagtgagctgtgatctcaccactgtattccagcctggaaaacagagcgagaccctgtctcaaaaaaataaaagaagtatgtctatgtaagatttgggaggcagagaatatgagcaaggtctctggttgaggatccgtgggatggctggaggagagtgagggagaacaggagggtggtgtggggttttatcctaagggcacccgggaatcctgtgggggacgggggggtctctggcccatcaccccacttcacactctcttccttgagctcctcctttggggtttgtatttttgtccttgttgataaaaatctctgatgtttgaactgctcctcatgaaccggagccatgtggggcatttaatcggcacactcccctttcatcctcactccacagtgaggggatgctctctggaggccactgtacagattgtatggatgcaggccacgtaacctgttaagggctgacccaggatttcatcccgcatctgagtctagggtgtgtgcctctaaccactgccttctactgagctttcactctctgtctacagagcttggcacgttttaggctgtcaataaatgtgtgagccacactgtggaggaccccactgaggtgccattaattgctacacatcaggatgcttccaagatataaccacattgttccacgtagccatagttcatgcattttcactgctacgtaatattccacagatgaatataccgttgcttatttgtccaccctgctggataaacttgatggatatgggttgtttccagtttggggctgttgcagacaagcgttctagaacagtctgatgatggatactggcaaaagggtccctagagtgttcagcagggagggcaatcgttggcttgcagagttcttgaatataagggcttatgtgatgatgccaacctgttctcaaaatgcttctaccaccttctcccacaacctgcagtgcagaagggatgctgtggagcccactctctctacctcccagtgctgtgggctccttgctctccgtcagtccagcagaggtaagagtgtgtcattgtgtaattaattaagtgcctgtgtcggaccacagtggatatgcggcccatctgacacaggagaagactgccgcttgggaagtgacctgcccaagctcacagaggacaaagggggtaagcgaagtgatggatgagtggaaggatggatgaacaatgattgaaagaaagagagagtttgccctaccccacagctccagctgccagaagctgagggggcagctacttcccacccagcctgggagggagggaaggagggaagctcagggcactcagctcacctgaaattctgggcacaagccgcctcacgacggtagtcacactcccaagccagctcctgctgcaaggcctgcaggctctgctcggcaaacaggcctgtgggggaggtgtgtcagccagggaagggccccgagcgcccactggtggatgccttctcctgccaaccctctctctcctgtctcccgcgctgtccctcacagctcctactctaggcctgtgacccacatctgtccctctcctgtctcccacgcagctcctgctcctgcctctgacctgcatctgtccctctcctgtctcccccgctgccccttgcagctcctgctccaggcctctgacctgcatcgtatcatctgtctacacatttccctcgtccttcatagcaccacagggttccccggggtcttccgaagccttttctgggctctgtctcttgcacatgcctgcaccccagtccctggcagctctttcagagtcacgcctgcctctattctgtctccttttcatactgactctcacgttgctcactgcatctgaatctcacttctgggcctggctttccctctccctctccgtctcttacacaaacacaacccaccctcctttctctaggcgcctcctcacgtgccatccccaggactgtccttttctgctctgccgcacctacaatcccgctccctgcatgcacaccctctgagagtctgctgctgtatcttggccctgggctcccgtctctctaaggctctgttaaaatccataaggcttttcccacacctgctcatgctccctgggctctccccgccttggtgtcctttctgtctctgacactcccgctcacaacgccagcacaccctgcccgtgctctcctctgggctccccctcctgctttctctctctgggcatagcccctttgggaggtcagcagaggagtgggtgggcgcctcacccgcgggcagggccgcgctcatcttgagtaccgccagcaggttctggacatcgctctgaatgctctgggctatgccggggtactgtaaagggagaagggagggagagaaggtgggagtcacttctctgggctagcagggtgcccgcccctaccctgcccagcctcccctctcacctggatcttcacggccacctccgtcccgtccctcagcaggccctggtgcacctgcccaattgaggcagcggcaaagggcacctcctccaaggaggccaccttggcctgccagtccctgccgagctcctcttcaagaactctctgcggggagtggtcacagccatcatcattgtggcagagttcattccccaggctgagtgctttacgtgttgataaccccagcactcaccacatgcagggccctgggctaagctcttggctgccaccccctttgcagatgaggaaactgaggctcagagagagctcccttgtgcaagtgactagccaggcactggcagactgtgaggctcagcctagcctgtgtcccctgaacctggactccctgggctgttgtggggattgctattatttatagttaagactcataacaatcctttttttttttttttttttgagacagggtcttgttctgtagcccaggctggagtgtagtggcactctcacggctcactgcagcatcaacctcccgagctcaagccatcctcctgcctcctgaatagctgggactacagatatgtgccactgtgcccagctaattattactgttattatgtttagtagagacaaggtctcactatgttgcccagggtggtctggaagtcctgagctcaaatgatcctcccaccgcagcctcccaaagtgctgggattacaggcatgagccattacacgtggccaaccatcctttattatgctcttatatgttattattaactcacagttactgtgatcaagaagagctaaaatttacaatgggcttcctgtgggccaggtcctattcagagtggcccagagagaggcagtacctgcctggggccgcatggcgaataagcagaacagggatgggagagcaggtgggtggcggaatcctggattccatgccttacccagttattagaacagctcatgtcctgggcacttacttggtgccaggcgccgtgccaacctattacagacacgatctcctttaattaaaaaaacagtaataatcacagctaacacctgcatgttgctcacagtgaatcaggggccgttctcagtgctcagtgtaaactgatttatgtgaccctatgatgtgggtgtggctgtcactatcgccatttcccagggaagggaactgaagcacagagaggtcaggctgctgttccctgttttaatcaccacagcaatgctaggaggtgtgtactctggtgattcccattttacagatggggaaagtgaggctcagaggcagggagtggggcagtgaagccaggaaggtcaggcaggtcagaggagatggagcctgcctccctcaccgccctcccccactgggcactcaccagcatctgccagcggggcatgaagtcggcgctctggcggacccgctcaaagatgtgctgcagctgagggctgatgaagctgttgtcttgggagacagtggaaccaggggggaagtaagcgaagaggtgaggagggaccccgtgtgagtatctgaagttggggcctgttggtgggtagggctggggtagaagggaggtcaggggtcaggagtcgagggtcatgctgtaccctggatgctgagcatctggccaaccttgagggcggcccctcgaactgtacataaggtctgcacaatccgctcggcattggcctccgacaggaaggggctggagtccagcccagaaccaccctctggggagagaacaaccattagaattataaccacaaatatcatcactgcggccaggcccggcggcccacgcctgtaatcccagcactttgggagacccaggcgggatgaacacaggagtctgagaccagtctgggcaacagtgacatcctttctctattaaaaaaaatatatatcatctgcacaccaacaggaatggctaaaacgaaatacggaggccaggcttgttggctcgcgcctataatcccaacactgggaggtcaatgcaggaggatggcttgagtcaaggagttccagaccagcctggataacaaagcaagaccctgtctctaattagctgggtgtatggtggcatgtgcctgtagtcccagctactcaggaggctgaggcaggaggattgcttgagccctggaggttgaggctgcaatgaactgtgatcgcaccattgcactccagcctgggcaaccaagcaataccctgtctcgggaaaaaaaaaaaaaaaagaaaagaaagaaagaaaaataaacataagttaaaacaaattgcaggagagtcaaagagtaactactacagtattgaatagatgagctatcactacacacaacagcccaggtgggtctcaaaaatgtaatgctgagtgaaagcagccgggtgcatgaaatcatcacccagttacactgatataaagagcaaaacaaggccaaacaaatccagggtccaggagccaagacagaggtcacccttggtgaggggagtgaccaggtggggacatgagaagggcaacgattctcgaaatgtgggccagggacccctgagggtccctgagaccattcagaggggtctgagagatcaaactatttttatcgtaacattaagatgttattttcccctttctgctctcatgcgtctaagaacattcactggagttctccagaggctccaggacatgtgaggacaccatcagactgacagctgatggaatgtgtacgtgtgtactcttgtgttttaaaaatatctctgtatttttgttgtgtttttgagacagtgtctcactctatcacccaggctggagtgcagcggcacaatcatggctcactgcaacctcctgggcccaagtgatcctcctgccttaacctcctgagtagctgggactacaggtatgcaccaccatgcttggctaatatttttactttctgtaaaaatggggcctcgctatgtcactcagactggtctcaaattcctgacctcaagggatcctcccgccccagcttcccaaagtgttgggattacaggcgtaagccaccgcacctggcctaaaaatttctcagttttaatttctaatatggtagacattgataactataatccacataaataagctctttggaggctcattctaacagttttattgagaaataattcacatactgttataattcaccatttaagttatataattcaatgattattagtatattcacagagttgtgcaagcatcaccagaatcaattttaggacagttacaccacgcaaaaaagaaacctggctgggagtgctggctcatgcctgtaatcccagcactttgggacgtcggggcgggatcacttgagttcatgagtttgagaccagcctgggcaatatggtaaaaccctgtttctacaaaaaatacaaaaattagctgggcatggtggtgcatgcctatagtcccagctactcaggaggctgaggcaggaagatcacttggacccaggaggtagaggttacagtgagccgtgatcccgccaccgcactccagcctgggtgacagagtgagaccttgtctcaaaaaaagaaaaaaaaaaaagaaaccctatacccattagcagtcactcttcatttcccccaatctccccaggccttgacaaccactaatctactttatgtccctacagattttcctattttgtacatttcatattaatggaatcattcaatatgtggtttttcagtgtgtggttgcttttacttagtgttttttttttttgaaacagtgtctcgctctgtctccaaggctggagtacaatggcatgatcttggttcactgcaacctccgcctccccggttcaagcaattctcctgccttaccccccacccaagtagctggggttacaggcacccaccaccacatccagctaattttttgtatttttagtagaatcaggatttcgccatattggacaggctggtcttgaactcctcacctcaggtgatccacctgcctcggcctgccaaagtgctgggattacaggcgtgagccaccgcaaccggcctcacttagtgttttcaagattcatctacattgcagcatgtgtcagcccttcattcctttttatggctggataatattccattgtatgcctatcacattttattcatccattcatcagttttaaaggtgtgcagggatcctgagaccaagaagtttgagagcagctattctagggtttcttactctgggtacggacaaatgtactttgtgaaaacgcaccaagccatacacttacaggtatgtgtacctgggtttatatgcaaattacatttcagctttggcaaaacatttatttttctttttttaatatgaacactttatgaatttatgtgtcatctttgcacagaggccgtgctaattttctctgtctcattccaatttttatttatatgtgatgctgaagcaagcacagcacaacaaagcaattcttaagcctttattaattttgaaggccagttgtggtggctcacagctgtaatcccagcactttaggaggccagggtaagaggatctcttgagcccagaagttcaaagctgcagtgagccatgactcaccactgcactctagcctgggtgacagcaagactctatctcttaaaataaaatttaaaataaaataaaatgttattgagctcattattgagctgttccaggcagaatcctaagtgtctttgtggattctctggctgaatgcccacaatcacacctggaagtaagaattatcaatcctttaattttcaaggtgagaaagcaagagactcaaagaggtgcagcacctatccctgggtcacatagcatggaagtggcagagtggggtgtagactcaggctggtcatacccaaaccctaatcctccacctaccctcaactttttattttgaaaaaaatatccaggctgggtgtggtggctcatgcctgtaatcccagcactttgggaggctgagcagggaggatcacttgaggctaggagttccagaccggcctgggcaacatggcaaaaccttctctctacaaaaaatacaaaaaattagccaggcgtggtggcacgtgtctataatcccagctatgcaggaggctgaggtgggaggatcacctgagcctggggaagtcaaggctgcagtgagccatgatcgtaccattgcattccagcctgggtgacacagcaagaccctgtctccaaaaaaaaaaagacagaaaaaaatccaaacagaaaagttgcatgcataatatcgtgaacacctgcacacccgcacaccctccacctcgattcaacatggtaccattctgcttcgtctgctttatctgtgcgtgtacccacacacttactattattattttttgctgacccacttgcatgtagttgcacttaagctttgctaagaataaggatattcccctacacaatcacagtaccataatcacatgtaagaaaattaacaccaattccttaacatctgccatgcagtccatattcagattttccatttgtctccaaaaagtctttcatggctgttttttccaaactgatatgcaatcatggttcagatgctccatttgtcaaataatgtctctttcatctgtttttaatctggaatatccacccccacttgtttcaagacattgacttgttgagggaacctccacctaccctcaactttttattttattttttataacggcaaatgctacacatctaattccatctctgatgtacacagaccctcgctggcacttctattttcagctttctgctcctgctccaagttaggaactcccaatggcttaaatgttttctcagataatctaatatgtggctgggcacagtggctcatgctataatcccagcactttgggaggccaaggcgggtggatcatgaggtcaggagttgaagaccagcctggccaacatggtgaaaccgtctctactaaaaatacaaaaattaaccaagcgtggtggcatgtgcctataatcccagctacttgggaggctgaggcaggagaattgcttaaacctgggaggtggaggttgcagtgagccaagactgcgccattgtactccagcctgagcgacagagtgagactccatctcaaattaaaaaaaaaaaatctaatatgcttctcttaatcatgaccctgatagtggtttaggcctgttcaaagcacttcacaatgactctaagaggtgggtaaattatcaccacctccatcttccgcatgaggaaactggagctcagaggggtgaagtcacttgccccaggtcacacagcaaagccaggatctgaacccaggcagtgtggctcactcacctgactgcagacgacctcctggcatggacttcttagccatctcggccagtactcctagccccaagcccacagccagtcctggagtgcaagagaagaacatgagtgcccgtttgcctggggtgcccccagcctaacccactctcctttctcagtttttctccaagaatgcttgtctcccaactctttttattttttcttttgtttgagatggagtctcgctctgttgcccaggctggagtgtggtggcacaatcttggttcactgcaacctccacctcccgggttcaagcgattctcctgcctcagcctcccgagtagctgggattacaggcacgcgcccaccacgcctggctaaattttttttgtatttttagtagagacggggtttcaccgtgttggccaggctggtctcgaactcctgacctcaggtgatcctcccgcctcggcctcccaaagtgctgggattataggcatgagacaccgcactcagtcttgtctcccaattctttgtatctctgtttccaaatcagtctctgactctgttcctgcatggggctccctttaaggtgcagcttcctctttctttaaccctttctccatgtctctgtctccctcccagcagttctcagccctggctgcacattccagttaccagaggagctccggtaaatataatgcccagactccactccccaaattctgattaaattggcctgagacatgggaatttgtgttttgttaaaaagcacctcagataattctaatgtgcgatcaaggttaagaaggcccctcggccgggcacagtggctcatgcctatgatcccagcactttgggaggccgaggtgggcagatcatctgaagtcaggaggtcgagaccagcctggccaacgtggagaaaccctgtctctactaaaaatacaaaatcagccgggcgtggtggtgcatgcctgtaatcccagctactcaagaggctgaggcaggagaatcgcttgaacctgggagacagaggttgcggtgagccgagatcacaccattgcactccagcctgggaaacaagagagaaactccgtctcaaaaaaaaaaaaaaaaagaaggccccgaaacaattgtcctaggtccctctgtcttctggtgactcttctttctctgtccacacctcctcttctttatgcttatctctttttctttttagagacagggtctcactctgtcgcccaggctggagtgcaatggcaccatcataactcactgcagcctcaaattcctgagctcaagtgatcctcttccctcagcctcctgagtagctgagaccacacgtgcataccaccacgctcacctaattttttattgagacagggtctcactatgttgcccaggctggtctggaactccagaactcacgtgatcctcctgcctcggcctcccaaagtgctgggattacaggtgtgggctaccaggcttgacctctccctttctaagccagttatttctgcatctcttgccttctccccatttgtcctatctatctagatctctttctctcttttcctccctttgatgttatctctccatctctgatttcctctgctacctctcctcttgtccctaaagacgtctcgggtctctctccttcttttgttgtcaccatctctgtcaattaccatatctggcattttctgtgtcctttctacatgtcaggggctgttcccagtgccttctgtgcacttactaatttttgtccttacatgaggtctccaccttcataaaatgtattttacagaaaacttccattttacagaaaaggaaattgaggttcagagaagtgaagtaatttgcccagagtcacgtcacaaagcgaggacacagcagagtcatcccttaatccctgggcagcctggtgccaaagctctaaccagtgcctttgactgcctctgcagactgtgaatctatctatgtatatatatatagattttttttttttgagacagagtttcactcttgctgcccaggctggagtgcaatggtgcgatcttggttcactgcaatctctacctcctgggtacaagcaagtgaatctatatttttaaaacttgaaccaggcggggcatggtagctcacgcctataatcccagcactttgggaggctgaggcaggtggatcacgaggtgaggagttcgagatcagcttgaccaacatggtgaaaccccatctctactaaaaatacagaaattagcggtcaggcacagtggctcacgtctgtaatcctggcactttaggaggccaaggcaggcggatcatgaggtcaggagatcgagaccatcctggccaacatggtgaaaccctgtctccctaagaaaaaaaaaaaaaaaaacaacaaaaaatagttggacgtggtggcgtgcatctgtaacccccgctactcaggaggctgaggcaggagaattgcttgaacctgggaggtggaggttgcagtgagctgagatcatgccactgcactccagtctgggtgacagagcaagactccatctcaaaaacaaaaacaaaaacaaaacttgaaccatgatcagcaataagaagacatttacgttataaccagtgcagaccaaggtatatgtttcacgaaacaagactttcccttgctctacaggtgcatgcatattttctgtcctattcttctttttaaatgctggttgcaacccactaaattatttcatgtgacttgcacgacatccggctgtgtaacccaaagtcaagtgacctcccctttgttagcctcaatgtcctcatgtacggaatagaacactcattgattcagtgcagcatgtgtgtatatgggacactgcacattacaggttctcagtaaatgttattatggccaggagcagtggctcatgcctagaaccccagcacttcgggaggccgaggcaggaggatcgcttgagaccaacttgagcaacatagggagaccctatctctacaaaaaaatattttttaaattacccaggccaggcacagtggcttcccgggcaccgtggctcacatctgtaaatcccaacactttgggaggccgaagtgggtggatcacttgaggtcaggagttcaagaccagcctggccaacatggtgaaattctgtctctactaaaagtacaaaaattagccaggcggccaggtgtggtggctcacgcctgtaatcccagcacttgggaaggctgaggcaggcggatcacaaagcgaggacatagcagagtcatcccttgaaccctgggcagcctggtgccaaagctctaccactgcctgacaaacatggtgaaaccccgtctctactaaaaatacaaaaattagccgggtgtggtggatgcatgcctgtaatcccagctacttgggagtgtgaggcaggagaatcggcttgaacccgggaggtggaggttgcagtgagccaagatggcgccactgcactccagcctgggtgacagagggatactccgtctcaaaaaaaaaaaaaaaaaaatagccaggcatagtggcaggcacctgtaatcccagctactcaggaggctgtggcaggagaattgcttgaatgtaggaggcagaggttgcaatgagccaagacggtgccactgcactccagcctgggcaacagagcgagactctgtctcaaaggaaaaaaaaaaaaaaattacccgggcggatggtgcacaactgtggtcccagctactcaggaggctgaggcgagagaattgcttgagcccagaagtttgaggctgcagtgatcgcgccactgcactccagcctgggtgacaaagtgagactctgtctcaaaaaaaaaaaaaaaaattatcatttatgttcctcttgatttctcttggccttgcaggcccttgcctttgtctctctttttttgtctctctctctttcctgtctctgattcatcctctcccttgcttcaatctgtaaatgttgccctttctaattgaggtcacaccaagatcccccaaagtcacacctacccccaaagttggccaagcggctgatgcgggaggcaggcaccttgcgttctcgagagcggtcactcagctgggaaatggggacaaggtctgagggtgggaaagtgggcatcgtggccagagagtgcagccactctgccaccacacccttccccaagctcagggggccagcagtattcgtggggtgttgctgggtgggtgggggtaatgatacctggggccggggtgtcttcctgggacgggcctcccgtgccctgcgaatgtcctcctcacccaggcctctcccaggcccatcctggtaaaacttttgggcccaagaacctccacatggtccctgcaagagatatactttgataaggaggggaggacatgggatcacctggcccttctggacccctcctgtccttttaccctctgaagtctccctcagcctcttccccttggggacctgctccctagcctcttacccagcggtggggcccaggccccagggccccacaaggccaaccaacagtctggcccagctgtccaccggtcccccgaagtaggccccccaccttcagccacattgcctggaggagaagaggagggattattcaggtgggagttgcctggcttcttggccaggcccccatgttcctctgtgtccaccctctctcattcccacccactaaatacttcctccactattaatagattcccacagtttctcctggttctcccctggttgctaggaacccttagctcttcctgcaggcctcccaaaacccactttcccccctctcccaaccctcgccgttgctagggtccgcccccgttactagacacccacagttcctcaggggctacctctccacttctctgaaacccccctcgttgctatgcaccgccttcccctctgttggccctgtaggcacccgcaattcctccggtgtccccccgcccgatccccaccccgttactgagcacctccccccgttgctaagcacccactgctctcagcctccgagtccgcaacctgctggggccctcctgtgcttccgggagcctctgtatgcccgcccccttcggccagccaaccaatggcgcggcagcaactcgctgactggcacggagtttctccatctgtgcgcgggggaaggggccagagagaggccctagcgatggagcctggaattaaggtgggcatcgggggcccatctggggggattgctgaggcatcgcgggagcgcaagcgtgccctgtctgcccttccactcacctcaaagtgccttgtacgcgacagacccttctgttccctacactttcttgcaaagtctcccttacaaacctgacgcctctcttctgcacgaatatcttgccaaccccccttcttatttttacccctggcaggctcaacacaattcctttgaatacacattcttcccagcaaacatttcccttgcacatggagcccctccactttgcacaaacacccacattctggcacccaacctccttccttgtgcatataaatcccttgccttgcttgccaactgtttcccgctcacgccttcaactctctcgtgtacataccctcccccccacttgcacactgagtctctgttccctcacacaccctgttctctccgctccccgcccacctgcggaatggtgcgactgggagccctctgcttcctgtaggcctgacatttcccagaacacactcagccaagattcccagtgctgagtcaggaaccttggcatcccagaaaaccacctcccatcctatctttctttctctgtgtgtgtgtgtgtgtgtgtgtgtgcgcgcgcgcgttggaaagcctgctctccccacaacaggctgactcacccacttctcacagtctggaatagaggcatctggttggggcatctttcccaccactgggagagggagggatgccgatgcttcccccacagaaccccgctgccccaacccctcttgtcgggaatcaggcctctttgtctctattcccgtactgtgtgacctcagaaaagccctcatccctctctggacttctccttcccaacctgtatgaggtactaggtgggctcctgccttcgatttctctcattggtctgtgaaaaggtgactcattttagagccttggacctgtgcccaatgtctcccccagttgactcaatttcaagacaaaccacctcctctcccccttcagaggtgaacggctgactcaggagctgggtggcagctcagccttgggggcaaaatatatcaaaatcacctaggacaataaataatcctactgggctacaactgacagtgccaggcccggggccacatgcttcacatacatgagatcatgtcagatagccccgtagctgcaagcaaagggtagaggccggcagatctctgagcctctgttctcacgtgtaaaatggagccctggcatccctattgttcagccttggagaatgaactgaaatcgtgtcagggtctgatacagaacaagtactctatacatgacagagatttcttacggaaaatccaatggagcgtaagtcatttgctcagggtagcggagctgggaactggcagaggaaggtctcgaacccacacccgtgggaactccaagtctttgaaagtccgtcccgcccctgcgtgaagaatgggcgcgcggctggactcgtcaccgggggttttagggaaggttgaacttgtcattcaaccgtgtagggagggtggtttagtcacaggggtggagggagggggcccactggcgcgccaccaggaccccggtgccctagatgcatacctggccgcgcttcggatgctcagaggcaaaccccctccccttgggaggcggagtcggacaaggctccgtctcgttccgttccgtcacgtccggtggggcggggcttcggggctttcccctttgaggggagtatcggttaacccttgcgcggcggggcgggctggagctccgcgggccggaacccgggagtcggggctccccagccacacccctcgcgggatttaaagggataggaggggccgggtcggccgaagcccgaaccgaaggagcgggcatgaggcgctgcccgtgccgtgggagcctgaacgaggcggaggccggggcgctgcccgcggcggcccgcatgggactggaggcgccgcgaggagggcggcggcggcagccgggacagcagcgacctgggcccggcgcaggggccccggcggggcggccggaggggggcgggccctgggcccggacagaggggtccagcctccacagcgagcctgagagggccggcctcgggcctgcgccggggacagagagtccgcaggcagaattctggacagacggacagactgagcccgcggcagctggccttggagtagagaccgagaggcccaagcaaaagacggagccagacaggtccagcctccggacgcatctagaatggagctggtcagagctggagacgacttgtctttggacggagaccgggacagatggcctttggactgatccgcacaggtccgacctccagtttcagcccgaggaggccagcccctggacacagccaggggttcatgggccctggacagagctggaaacgcatgggtcacagactcagccagagagggtcaagtcctgggctgataacctctggacccaccagaacagttccagcctccagactcacccagaaggagcctgtccctcaaaagagccaagtgctgatggctcctggaaagaattgtatactgatggctccaggacacaacaggatattgaaggtccctggacagagccatatactgatggctcccagaaaaaacaggatactgaagcagccaggaaacagcctggcactggtggtttccaaatacaacaggatactgatggctcctggacacaacctagcactgacggttcccagacagcacctgggacagactgcctcttgggagagcctgaggatggcccattagaggaaccagagcctggagaattgctgactcacctgtactctcacctgaagtgtagccccctgtgccctgtgccccgcctcatcattacccctgagacccctgagcctgaggcccagccagtgggacccccctcccgggttgaggggggcagcggcggcttctcctctgcctcttctttcgacgagtctgaggatgacgtggtggccgggggcggaggtgccagcgatcccgaggacaggtctggggtgagtgggacccatcctgcccttgagccacatcacgcaaaactccttattcctccgcctttgcttaggaagttctctacccatttactgttagttgcccaccagcaatttcatctccgggaacctcttccatccactgacctcctccctctgacagccaggttactaattcactccaggcaccccttcttaattctctcctttccccttcctgcactgtctccactcctgggggtctacaatggagggccactgaccgactttatggggcccaggaacccctgaaattgtaggactaaggagcctgccgtgcgtgttcacatacattgttgcagcgacggtctgacatctgtctaatcctctggaatctgaagaacactgggatagggagacaggcagggtgcactttctaccccacatttcttaatctggggcctgtggctgtcttaaagggtcacaaaccttcaccaccccttagcctatttgtatgtacatttttctagggagcaaagcgattcccccagcttgcatcagattcgcaaaagggctgtgtgaccccaaacgccaaaggatccttggcctagccgggagcccacctggtctcccctgtgacccctacatccccaaggagccccctgaacactcttgtttactttgtccaccgtcacccccagcttgggtgtggctctcccctggtgaatcaggaggaccggccgggcaggttcagggagggcgggacagagcagaggccggtgtgaaactggagagcctcacgtggggctgggagccgtggggctgggagccgagtccggagtccatcagcttgccagcttgcctgctgaggcctctttttgctctggggcccctggctggagtctgccctgagccccgcttcaccccacatgccttccttggggacgtgttcacacatgtggccctagctgtgagagacagacctgccttgacgtgcctgtgcctgtgtgcaggggctgaccctcctgggccccattgcttttttctctctgcctgccctctcacttccttggcatctcagaacagctgagctggaagtgggtgaataataataataataataataataataacaacaacaattagcactcactcatgtttagccctgtgctaagtgctgtgcttttattaactcactcactcctcgcagcaaccctaatgaggtagatactttttttttttttctgagacagtctcgctctgttgcccaggctggagtgcagtggtgccatctcggctcactgcagccttcacttcctgggttcaagtgattgtcctgcctcagcctcctgagtaggtgagacaccaggtgcccgccaccacacctggctcatttctgtattttgagtagagacagggtttcatcatgttggccaggctgacctcaagactcctgacctcaagtgatccacccgcctcagcctcccgaagtgctggaattaccagcatgagccactgcacccggctgaggtagatactattattatccccttttacagatgaggaaactgaggcacagagaattcaagtcacttgtccaaggatatcaccttgcaagatgcagatcaaataattctaatccttactgtacaccagacactgttttaagttttttcttcttttttttttttagtcttttttgtcaatttttttctgtcattttttatcttaaaatagcatctatcttaattaagggctttgtatgtgttaactctgagtccttatgacagcactgagattgtctccattcaacagatgggggccaggctcagtggcccaagcctgtaatcccagcactttgggaggccgaggcagggggatcacctaaggtcaggagttcaagaccagcctggccaacatgatgaaaccctgtctctactaaaatacaaaaattagccaggcgtgtgatggcgggcacctgtaatcccagctacttgggaggctgaggcaggagaatcgcttgaatgtgggaggcggaggttgcagtgagccgagattgcaccactgcactccagcctgggtgacagagcaagactcggtctcaaaaaaaaaaaaacaaaaacaacagatggggaagctgaggcatagagaggtgagagattctttgcttagggttggccacgtcaagtcagagccaggattctaactcagttctggctgagtttcaaacccatcgtttaaaccctccagtgtgtagatctgttcctaacttgtctccctcccaggcctccctatctccagtttttttctcatccttccagaatctgcctccatggcccagctttgtctgctcaggtgccctctctgagagcagtcaggggctcagtgctgcgtttggagcctccggtctccaggcgccttcccagaatcgacttccttccctcctcctgaccccctctgctgtaactaggcctgagtacacactgttccttgaacactcttctgttgtcctgcctccacgcattgctcaagccgttcccactgcccagcatacccgtgcttccttctcccttaattttgaaatcctctctgaccgtaaaggctcagcttcctttctccctttcctccttccttccttctcaccatcctgtcctttttttaaaattgtgttctctttctttttctttttttggtagggatggggtcttgctatcttgcccaggctggtcttgaactcctgggctcaagtgatcctcctgcctcagcctcccaaagtgctgggattacaggtgtgctatcctattcttctaatgagacaaaaatcactccctaagcccctaccatgtatttggtcctatgttagctttgctggggaaacagcagtgaccaagacactcatggagctcccaggcccatgaaagagacagaccaatcagccgacagtcacagttcagagtggtcaggaggatgtgtgagcccagaaggaggtcactggccagacacagggtatcagagagggcttcctggaggaaggggcatataagctgagaccattgtgaaaaaaatccgagaaagcccagataaaccattggatctaactttttttttttttttggagggcgtgcagtgcggagtttcactctgttgcctaggctgaagtgcagtggcgagatctcagttcactgcaacctcagcctcccgggttcaagtgattctcctgcctcggcctcccaagtagctgggactacaagcgcacgccaccacgcccggctaatttttttttttagtagagagtgggtttcactatgttggccaggctggttctgagctcctgacctcaggtgatccacccacctcagcctcccaaagtgctgggattacaagcatgagccactgtgcccggcccggatctaacataaaacagagagagaagatattatgtttatgattaaggggccaggtgtggtggcttatgcctataatcccagcactttgggaggctgaggtgggaggattgcctgagcccagaaatttgagaccaccctgggcaacacagtgagacctcatctctactaaaaggaaaaaagaactagctagatgtggtggtatatgcctgttttccagctattcgggaggctaaagcaggaggattgcttgagcctgggaggcagaggttgcagtgagccaagatcacacctctgcactccagcctgggcaacagagtgagatcctgtctcaaaaaaaaaaaaaattactattaaaaaaatcccaactaacattcttcagtccaagcatcaaagaatgtttctggagcgtctgtcgtgtgccaggccatgtgctggggacataatcataaccatgacaaccccagtctctgccatcatgagcttgtagtccagcaagtgtgtaggggataagccccaaggcactgggatccaaccagagctagaaccccagcgctgtgtggggtgatgttaggtaagtggcttcacctctcagaccctctgtttcctcctttgtaacaccgagacgataatctccctggggttgtgtttttagaaattaagtaggttgtggcacactgagtctttgtcattgtgtctggaatgttccaggtacttagtaaacaggaacctttattaatcatctcttccccagggccggcagctggattggggagggactagcccttcccgaaccctgactccctcttaaccttcccactgtcaaagagatgtctgtgaggtagctgggctctgagggggcgggagagatgaacacgtccctgatcctggggtaggagagggatgagccatacagtttccttctctggaggtgacccactcttccagtacttgctaagggacttgacatgcttgtggggtgcagaatgtattcctgtgtgtgtatgtgttcatgaatcagacactaaccctgtctcaaaaagctcatagtttagtcggcatgatacaacgaaaaccctgttttctatttgcttctctggttttctttctttctttcttatttttttgagtcagggtctcactgggtcacccagtctggagtgcagtggcacaatcactgctcactgcagcctcaccctccagggctcaagtgatcctcccaccttagcctcctgagtagctgggactacaggtgcacaccaccacgcctagctgattcttaattttttatttatttatttatttattttttgagatggagtctcgctttctcgcccaggctggagtgcagtggcacaatctcggctcactgcaacctctgcctctcaggttcacaccattctcctgcctcagcctcccgagtagctgggactgcaggtgcccgccaccatgcccagctaattttttgtatttttagtagagacggggtttcactgtgttagccaggatggtctcaatctcctgacctcatgatccgcctgcctcagcctcccaaagtgctgggattacaggcatgagccactgcgcccggcctaatttttaaacattttgtagagatggggtcttgctatattgcccaggctggcctcaatctcctgggctcagtggtcctcccaccttggtttcccagtgttgagattacaggcgtaagccatcgtacccgctgcttttgtggtttcctttgttctctctctctttgtctacttctgttcatctttttcttttcatcattactttgtatctctctcttttagtcttcctatatttgttttgttttttttttgtttttgagacagtcttgctctgtcgcccaggctggagtgcagtggcgtgttcttggctcaccgcaacctctgcctctcgggttcaaacgactctcatgcctcagcctcctgagtagctgggactacaggtgtgtatcaccacgcccggctaatttttgtatttttagtagaggtggggtttcaccatgttggccaggctggtctcaaactcctgacctcaggtgatctgcccacctcaccctcccgaaatgctgggattacaggtgagagccaccacacccggcctatttctttatcttttagcaattctatacctgtctctgtattagtcagggtaggtcaggattttctgcagtaacaaagagcccccaaatcttagtgacttagaacaacaaaggattattttgctttatactacacattggtcacaggtcagtggtgggtcaagggctctgcttcatgctgtcttcactcagggtcccaggctgagggagcttccatttcttttcttactccctcccccactggggaacaaacgtggcgagtcataaactggctcttaaggctcctacccgaaagtgacacttctgctcccagttaattggccaaagcaaggccaggtgtggtggctcacacctataatcccagcactttggagaccaagatgggaggattgcatgaggccaggagttcaagaccagcctgggcaacatagcaagatgccataaagtagctgggcatggtggcacacgcctgtagtcctgactactcaggaggctgggatgggagcatcgcttgagtccaggagttggaggttgcagtgagctatgatggtgccattgtactgcagtctggctgacggagtgagacccggtctctaaaacaaaacaaaacaaacaaaaaacaacaatccccagttcaggagggcagggacatccctgaactaatagctggagctatgtggtgaacagctgtcatgactgccacggtctctgtcgctgtctctgtctctctgtcatcactatgtcatctgcctctctgtttctgtctctctctgtggtccatctccatccatcaactcctgcctctataattttccccaaaaggtctgacctggtttagggacagagatggggcttccaatatttgacactggtccctacataatggcttatgcctgaaaccccaacactttgggagactgaggcaggtggactgcttgaggtcaggagctcaagaccagcttgggcaacatggtgaaaccccatctctactaaaaatacaaaaattagccagacatggtggcatgcacctgtagtcccagctactcggagggtgaggcaggaggatcacttgaacctcggaggcagaggttgcagtgagccaagatcataccactgcactctggactaggtgacagagaccctgtctcaattaaaaaaaaaaaaaaaagaagatttggaactgtgtatgtgcagtggaagatgtaagggttgtttgttaaaccacaacaaaacctagcctgtccttactcataagatccttactcataagagaaggacagagagacatagatacaaagaaagtgatgacagaggggagaaatgggcaaagaatttcccctatcttgctgagggctttgggcgatcatgtgattgccgaactaagtggggctcactcaccccaacaagcctgggaacagtgatcccaggaagcccctggccctggaaagactgcaggtcccctttcgttccctctcatggcagcacctctagcccctgccttccctggccttggccctgaccccaccctgctctgctccctacagagcaaaccctggaagaagctgaagacagttctgaagtattcaccctttgtggtctccttccgaaaacactacccttgggtccagctttctggacatgctggtaagtggggtggtggtggacagagctgggcagagtctcctgggccagggaaagggatgttctctgtagtttagttcccccacctagtgatgggcttggtgacagtccccaccttatgggactgttatgggcagtgcttaggcctgggcctggcccttcgtatgtcagggcagagggctattccttgttattctggtggagagagggagcttcagacggacctgagctcaaaccctagttctgctctgtattcatgggtgaccttgggcaagttactttcctttactgggcctcagctgccccatctgttaatgtggagataaccttacctcccttgcaggattaaccgaagagttaaaatcaaaatgtatataaagattgaggccaggcacggtggcttacatctgtaatcctagcactttggcaggccaaaacaggaggatcgcttgagcccaggagtttaagaccaacctaggcaatatagtgagaccccgtttcaattaaaaaaaaaaaaagattggctgggcgcagtggctcatgcctgtaatcccaggcctttgggaggccgaggtgggtggatcccctgaggtcaggagtttaagaccagcctggccaatgtggtgaaatcccttctctactaaaaataaaaaaattagccaggcatggtggcgggtgcctgtaatcccagctactcaggaggctgaggcaggagaatcacttgaacccgggaggtgaaggttgcagtgagccaagatcgcagcattgcactgcagcctgagtgacaagagcgaaacttcgtctcaaaaaaaaaaaagactgaggcacaggactcttatgaatggaaatgatcactccttgccttctccgcgtgttcagagcatagcaggccttcagtaagtagcagctgtaacattttgcccccaggaccttgcaaatgcctgcagcacagagtagcacaatggtggcatatagtgctcttttgaaaggctaggccataaatatcttaggttttgtgggcctatggtctctgtcgcaactactcagctctgctgttacagcaggaaagctgccatagacactatgtaaacatatgagtgtgtctgtattccaataaaactttatttgcaaaaaccagcagcaggctggactagaaaagtgtgcccattggcaaatggcgacagtaagagaatttgtctgccttgtttgtctttagatctgacctggaaataaggcaagaccccctaaaactgtgtcaacacaagtttgccatctatatgtgttctggttactattgctgagtttattaaaaaaacaaaactcagcagagcacagcggctcatggctgtagttctagcactttgggaggctgaggtgggaggatcacttgagcccaggagtttgagaccagcctgggtgacatagtgagaccttgtctctacgaaaaataaagaaattaactgggcatggtggcatgcacctgtggtcccaggtacttgggagctgagggtgggaagatcacttgagtccaggaggtctgggatgcagtgagccttgatcgcaccacagtactctagcctagatgaccgagtgagaccctgtctcaaaaataaatacgccaggggcggtggctcacgcctgtaatcccagcactttgggaggccaaggcaggcggatcacgaggtcaggagatcgagaccatcctggctaacaaagtgaaaccccgtctctactaaaaatacaaaaaattagccgggcatggtggcgggcgcctgtaatcccagctactcgggaggctgaggcaggagaatggcgtgaacccgggaggcggaggttgcagtgagccgagatagcaccactgcactccagcctgggtgacagagcgagactctgtctcaaaaataaataaataaataaaataaaataaaataaatacaaaacaaaacccaaaaaccccaagacttagtgatggttaaaaaaaataacttagtagaataaaacaatcattttattgacctcagaagttttgggtcagcaattcagacaggatggcagggatggcttttcactgctccacaatatctgggaactcagctagggacacctggaggctacaagctgaaaacttttggaggttcattcacttgcatgcgtggtgattgatgctggctattggctggggtctcagatggggctgccacgtggctttgccatgtagctccttgagcttcctcacagtatggtggcctcagagtactcagatttctaacaagacagctcaggactaccttgaaggtaagtgtctctgccaacagaagtcatgcagtagcacttctgccataaaccgtcccatatttaatgggagagcaatctattttttatttattcatttaattttgagataggatctcagtgttgcccaggcgggagtgcagtggtgcagtcatagctcattgcagccttgaactcctggccttaaaggatcctcctgcctcaacctcccagagtgttgggattataggcatgagccactgcacccagcttgggagagcaattaagagtatactccttgatgggaaaattctataagagcaggatcaggaatgggtctgagacccactgtgatcaggagatactgttgtagccaactttggaaaatgtaatccaggctggacataatcacagcactttgggaggctgagatgggaggatcatttgaggccaggagttcgagaccagcctgggcatcatagcaacactaccccaacccgacattacacattttttttttttagattagctgggagtggtgggggtgcacacctgtagtcctagctactctggtggttgaggtgggaggatcacctgaatctaggagcttgaggctgcagtgagctatgattataccactcaatttcagcctgggtgacagagtgagatcctctcaaataaaaaaagaaaaagaaaatataatctgaaaatacagctggccactagaagaaattagaattattataatctatacactctgcgtggtccaggaaatgcttgatctataaattaacttaaataggccctggttgttagcaccttgggattccaggcagcagcaaaagcaaatccactctggagagtgacgctctggacttagatctcacagaattcccacagatgatcacatgtgtacaatcaaaaattacaaaacaaattaggatatcctgtgctgggaacaggacttggtttaagcaacagagaacagaaattcgccctttccttaccaacccctgggcaagacttttaagagttgcggcctgggcacagtggctcacgcttgtaatcccagcactttgggaggccaaggcgggtggatcatctgaggtcaggagttcaagaccagcctgaccaacaaggtgaaaccctgtctctactaaaaatacaaaaattagctgggcttggtggtgtgcacctgtaatcccagctacttgagaggctgaagcaggagaattgcttgaacccgggaggcggaggttgcagtgagccgagatcgcaccattgcactccagcctgggcaacagagtgggactccatctcaaaaaaataaaataaaatcttaaaatcattaaaaaaaaagttgcagggagagaaagcattgcaggagggtcgggcaagataatggtggccaggatctgatgcaaacaggcagctgcggagaggttctcttcctgatccagttcctgatcctctcatttattctaccacctttagggaacttccaggcaggagaggatggtcggattctgaaacgtttctgtcagtgtgagcagcgcagcctggagcagctgatgaaagacccgctgcgacctttcgtgcctgcctactatggcatggtgctgcaggatggccagaccttcaaccagatggaagacctcctggctgactttgagggcccctccattatggactgcaagatgggcagcaggtggggctggggcagccctggggcagggatggagggcagggggtgggcattattgaaaatattggcctggccaggcgcggtggctcacgcctgtaatcccagcactttgggaggccgaggctggtggatcacctgaggttgggagttccaaaccagcctgaccaacgtggtgaagccctgtctctactaaaaatacaaaaaattagccaggcgtggtggtgcatgcctgtaatcccagctactcaggaggctgaggcaggagaattgcctgaacctgggaggtggaggttgcggtgagctgagattgagccattgcactccagcctgggcaacaagagtggaaccctgtctcaaaaaaaagaaaagaaaagaaaagaaaatagcgccaagtccattttcaaagtggttgtaccagtgtaccttcccaccaccatgtatgagtgttacagtcgtcccagattctcaccggtgcttggtactgtctgttttattaacttaaaccattccgatgggtttggaataggatccctttttttcctctttgagacagagtcttactctatcgcccaggctggagtgcagtggcacgatctcggctcactgcaatctccacctcctgggtttaagtgattctcctgtgtaaaccaagtagctaggattacaagcgcccgccaccacacctggctaatttttgtattattagtagagatggggtttcaccatgttggccaggctggtctggaactcctgacctcagatgatccacccactacggcctcccagaatgctgggattataggcgtgagccaccacgcctagtctgcaagaagtgaactctaattgctttctccagctgggttcagtggctctcacctataatcccaacactctgggaggctgtatacacacacacacacagacacacacacacagacacacacatagtcttcaactctcccatttcattcttttagtagtcttttgataaacatatttttataaacaaaatagtatttgtattattactcttttttgagacagagtctcattctgttgccccgactgaagtgaaggagcatgattatagctcacagtagccttgaactcctgggctcaggcggtcctttcaccttagcctccagagtagctgggactataggtatgtcccaccaggcttggctatattttattttttatagagacatggtctccctgtactgcccaggctggtcttgaacccctgagctcaagtgatcctccttcttctgccccctgagtagctgggactgtaggtgcatactatcacacctagctaattttcaattttttgtagagacaggctatttaggaaaagctctgaatccatgcttttccgttctcacaccactgccacaacaatgagagcacagaagacttctgtgaccaaatgtttaggttttttaaccccacacaccaagcaacggacaccagctggatgtcctccaattcaagtctaaaaccatctacctggaaatagtgtcagatcccacaggttggggactcagtccccaagactgccccccagttacagacaccagtcataagttcaggccttcgaaacttctgactgattggctccaagttggagttcccatgtcctcctctttgggttcaaataatttgctggagtggctcaaataactcagggggatacttacttacctttactggtttaatataaagcaggggtccccaacccctgggccgcagaccagtaccggtccatggcctcttaggaacggggccccaccgtaggaggccagcgagcattaccgcttgaactccacctcctgtcagactagcgggcaggagattctctggagggcgaaccctattgtgaactgtgcctgcaagggatctagattgtatgctcctatgagaatctaattgatacttgatgacctgaggtagaagagtttcatccagaaaccatccccctcacagtctgtgggaaaaattatcttctacaaaaccagtccctggttgggtactgctacaaaggatactgcaaaagatgaagagaagtgtagggcaaggtatgggggaaggggtacggagcttccatgccctccctgggcgcaccacgctccaggaacctccacagggtcagctatctggaagctcctgagcccaatccttggtttttttttttttttttttttttttgagagggagtcttgctctgtgtcccaggctggaatgcagtggcctgatccgcccgccttggcctcccaaagtgctgggattagagatgtgagccaccatgcccagcctaatccttgggtttttatggaggctttaagacaccagcattccttcccccagagtatagggtgggatcctctctggggagggtcctaagacccacagtcaggaaggtggggaaagattagagtcctgccttggggcaggtgaaaggagggcaggaggaggtcagagattttggtttcttgagccagcttctgagatctaacacacctaaaattataacaaaagattgtggctgggcgcagtggctcatgcctgtaatcccagcactttgggaggccaaggcaggcagatcacttgaggccagttcaagacaagcctgggcaacatggtgaaactctgactctactaaaaaaatacaaaaatgtgccaggtgtggtggtatactcttgtaattccagctactcaggaggctgaggtgggaggatcacttgaacccgggaggtcctagaagttgcagtgagccaagatcacgccactgtactccagccttggtgacagagcaagactccatctcaaaaaaaaaaaaaaaaaaaggctgggcgtagtggctcacacttgtaaatgggaggcagaggcaggccgatcacgaggtcaggagttcgagaccagcctggccaacatcgtgaaaccccatctctactaaaaatacaaaaaattatccgggtgtggtggcgggcacctgtaatcccagctactcaggaggctgaggcaggagaatcgcttgaatccgcgaggcagaggttgcagtgacccgagatcaccaccattccattgcactctagctcgggcgggcgtcaaaaaaaaaaaaaaaaaaaaaaaaaagattgtaacaagggctatgagagttaccagccaggaaccatagagggaaaccaatatacattgtaactaacaccgggtctcgctatgttgccgaggctgatcttgactttctgggctcaagtgaacctcctgccttggcctcccaaagtgttggggttacagatgtgaacactgcacctggccctacctttaatttagtccagtttgtcagtttttttcattgtgtttaagaaatcttttcctactccaagatcatgcaaatattatgttttcttctacaagctttattgttttagctttcatatttagacctacattccagatagaattaatgtttctgtgtgtgggaggtagggatcaggttcatttttttccatatggattgttgacccagcactgtttattgaaaagacttccctttccccactgaattgcagtgcctagtcataactgcacaactctacgtgtgtgtctttgtggactctgttgtattctgtgcattgatttgcccattcttgtgccacactgtggctttatgtcttaatatcaggaagggtaagccctccagtttgttctacataatttcctttgtcacatcctctgtgtgctcaggacctatctggaagaggagctagtgaaggcacgggaacgtccccgtccccggaaggacatgtatgagaagatggtggctgtggaccctggggcccctacccctgaggagcatgcccagggtgcagtcaccaagccccgctacatgcagtggagggaaaccatgagctccacctctaccctgggcttccggatcgagggcatcaaggtgaggaccaggaaccgcctggcctgtcccgggaaggcctatagccagatcccaggcagggcttcttggggaaagccacgagagagtgcaggagacggcgtgggatgaaaggctggggctggggaagcccagcctctttcttacctccatacccatcagagcccaggttctgtttatccgtctgcctgagcatctcctgagtccatcttttcctcctctccttctccatggtcatgtcctagtccagccccatcttctcctgcctctgtctccctgggcatcctggccctggtctccctgcagcacaagagctggagggatccctttcccccagctatggagaaggtttctctttttctttcttgcattcctttttctttgtcaaattaaatataattgtatgaataggccaggcatggtggctcatgcctgtaatcccagcactttgggaggccaaggcaggaggattgcttgaggccaggagtagttcaggactaagctggccaacatagggagcttctgtttctagaagaaaaaaaaattgtttgaatagctagtcacacagttcaaaagtcaaaataatattataaaagggtaaatgtggagaaatttctctcccaactctgctgctgtccttcccattctgtccctctatccctctacctgctcatggggaaccactttgtcagtttcttgtatttcttcctgttagtgccagtaaatggagttgtagatccgaaatgttcctcagtacgcatactgattggtactttgctattttcacttaatagtaacaccctgcagagttttccacatcattccatagaaagcttcctctttctgtttttttttcccccacagctatgtaacactgtttttgtgactgtgcctggtcccctatagacagacacctgggttgtttccattttttgccattagcaggcctcaaagaatcactttgtatataagacattttgcaagtatgcagattgagctgtagatttccagaagcaggactcctgggtcaaagctt